European Patent Application EP 4 321 522 A1, published February 14, 2024. Title: CYTOTOXIC COMPOUNDS AND CONJUGATES THEREOF. Applicant: Seagen Inc. Application US. The sequence listing filed with the application follows.

SEQUENCE LISTING (1044 sequences)

SEQ ID NO: 1 - protein, 453 aa, synthetic construct
QVQLVQSGAEVKKPGSSVKVSCKTSGDTFSTAAISWVRQAPGQGLEWMGGIIPIFGKAHYAQKFQGRVTITADESTSTAYMELSSLRSEDTAVYFCARKFHFVSGSPFGMDVWGQGTTVTVSSASTKGPSVFPLAPSSKSTSGGTAALGCLVKDYFPEPVTVSWNSGALTSGVHTFPAVLQSSGLYSLSSVVTVPSSSLGTQTYICNVNHKPSNTKVDKKVEPKSCDKTHTCPPCPAPELLGGPSVFLFPPKPKDTLMISRTPEVTCVVVDVSHEDPEVKFNWYVDGVEVHNAKTKPREEQYNSTYRVVSVLTVLHQDWLNGKEYKCKVSNKALPAPIEKTISKAKGQPREPQVYTLPPSRDELTKNQVSLTCLVKGFYPSDIAVEWESNGQPENNYKTTPPVLDSDGSFFLYSKLTVDKSRWQQGNVFSCSVMHEALHNHYTQKSLSLSPGK

SEQ ID NO: 2 - protein, 452 aa, synthetic construct
QVQLVQSGAEVKKPGSSVKVSCKTSGDTFSTAAISWVRQAPGQGLEWMGGIIPIFGKAHYAQKFQGRVTITADESTSTAYMELSSLRSEDTAVYFCARKFHFVSGSPFGMDVWGQGTTVTVSSASTKGPSVFPLAPSSKSTSGGTAALGCLVKDYFPEPVTVSWNSGALTSGVHTFPAVLQSSGLYSLSSVVTVPSSSLGTQTYICNVNHKPSNTKVDKKVEPKSCDKTHTCPPCPAPELLGGPSVFLFPPKPKDTLMISRTPEVTCVVVDVSHEDPEVKFNWYVDGVEVHNAKTKPREEQYNSTYRVVSVLTVLHQDWLNGKEYKCKVSNKALPAPIEKTISKAKGQPREPQVYTLPPSRDELTKNQVSLTCLVKGFYPSDIAVEWESNGQPENNYKTTPPVLDSDGSFFLYSKLTVDKSRWQQGNVFSCSVMHEALHNHYTQKSLSLSPG

SEQ ID NO: 3 - protein, 453 aa, synthetic construct
QVQLVQSGAEVKKPGSSVKVSCKTSGDTFSTAAISWVRQAPGQGLEWMGGIIPIFGKAHYAQKFQGRVTITADESTSTAYMELSSLRSEDTAVYFCARKFHFVSGSPFGMDVWGQGTTVTVSSASTKGPSVFPLAPSSKSTSGGTAALGCLVKDYFPEPVTVSWNSGALTSGVHTFPAVLQSSGLYSLSSVVTVPSSSLGTQTYICNVNHKPSNTKVDKKVEPKSCDKTHTCPPCPAPEAAGGPSVFLFPPKPKDTLMISRTPEVTCVVVDVSHEDPEVKFNWYVDGVEVHNAKTKPREEQYNSTYRVVSVLTVLHQDWLNGKEYKCKVSNKALPAPIEKTISKAKGQPREPQVYTLPPSRDELTKNQVSLTCLVKGFYPSDIAVEWESNGQPENNYKTTPPVLDSDGSFFLYSKLTVDKSRWQQGNVFSCSVMHEALHNHYTQKSLSLSPGK

SEQ ID NO: 4 - protein, 452 aa, synthetic construct
QVQLVQSGAEVKKPGSSVKVSCKTSGDTFSTAAISWVRQAPGQGLEWMGGIIPIFGKAHYAQKFQGRVTITADESTSTAYMELSSLRSEDTAVYFCARKFHFVSGSPFGMDVWGQGTTVTVSSASTKGPSVFPLAPSSKSTSGGTAALGCLVKDYFPEPVTVSWNSGALTSGVHTFPAVLQSSGLYSLSSVVTVPSSSLGTQTYICNVNHKPSNTKVDKKVEPKSCDKTHTCPPCPAPEAAGGPSVFLFPPKPKDTLMISRTPEVTCVVVDVSHEDPEVKFNWYVDGVEVHNAKTKPREEQYNSTYRVVSVLTVLHQDWLNGKEYKCKVSNKALPAPIEKTISKAKGQPREPQVYTLPPSRDELTKNQVSLTCLVKGFYPSDIAVEWESNGQPENNYKTTPPVLDSDGSFFLYSKLTVDKSRWQQGNVFSCSVMHEALHNHYTQKSLSLSPG

SEQ ID NO: 5 - protein, 213 aa, synthetic construct
EIVLTQSPATLSLSPGERATLSCRASQSVSSYLAWYQQKPGQAPRLLIYDASNRATGIPARFSGSGSGTDFTLTISSLEPEDFAVYYCQQRSNWPTFGQGTKVEIKRTVAAPSVFIFPPSDEQLKSGTASVVCLLNNFYPREAKVQWKVDNALQSGNSQESVTEQDSKDSTYSLSSTLTLSKADYEKHKVYACEVTHQGLSSPVTKSFNRGEC

SEQ ID NO: 6 - protein, 453 aa, synthetic construct
QVQLVQSGAEVKKPGSSVKVSCKTSGDTFSTAAISWVRQAPGQGLEWMGGIIPIFGKAHYAQKFQGRVTITADESTSTAYMELSSLRSEDTAVYFCARKFHFVSGSPFGMDVWGQGTTVTVSSASTKGPSVFPLAPSSKSTSGGTAALGCLVKDYFPEPVTVSWNSGALTSGVHTFPAVLQSSGLYSLSSVVTVPSSSLGTQTYICNVNHKPSNTKVDKKVEPKSCDKTHTCPPCPAPEAAGGPCVFLFPPKPKDTLMISRTPEVTCVVVDVSHEDPEVKFNWYVDGVEVHNAKTKPREEQYNSTYRVVSVLTVLHQDWLNGKEYKCKVSNKALPAPIEKTISKAKGQPREPQVYTLPPSRDELTKNQVSLTCLVKGFYPSDIAVEWESNGQPENNYKTTPPVLDSDGSFFLYSKLTVDKSRWQQGNVFSCSVMHEALHNHYTQKSLSLSPGK

SEQ ID NO: 7 - protein, 452 aa, synthetic construct
QVQLVQSGAEVKKPGSSVKVSCKTSGDTFSTAAISWVRQAPGQGLEWMGGIIPIFGKAHYAQKFQGRVTITADESTSTAYMELSSLRSEDTAVYFCARKFHFVSGSPFGMDVWGQGTTVTVSSASTKGPSVFPLAPSSKSTSGGTAALGCLVKDYFPEPVTVSWNSGALTSGVHTFPAVLQSSGLYSLSSVVTVPSSSLGTQTYICNVNHKPSNTKVDKKVEPKSCDKTHTCPPCPAPEAAGGPCVFLFPPKPKDTLMISRTPEVTCVVVDVSHEDPEVKFNWYVDGVEVHNAKTKPREEQYNSTYRVVSVLTVLHQDWLNGKEYKCKVSNKALPAPIEKTISKAKGQPREPQVYTLPPSRDELTKNQVSLTCLVKGFYPSDIAVEWESNGQPENNYKTTPPVLDSDGSFFLYSKLTVDKSRWQQGNVFSCSVMHEALHNHYTQKSLSLSPG

SEQ ID NO: 8 - protein, 453 aa, synthetic construct
QVQLVQSGAEVKKPGSSVKVSCKTSGDTFSTAAISWVRQAPGQGLEWMGGIIPIFGKAHYAQKFQGRVTITADESTSTAYMELSSLRSEDTAVYFCARKFHFVSGSPFGMDVWGQGTTVTVSSAKTTAPSVYPLAPVCGDTTGSSVTLGCLVKGYFPEPVTLTWNSGSLSSGVHTFPAVLQSDLYTLSSSVTVTSSTWPSQSITCNVAHPASSTKVDKKIEPRGPTIKPCPPCKCPAPNAAGGPSVFIFPPKIKDVLMISLSPIVTCVVVDVSEDDPDVQISWFVNNVEVHTAQTQTHREDYNSTLRVVSALPIQHQDWMSGKEFKCKVNNKDLPAPIERTISKPKGSVRAPQVYVLPPPEEEMTKKQVTLTCMVTDFMPEDIYVEWTNNGKTELNYKNTEPVLDSDGSYFMYSKLRVEKKNWVERNSYSCSVVHEGLHNHHTTKSFSRTPGK

SEQ ID NO: 9 - protein, 452 aa, synthetic construct
QVQLVQSGAEVKKPGSSVKVSCKTSGDTFSTAAISWVRQAPGQGLEWMGGIIPIFGKAHYAQKFQGRVTITADESTSTAYMELSSLRSEDTAVYFCARKFHFVSGSPFGMDVWGQGTTVTVSSAKTTAPSVYPLAPVCGDTTGSSVTLGCLVKGYFPEPVTLTWNSGSLSSGVHTFPAVLQSDLYTLSSSVTVTSSTWPSQSITCNVAHPASSTKVDKKIEPRGPTIKPCPPCKCPAPNAAGGPSVFIFPPKIKDVLMISLSPIVTCVVVDVSEDDPDVQISWFVNNVEVHTAQTQTHREDYNSTLRVVSALPIQHQDWMSGKEFKCKVNNKDLPAPIERTISKPKGSVRAPQVYVLPPPEEEMTKKQVTLTCMVTDFMPEDIYVEWTNNGKTELNYKNTEPVLDSDGSYFMYSKLRVEKKNWVERNSYSCSVVHEGLHNHHTTKSFSRTPG

SEQ ID NO: 10 - protein, 213 aa, synthetic construct
EIVLTQSPATLSLSPGERATLSCRASQSVSSYLAWYQQKPGQAPRLLIYDASNRATGIPARFSGSGSGTDFTLTISSLEPEDFAVYYCQQRSNWPTFGQGTKVEIKRADAAPTVSIFPPSSEQLTSGGASVVCFLNNFYPKDINVKWKIDGSERQNGVLNSWTDQDSKDSTYSMSSTLTLTKDEYERHNSYTCEATHKTSTSPIVKSFNRNEC

SEQ ID NO: 11 - protein, 453 aa, synthetic construct
QVQLVQSGAEVKKPGSSVKVSCKTSGDTFSTAAISWVRQAPGQGLEWMGGIIPIFGKAHYAQKFQGRVTITADESTSTAYMELSSLRSEDTAVYFCARKFHFVSGSPFGMDVWGQGTTVTVSSAKTTAPSVYPLAPVCGDTTGSSVTLGCLVKGYFPEPVTLTWNSGSLSSGVHTFPAVLQSDLYTLSSSVTVTSSTWPSQSITCNVAHPASSTKVDKKIEPRGPTIKPCPPCKCPAPNAAGGPCVFIFPPKIKDVLMISLSPIVTCVVVDVSEDDPDVQISWFVNNVEVHTAQTQTHREDYNSTLRVVSALPIQHQDWMSGKEFKCKVNNKDLPAPIERTISKPKGSVRAPQVYVLPPPEEEMTKKQVTLTCMVTDFMPEDIYVEWTNNGKTELNYKNTEPVLDSDGSYFMYSKLRVEKKNWVERNSYSCSVVHEGLHNHHTTKSFSRTPGK

SEQ ID NO: 12 - protein, 452 aa, synthetic construct
QVQLVQSGAEVKKPGSSVKVSCKTSGDTFSTAAISWVRQAPGQGLEWMGGIIPIFGKAHYAQKFQGRVTITADESTSTAYMELSSLRSEDTAVYFCARKFHFVSGSPFGMDVWGQGTTVTVSSAKTTAPSVYPLAPVCGDTTGSSVTLGCLVKGYFPEPVTLTWNSGSLSSGVHTFPAVLQSDLYTLSSSVTVTSSTWPSQSITCNVAHPASSTKVDKKIEPRGPTIKPCPPCKCPAPNAAGGPCVFIFPPKIKDVLMISLSPIVTCVVVDVSEDDPDVQISWFVNNVEVHTAQTQTHREDYNSTLRVVSALPIQHQDWMSGKEFKCKVNNKDLPAPIERTISKPKGSVRAPQVYVLPPPEEEMTKKQVTLTCMVTDFMPEDIYVEWTNNGKTELNYKNTEPVLDSDGSYFMYSKLRVEKKNWVERNSYSCSVVHEGLHNHHTTKSFSRTPG

SEQ ID NO: 13 - protein, 5 aa, synthetic construct
TAAIS

SEQ ID NO: 14 - protein, 17 aa, synthetic construct
GIIPIFGKAHYAQKFQG

SEQ ID NO: 15 - protein, 14 aa, synthetic construct
KFHFVSGSPFGMDV

SEQ ID NO: 16 - protein, 11 aa, synthetic construct
RASQSVSSYLA

SEQ ID NO: 17 - protein, 7 aa, synthetic construct
DASNRAT

SEQ ID NO: 18 - protein, 8 aa, synthetic construct
QQRSNWPT

SEQ ID NO: 19 - protein, 123 aa, synthetic construct
QVQLVQSGAEVKKPGSSVKVSCKTSGDTFSTAAISWVRQAPGQGLEWMGGIIPIFGKAHYAQKFQGRVTITADESTSTAYMELSSLRSEDTAVYFCARKFHFVSGSPFGMDVWGQGTTVTVSS

SEQ ID NO: 20 - protein, 106 aa, synthetic construct
EIVLTQSPATLSLSPGERATLSCRASQSVSSYLAWYQQKPGQAPRLLIYDASNRATGIPARFSGSGSGTDFTLTISSLEPEDFAVYYCQQRSNWPTFGQGTKVEIK

SEQ ID NO: 21 - protein, 5 aa, synthetic construct
HYMMA

SEQ ID NO: 22 - protein, 17 aa, synthetic construct
RIGPSGGPTHYADSVKG

SEQ ID NO: 23 - protein, 19 aa, synthetic construct
YDSGYDYVAVAGPAEYFQH

SEQ ID NO: 24 - protein, 11 aa, synthetic construct
RASQSISTWLA

SEQ ID NO: 25 - protein, 7 aa, synthetic construct
KASNLHT

SEQ ID NO: 26 - protein, 9 aa, synthetic construct
QQYNSYSRT

SEQ ID NO: 27 - protein, 128 aa, synthetic construct
EVQLLESGGGLVQPGGSLRLSCAASGFTFSHYMMAWVRQAPGKGLEWVSRIGPSGGPTHYADSVKGRFTISRDNSKNTLYLQMNSLRAEDTAVYYCAGYDSGYDYVAVAGPAEYFQHWGQGTLVTVSS

SEQ ID NO: 28 - protein, 107 aa, synthetic construct
DIQMTQSPSSLSASVGDRVTITCRASQSISTWLAWYQQKPGKAPKLLIYKASNLHTGVPSRFSGSGSGTEFSLTISGLQPDDFATYYCQQYNSYSRTFGQGTKVEIK

SEQ ID NO: 29 - protein, 458 aa, synthetic construct
EVQLLESGGGLVQPGGSLRLSCAASGFTFSHYMMAWVRQAPGKGLEWVSRIGPSGGPTHYADSVKGRFTISRDNSKNTLYLQMNSLRAEDTAVYYCAGYDSGYDYVAVAGPAEYFQHWGQGTLVTVSSASTKGPSVFPLAPSSKSTSGGTAALGCLVKDYFPEPVTVSWNSGALTSGVHTFPAVLQSSGLYSLSSVVTVPSSSLGTQTYICNVNHKPSNTKVDKKVEPKSCDKTHTCPPCPAPELLGGPSVFLFPPKPKDTLMISRTPEVTCVVVDVSHEDPEVKFNWYVDGVEVHNAKTKPREEQYNSTYRVVSVLTVLHQDWLNGKEYKCKVSNKALPAPIEKTISKAKGQPREPQVYTLPPSRDELTKNQVSLTCLVKGFYPSDIAVEWESNGQPENNYKTTPPVLDSDGSFFLYSKLTVDKSRWQQGNVFSCSVMHEALHNHYTQKSLSLSPGK

SEQ ID NO: 30 - protein, 457 aa, synthetic construct
EVQLLESGGGLVQPGGSLRLSCAASGFTFSHYMMAWVRQAPGKGLEWVSRIGPSGGPTHYADSVKGRFTISRDNSKNTLYLQMNSLRAEDTAVYYCAGYDSGYDYVAVAGPAEYFQHWGQGTLVTVSSASTKGPSVFPLAPSSKSTSGGTAALGCLVKDYFPEPVTVSWNSGALTSGVHTFPAVLQSSGLYSLSSVVTVPSSSLGTQTYICNVNHKPSNTKVDKKVEPKSCDKTHTCPPCPAPELLGGPSVFLFPPKPKDTLMISRTPEVTCVVVDVSHEDPEVKFNWYVDGVEVHNAKTKPREEQYNSTYRVVSVLTVLHQDWLNGKEYKCKVSNKALPAPIEKTISKAKGQPREPQVYTLPPSRDELTKNQVSLTCLVKGFYPSDIAVEWESNGQPENNYKTTPPVLDSDGSFFLYSKLTVDKSRWQQGNVFSCSVMHEALHNHYTQKSLSLSPG

SEQ ID NO: 31 - protein, 214 aa, synthetic construct
DIQMTQSPSSLSASVGDRVTITCRASQSISTWLAWYQQKPGKAPKLLIYKASNLHTGVPSRFSGSGSGTEFSLTISGLQPDDFATYYCQQYNSYSRTFGQGTKVEIKRTVAAPSVFIFPPSDEQLKSGTASVVCLLNNFYPREAKVQWKVDNALQSGNSQESVTEQDSKDSTYSLSSTLTLSKADYEKHKVYACEVTHQGLSSPVTKSFNRGEC

SEQ ID NO: 32 - protein, 458 aa, synthetic construct
EVQLLESGGGLVQPGGSLRLSCAASGFTFSHYMMAWVRQAPGKGLEWVSRIGPSGGPTHYADSVKGRFTISRDNSKNTLYLQMNSLRAEDTAVYYCAGYDSGYDYVAVAGPAEYFQHWGQGTLVTVSSAKTTAPSVYPLAPVCGDTTGSSVTLGCLVKGYFPEPVTLTWNSGSLSSGVHTFPAVLQSDLYTLSSSVTVTSSTWPSQSITCNVAHPASSTKVDKKIEPRGPTIKPCPPCKCPAPNLLGGPSVFIFPPKIKDVLMISLSPIVTCVVVDVSEDDPDVQISWFVNNVEVHTAQTQTHREDYNSTLRVVSALPIQHQDWMSGKEFKCKVNNKDLPAPIERTISKPKGSVRAPQVYVLPPPEEEMTKKQVTLTCMVTDFMPEDIYVEWTNNGKTELNYKNTEPVLDSDGSYFMYSKLRVEKKNWVERNSYSCSVVHEGLHNHHTTKSFSRTPGK

SEQ ID NO: 33 - protein, 457 aa, synthetic construct
EVQLLESGGGLVQPGGSLRLSCAASGFTFSHYMMAWVRQAPGKGLEWVSRIGPSGGPTHYADSVKGRFTISRDNSKNTLYLQMNSLRAEDTAVYYCAGYDSGYDYVAVAGPAEYFQHWGQGTLVTVSSAKTTAPSVYPLAPVCGDTTGSSVTLGCLVKGYFPEPVTLTWNSGSLSSGVHTFPAVLQSDLYTLSSSVTVTSSTWPSQSITCNVAHPASSTKVDKKIEPRGPTIKPCPPCKCPAPNLLGGPSVFIFPPKIKDVLMISLSPIVTCVVVDVSEDDPDVQISWFVNNVEVHTAQTQTHREDYNSTLRVVSALPIQHQDWMSGKEFKCKVNNKDLPAPIERTISKPKGSVRAPQVYVLPPPEEEMTKKQVTLTCMVTDFMPEDIYVEWTNNGKTELNYKNTEPVLDSDGSYFMYSKLRVEKKNWVERNSYSCSVVHEGLHNHHTTKSFSRTPG

SEQ ID NO: 34 - protein, 214 aa, synthetic construct
DIQMTQSPSSLSASVGDRVTITCRASQSISTWLAWYQQKPGKAPKLLIYKASNLHTGVPSRFSGSGSGTEFSLTISGLQPDDFATYYCQQYNSYSRTFGQGTKVEIKRADAAPTVSIFPPSSEQLTSGGASVVCFLNNFYPKDINVKWKIDGSERQNGVLNSWTDQDSKDSTYSMSSTLTLTKDEYERHNSYTCEATHKTSTSPIVKSFNRNEC

SEQ ID NO: 35 - protein, 458 aa, synthetic construct
EVQLLESGGGLVQPGGSLRLSCAASGFTFSHYMMAWVRQAPGKGLEWVSRIGPSGGPTHYADSVKGRFTISRDNSKNTLYLQMNSLRAEDTAVYYCAGYDSGYDYVAVAGPAEYFQHWGQGTLVTVSSAKTTAPSVYPLAPVCGDTTGSSVTLGCLVKGYFPEPVTLTWNSGSLSSGVHTFPAVLQSDLYTLSSSVTVTSSTWPSQSITCNVAHPASSTKVDKKIEPRGPTIKPCPPCKCPAPNAAGGPSVFIFPPKIKDVLMISLSPIVTCVVVDVSEDDPDVQISWFVNNVEVHTAQTQTHREDYNSTLRVVSALPIQHQDWMSGKEFKCKVNNKDLGAPIERTISKPKGSVRAPQVYVLPPPEEEMTKKQVTLTCMVTDFMPEDIYVEWTNNGKTELNYKNTEPVLDSDGSYFMYSKLRVEKKNWVERNSYSCSVVHEGLHNHHTTKSFSRTPGK

SEQ ID NO: 36 - protein, 457 aa, synthetic construct
EVQLLESGGGLVQPGGSLRLSCAASGFTFSHYMMAWVRQAPGKGLEWVSRIGPSGGPTHYADSVKGRFTISRDNSKNTLYLQMNSLRAEDTAVYYCAGYDSGYDYVAVAGPAEYFQHWGQGTLVTVSSAKTTAPSVYPLAPVCGDTTGSSVTLGCLVKGYFPEPVTLTWNSGSLSSGVHTFPAVLQSDLYTLSSSVTVTSSTWPSQSITCNVAHPASSTKVDKKIEPRGPTIKPCPPCKCPAPNAAGGPSVFIFPPKIKDVLMISLSPIVTCVVVDVSEDDPDVQISWFVNNVEVHTAQTQTHREDYNSTLRVVSALPIQHQDWMSGKEFKCKVNNKDLGAPIERTISKPKGSVRAPQVYVLPPPEEEMTKKQVTLTCMVTDFMPEDIYVEWTNNGKTELNYKNTEPVLDSDGSYFMYSKLRVEKKNWVERNSYSCSVVHEGLHNHHTTKSFSRTPG

SEQ ID NO: 37 - protein, 214 aa, synthetic construct; identical to SEQ ID NO: 34

SEQ ID NO: 38 - protein, 5 aa, synthetic construct
DYYIT

SEQ ID NO: 39 - protein, 17 aa, synthetic construct
WIYPGSGNTKYNEKFKG

SEQ ID NO: 40 - protein, 8 aa, synthetic construct
YGNYWFAY

SEQ ID NO: 41 - protein, 15 aa, synthetic construct
KASQSVDFDGDSYMN

SEQ ID NO: 42 - protein, 7 aa, synthetic construct
AASNLES

SEQ ID NO: 43 - protein, 9 aa, synthetic construct
QQSNEDPWT

SEQ ID NO: 44 - protein, 117 aa, synthetic construct
QIQLQQSGPEVVKPGASVKISCKASGYTFTDYYITWVKQKPGQGLEWIGWIYPGSGNTKYNEKFKGKATLTVDTSSSTAFMQLSSLTSEDTAVYFCANYGNYWFAYWGQGTQVTVSA

SEQ ID NO: 45 - protein, 111 aa, synthetic construct
DIVLTQSPASLAVSLGQRATISCKASQSVDFDGDSYMNWYQQKPGQPPKVLIYAASNLESGIPARFSGSGSGTDFTLNIHPVEEEDAATYYCQQSNEDPWTFGGGTKLEIK

SEQ ID NO: 46 - protein, 447 aa, synthetic construct
QIQLQQSGPEVVKPGASVKISCKASGYTFTDYYITWVKQKPGQGLEWIGWIYPGSGNTKYNEKFKGKATLTVDTSSSTAFMQLSSLTSEDTAVYFCANYGNYWFAYWGQGTQVTVSAASTKGPSVFPLAPSSKSTSGGTAALGCLVKDYFPEPVTVSWNSGALTSGVHTFPAVLQSSGLYSLSSVVTVPSSSLGTQTYICNVNHKPSNTKVDKKVEPKSCDKTHTCPPCPAPELLGGPSVFLFPPKPKDTLMISRTPEVTCVVVDVSHEDPEVKFNWYVDGVEVHNAKTKPREEQYNSTYRVVSVLTVLHQDWLNGKEYKCKVSNKALPAPIEKTISKAKGQPREPQVYTLPPSRDELTKNQVSLTCLVKGFYPSDIAVEWESNGQPENNYKTTPPVLDSDGSFFLYSKLTVDKSRWQQGNVFSCSVMHEALHNHYTQKSLSLSPGK

SEQ ID NO: 47 - protein, 446 aa, synthetic construct
QIQLQQSGPEVVKPGASVKISCKASGYTFTDYYITWVKQKPGQGLEWIGWIYPGSGNTKYNEKFKGKATLTVDTSSSTAFMQLSSLTSEDTAVYFCANYGNYWFAYWGQGTQVTVSAASTKGPSVFPLAPSSKSTSGGTAALGCLVKDYFPEPVTVSWNSGALTSGVHTFPAVLQSSGLYSLSSVVTVPSSSLGTQTYICNVNHKPSNTKVDKKVEPKSCDKTHTCPPCPAPELLGGPSVFLFPPKPKDTLMISRTPEVTCVVVDVSHEDPEVKFNWYVDGVEVHNAKTKPREEQYNSTYRVVSVLTVLHQDWLNGKEYKCKVSNKALPAPIEKTISKAKGQPREPQVYTLPPSRDELTKNQVSLTCLVKGFYPSDIAVEWESNGQPENNYKTTPPVLDSDGSFFLYSKLTVDKSRWQQGNVFSCSVMHEALHNHYTQKSLSLSPG

SEQ ID NO: 48 - protein, 218 aa, synthetic construct
DIVLTQSPASLAVSLGQRATISCKASQSVDFDGDSYMNWYQQKPGQPPKVLIYAASNLESGIPARFSGSGSGTDFTLNIHPVEEEDAATYYCQQSNEDPWTFGGGTKLEIKRTVAAPSVFIFPPSDEQLKSGTASVVCLLNNFYPREAKVQWKVDNALQSGNSQESVTEQDSKDSTYSLSSTLTLSKADYEKHKVYACEVTHQGLSSPVTKSFNRGEC

SEQ ID NO: 49 - protein, 5 aa, synthetic construct
SGYWN

SEQ ID NO: 50 - protein, 16 aa, synthetic construct
YISDSGITYYNPSLKS

SEQ ID NO: 51 - protein, 11 aa, synthetic construct
RTLATYYAMDY

SEQ ID NO: 52 - protein, 16 aa, synthetic construct
RASQSLVHSDGNTYLH

SEQ ID NO: 53 - protein, 7 aa, synthetic construct
RVSNRFS

SEQ ID NO: 54 - protein, 9 aa, synthetic construct
SQSTHVPPT

SEQ ID NO: 55 - protein, 119 aa, synthetic construct
QVQLQESGPGLVKPSETLSLTCTVSGDSITSGYWNWIRQPPGKGLEYIGYISDSGITYYNPSLKSRVTISRDTSKNQYSLKLSSVTAADTAVYYCARRTLATYYAMDYWGQGTLVTVSS

SEQ ID NO: 56 - protein, 112 aa, synthetic construct
DFVMTQSPLSLPVTLGQPASISCRASQSLVHSDGNTYLHWYQQRPGQSPRLLIYRVSNRFSGVPDRFSGSGSGTDFTLKISRVEAEDVGVYYCSQSTHVPPTFGQGTKLEIK

SEQ ID NO: 57 - protein, 449 aa, synthetic construct
QVQLQESGPGLVKPSETLSLTCTVSGDSITSGYWNWIRQPPGKGLEYIGYISDSGITYYNPSLKSRVTISRDTSKNQYSLKLSSVTAADTAVYYCARRTLATYYAMDYWGQGTLVTVSSASTKGPSVFPLAPSSKSTSGGTAALGCLVKDYFPEPVTVSWNSGALTSGVHTFPAVLQSSGLYSLSSVVTVPSSSLGTQTYICNVNHKPSNTKVDKKVEPKSCDKTHTCPPCPAPELLGGPSVFLFPPKPKDTLMISRTPEVTCVVVDVSHEDPEVKFNWYVDGVEVHNAKTKPREEQYNSTYRVVSVLTVLHQDWLNGKEYKCKVSNKALPAPIEKTISKAKGQPREPQVYTLPPSRDELTKNQVSLTCLVKGFYPSDIAVEWESNGQPENNYKTTPPVLDSDGSFFLYSKLTVDKSRWQQGNVFSCSVMHEALHNHYTQKSLSLSPGK

SEQ ID NO: 58 - protein, 448 aa, synthetic construct
QVQLQESGPGLVKPSETLSLTCTVSGDSITSGYWNWIRQPPGKGLEYIGYISDSGITYYNPSLKSRVTISRDTSKNQYSLKLSSVTAADTAVYYCARRTLATYYAMDYWGQGTLVTVSSASTKGPSVFPLAPSSKSTSGGTAALGCLVKDYFPEPVTVSWNSGALTSGVHTFPAVLQSSGLYSLSSVVTVPSSSLGTQTYICNVNHKPSNTKVDKKVEPKSCDKTHTCPPCPAPELLGGPSVFLFPPKPKDTLMISRTPEVTCVVVDVSHEDPEVKFNWYVDGVEVHNAKTKPREEQYNSTYRVVSVLTVLHQDWLNGKEYKCKVSNKALPAPIEKTISKAKGQPREPQVYTLPPSRDELTKNQVSLTCLVKGFYPSDIAVEWESNGQPENNYKTTPPVLDSDGSFFLYSKLTVDKSRWQQGNVFSCSVMHEALHNHYTQKSLSLSPG

SEQ ID NO: 59 - protein, 219 aa, synthetic construct
DFVMTQSPLSLPVTLGQPASISCRASQSLVHSDGNTYLHWYQQRPGQSPRLLIYRVSNRFSGVPDRFSGSGSGTDFTLKISRVEAEDVGVYYCSQSTHVPPTFGQGTKLEIKRTVAAPSVFIFPPSDEQLKSGTASVVCLLNNFYPREAKVQWKVDNALQSGNSQESVTEQDSKDSTYSLSSTLTLSKADYEKHKVYACEVTHQGLSSPVTKSFNRGEC

SEQ ID NO: 60 - protein, 449 aa, synthetic construct
QVQLQESGPGLVKPSETLSLTCTVSGDSITSGYWNWIRQPPGKGLEYIGYISDSGITYYNPSLKSRVTISRDTSKNQYSLKLSSVTAADTAVYYCARRTLATYYAMDYWGQGTLVTVSSASTKGPSVFPLAPSSKSTSGGTAALGCLVKDYFPEPVTVSWNSGALTSGVHTFPAVLQSSGLYSLSSVVTVPSSSLGTQTYICNVNHKPSNTKVDKKVEPKSCDKTHTCPPCPAPEAAGGPSVFLFPPKPKDTLMISRTPEVTCVVVDVSHEDPEVKFNWYVDGVEVHNAKTKPREEQYNSTYRVVSVLTVLHQDWLNGKEYKCAVSNKALPAPIEKTISKAKGQPREPQVYTLPPSRDELTKNQVSLTCLVKGFYPSDIAVEWESNGQPENNYKTTPPVLDSDGSFFLYSKLTVDKSRWQQGNVFSCSVMHEALHNHYTQKSLSLSPGK

SEQ ID NO: 61 - protein, 448 aa, synthetic construct
QVQLQESGPGLVKPSETLSLTCTVSGDSITSGYWNWIRQPPGKGLEYIGYISDSGITYYNPSLKSRVTISRDTSKNQYSLKLSSVTAADTAVYYCARRTLATYYAMDYWGQGTLVTVSSASTKGPSVFPLAPSSKSTSGGTAALGCLVKDYFPEPVTVSWNSGALTSGVHTFPAVLQSSGLYSLSSVVTVPSSSLGTQTYICNVNHKPSNTKVDKKVEPKSCDKTHTCPPCPAPEAAGGPSVFLFPPKPKDTLMISRTPEVTCVVVDVSHEDPEVKFNWYVDGVEVHNAKTKPREEQYNSTYRVVSVLTVLHQDWLNGKEYKCAVSNKALPAPIEKTISKAKGQPREPQVYTLPPSRDELTKNQVSLTCLVKGFYPSDIAVEWESNGQPENNYKTTPPVLDSDGSFFLYSKLTVDKSRWQQGNVFSCSVMHEALHNHYTQKSLSLSPG

SEQ ID NO: 62 - protein, 219 aa, synthetic construct; identical to SEQ ID NO: 59

SEQ ID NO: 63 - protein, 5 aa, synthetic construct
DYNVN

SEQ ID NO: 64 - protein, 17 aa, synthetic construct
VINPKYGTTRYNQKFKG

SEQ ID NO: 65 - protein, 7 aa, synthetic construct
GLNAWDY

SEQ ID NO: 66 - protein, 11 aa, synthetic construct
GASENIYGALN

SEQ ID NO: 67 - protein, 7 aa, synthetic construct
GATNLED

SEQ ID NO: 68 - protein, 9 aa, synthetic construct
QNVLTTPYT

SEQ ID NO: 69 - protein, 116 aa, synthetic construct
QFQLVQSGAEVKKPGASVKVSCKASGYSFTDYNVNWVRQAPGQGLEWIGVINPKYGTTRYNQKFKGRATLTVDKSTSTAYMELSSLRSEDTAVYYCTRGLNAWDYWGQGTLVTVSS

SEQ ID NO: 70 - protein, 107 aa, synthetic construct
DIQMTQSPSSLSASVGDRVTITCGASENIYGALNWYQQKPGKAPKLLIYGATNLEDGVPSRFSGSGSGRDYTFTISSLQPEDIATYYCQNVLTTPYTFGQGTKLEIK

SEQ ID NO: 71 - protein, 446 aa, synthetic construct
QFQLVQSGAEVKKPGASVKVSCKASGYSFTDYNVNWVRQAPGQGLEWIGVINPKYGTTRYNQKFKGRATLTVDKSTSTAYMELSSLRSEDTAVYYCTRGLNAWDYWGQGTLVTVSSASTKGPSVFPLAPSSKSTSGGTAALGCLVKDYFPEPVTVSWNSGALTSGVHTFPAVLQSSGLYSLSSVVTVPSSSLGTQTYICNVNHKPSNTKVDKKVEPKSCDKTHTCPPCPAPELLGGPSVFLFPPKPKDTLMISRTPEVTCVVVDVSHEDPEVKFNWYVDGVEVHNAKTKPREEQYNSTYRVVSVLTVLHQDWLNGKEYKCKVSNKALPAPIEKTISKAKGQPREPQVYTLPPSRDELTKNQVSLTCLVKGFYPSDIAVEWESNGQPENNYKTTPPVLDSDGSFFLYSKLTVDKSRWQQGNVFSCSVMHEALHNHYTQKSLSLSPGK

SEQ ID NO: 72 - protein, 445 aa, synthetic construct
QFQLVQSGAEVKKPGASVKVSCKASGYSFTDYNVNWVRQAPGQGLEWIGVINPKYGTTRYNQKFKGRATLTVDKSTSTAYMELSSLRSEDTAVYYCTRGLNAWDYWGQGTLVTVSSASTKGPSVFPLAPSSKSTSGGTAALGCLVKDYFPEPVTVSWNSGALTSGVHTFPAVLQSSGLYSLSSVVTVPSSSLGTQTYICNVNHKPSNTKVDKKVEPKSCDKTHTCPPCPAPELLGGPSVFLFPPKPKDTLMISRTPEVTCVVVDVSHEDPEVKFNWYVDGVEVHNAKTKPREEQYNSTYRVVSVLTVLHQDWLNGKEYKCKVSNKALPAPIEKTISKAKGQPREPQVYTLPPSRDELTKNQVSLTCLVKGFYPSDIAVEWESNGQPENNYKTTPPVLDSDGSFFLYSKLTVDKSRWQQGNVFSCSVMHEALHNHYTQKSLSLSPG

SEQ ID NO: 73 - protein, 214 aa, synthetic construct
DIQMTQSPSSLSASVGDRVTITCGASENIYGALNWYQQKPGKAPKLLIYGATNLEDGVPSRFSGSGSGRDYTFTISSLQPEDIATYYCQNVLTTPYTFGQGTKLEIKRTVAAPSVFIFPPSDEQLKSGTASVVCLLNNFYPREAKVQWKVDNALQSGNSQESVTEQDSKDSTYSLSSTLTLSKADYEKHKVYACEVTHQGLSSPVTKSFNRGEC

SEQ ID NO: 74 - protein, 446 aa, synthetic construct
QFQLVQSGAEVKKPGASVKVSCKASGYSFTDYNVNWVRQAPGQGLEWIGVINPKYGTTRYNQKFKGRATLTVDKSTSTAYMELSSLRSEDTAVYYCTRGLNAWDYWGQGTLVTVSSASTKGPSVFPLAPSSKSTSGGTAALGCLVKDYFPEPVTVSWNSGALTSGVHTFPAVLQSSGLYSLSSVVTVPSSSLGTQTYICNVNHKPSNTKVDKKVEPKSCDKTHTCPPCPAPEAAGGPSVFLFPPKPKDTLMISRTPEVTCVVVDVSHEDPEVKFNWYVDGVEVHNAKTKPREEQYNSTYRVVSVLTVLHQDWLNGKEYKCAVSNKALPAPIEKTISKAKGQPREPQVYTLPPSRDELTKNQVSLTCLVKGFYPSDIAVEWESNGQPENNYKTTPPVLDSDGSFFLYSKLTVDKSRWQQGNVFSCSVMHEALHNHYTQKSLSLSPGK

SEQ ID NO: 75 - protein, 445 aa, synthetic construct
QFQLVQSGAEVKKPGASVKVSCKASGYSFTDYNVNWVRQAPGQGLEWIGVINPKYGTTRYNQKFKGRATLTVDKSTSTAYMELSSLRSEDTAVYYCTRGLNAWDYWGQGTLVTVSSASTKGPSVFPLAPSSKSTSGGTAALGCLVKDYFPEPVTVSWNSGALTSGVHTFPAVLQSSGLYSLSSVVTVPSSSLGTQTYICNVNHKPSNTKVDKKVEPKSCDKTHTCPPCPAPEAAGGPSVFLFPPKPKDTLMISRTPEVTCVVVDVSHEDPEVKFNWYVDGVEVHNAKTKPREEQYNSTYRVVSVLTVLHQDWLNGKEYKCAVSNKALPAPIEKTISKAKGQPREPQVYTLPPSRDELTKNQVSLTCLVKGFYPSDIAVEWESNGQPENNYKTTPPVLDSDGSFFLYSKLTVDKSRWQQGNVFSCSVMHEALHNHYTQKSLSLSPG

SEQ ID NO: 76 - protein, 214 aa, synthetic construct; identical to SEQ ID NO: 73

SEQ ID NO: 77 - protein, 7 aa, synthetic construct
SGSYYWG

SEQ ID NO: 78 - protein, 16 aa, synthetic construct
NIYYSGSTYYNPSLRS

SEQ ID NO: 79 - protein, 10 aa, synthetic construct
EGSYPNQFDP

SEQ ID NO: 80 - protein, 11 aa, synthetic construct
RASQSVSSNLA

SEQ ID NO: 81 - protein, 7 aa, synthetic construct
GASTRAT

SEQ ID NO: 82 - protein, 9 aa, synthetic construct
QQYHSFPFT

SEQ ID NO: 83 - protein, 120 aa, synthetic construct
QLQLQESGPGLVKPSETLSLTCTVSGGSIKSGSYYWGWIRQPPGKGLEWIGNIYYSGSTYYNPSLRSRVTISVDTSKNQFSLKLSSVTAADTAVYYCAREGSYPNQFDPWGQGTLVTVSS

SEQ ID NO: 84 - protein, 107 aa, synthetic construct
EIVMTQSPATLSVSPGERATLSCRASQSVSSNLAWYQQKPGQAPRLLIYGASTRATGIPARFSGSGSGTEFTLTISSLQSEDFAVYYCQQYHSFPFTFGGGTKVEIK

SEQ ID NO: 85 - protein, 450 aa, synthetic construct
QLQLQESGPGLVKPSETLSLTCTVSGGSIKSGSYYWGWIRQPPGKGLEWIGNIYYSGSTYYNPSLRSRVTISVDTSKNQFSLKLSSVTAADTAVYYCAREGSYPNQFDPWGQGTLVTVSSASTKGPSVFPLAPSSKSTSGGTAALGCLVKDYFPEPVTVSWNSGALTSGVHTFPAVLQSSGLYSLSSVVTVPSSSLGTQTYICNVNHKPSNTKVDKKVEPKSCDKTHTCPPCPAPELLGGPSVFLFPPKPKDTLMISRTPEVTCVVVDVSHEDPEVKFNWYVDGVEVHNAKTKPREEQYNSTYRVVSVLTVLHQDWLNGKEYKCKVSNKALPAPIEKTISKAKGQPREPQVYTLPPSRDELTKNQVSLTCLVKGFYPSDIAVEWESNGQPENNYKTTPPVLDSDGSFFLYSKLTVDKSRWQQGNVFSCSVMHEALHNHYTQKSLSLSPGK

SEQ ID NO: 86 - protein, 449 aa, synthetic construct
QLQLQESGPGLVKPSETLSLTCTVSGGSIKSGSYYWGWIRQPPGKGLEWIGNIYYSGSTYYNPSLRSRVTISVDTSKNQFSLKLSSVTAADTAVYYCAREGSYPNQFDPWGQGTLVTVSSASTKGPSVFPLAPSSKSTSGGTAALGCLVKDYFPEPVTVSWNSGALTSGVHTFPAVLQSSGLYSLSSVVTVPSSSLGTQTYICNVNHKPSNTKVDKKVEPKSCDKTHTCPPCPAPELLGGPSVFLFPPKPKDTLMISRTPEVTCVVVDVSHEDPEVKFNWYVDGVEVHNAKTKPREEQYNSTYRVVSVLTVLHQDWLNGKEYKCKVSNKALPAPIEKTISKAKGQPREPQVYTLPPSRDELTKNQVSLTCLVKGFYPSDIAVEWESNGQPENNYKTTPPVLDSDGSFFLYSKLTVDKSRWQQGNVFSCSVMHEALHNHYTQKSLSLSPG

SEQ ID NO: 87 - protein, 214 aa, synthetic construct
EIVMTQSPATLSVSPGERATLSCRASQSVSSNLAWYQQKPGQAPRLLIYGASTRATGIPARFSGSGSGTEFTLTISSLQSEDFAVYYCQQYHSFPFTFGGGTKVEIKRTVAAPSVFIFPPSDEQLKSGTASVVCLLNNFYPREAKVQWKVDNALQSGNSQESVTEQDSKDSTYSLSSTLTLSKADYEKHKVYACEVTHQGLSSPVTKSFNRGEC

SEQ ID NO: 88 - protein, 450 aa, synthetic construct
QLQLQESGPGLVKPSETLSLTCTVSGGSIKSGSYYWGWIRQPPGKGLEWIGNIYYSGSTYYNPSLRSRVTISVDTSKNQFSLKLSSVTAADTAVYYCAREGSYPNQFDPWGQGTLVTVSSASTKGPSVFPLAPSSKSTSGGTAALGCLVKDYFPEPVTVSWNSGALTSGVHTFPAVLQSSGLYSLSSVVTVPSSSLGTQTYICNVNHKPSNTKVDKKVEPKSCDKTHTCPPCPAPEAAGGPSVFLFPPKPKDTLMISRTPEVTCVVVDVSHEDPEVKFNWYVDGVEVHNAKTKPREEQYNSTYRVVSVLTVLHQDWLNGKEYKCAVSNKALPAPIEKTISKAKGQPREPQVYTLPPSRDELTKNQVSLTCLVKGFYPSDIAVEWESNGQPENNYKTTPPVLDSDGSFFLYSKLTVDKSRWQQGNVFSCSVMHEALHNHYTQKSLSLSPGK

SEQ ID NO: 89 - protein, 449 aa, synthetic construct
QLQLQESGPGLVKPSETLSLTCTVSGGSIKSGSYYWGWIRQPPGKGLEWIGNIYYSGSTYYNPSLRSRVTISVDTSKNQFSLKLSSVTAADTAVYYCAREGSYPNQFDPWGQGTLVTVSSASTKGPSVFPLAPSSKSTSGGTAALGCLVKDYFPEPVTVSWNSGALTSGVHTFPAVLQSSGLYSLSSVVTVPSSSLGTQTYICNVNHKPSNTKVDKKVEPKSCDKTHTCPPCPAPEAAGGPSVFLFPPKPKDTLMISRTPEVTCVVVDVSHEDPEVKFNWYVDGVEVHNAKTKPREEQYNSTYRVVSVLTVLHQDWLNGKEYKCAVSNKALPAPIEKTISKAKGQPREPQVYTLPPSRDELTKNQVSLTCLVKGFYPSDIAVEWESNGQPENNYKTTPPVLDSDGSFFLYSKLTVDKSRWQQGNVFSCSVMHEALHNHYTQKSLSLSPG

SEQ ID NO: 90 - protein, 214 aa, synthetic construct; identical to SEQ ID NO: 87

SEQ ID NO: 91 - protein, 11 aa, synthetic construct
GSISSSSYYWG

SEQ ID NO: 92 - protein, 16 aa, synthetic construct
NIYYSGSTYYNPSLKS

SEQ ID NO: 93 - protein, 12 aa, synthetic construct
AREGSYPNWFDP

SEQ ID NO: 94 - protein, 11 aa, synthetic construct
RASQSVSSNLA

SEQ ID NO: 95 - protein, 7 aa, synthetic construct
GASTRAT

SEQ ID NO: 96 - protein, 9 aa, synthetic construct
QQYHSFPFT

SEQ ID NO: 97 - protein, 120 aa, synthetic construct
QLQLQESGPGLVKPSETLSLTCTVSGGSISSSSYYWGWIRQPPGKGLEWIGNIYYSGSTYYNPSLKSRVTISVDTSKNQFSLKLSSVTAADTAVYYCAREGSYPNWFDPWGQGTLVTVSS

SEQ ID NO: 98 - protein, 107 aa, synthetic construct; identical to SEQ ID NO: 84

SEQ ID NO: 99 - protein, 11 aa, synthetic construct
GSIKSGSHYWG

SEQ ID NO: 100 - protein, 16 aa, synthetic construct
NIYYSGSTYYNPSLRS

SEQ ID NO: 101 - protein, 12 aa, synthetic construct
AREGSYPNWFDP

SEQ ID NO: 102 - protein, 11 aa, synthetic construct
RASQSVSSNLA

SEQ ID NO: 103 - protein, 7 aa, synthetic construct
GASTRAT

SEQ ID NO: 104 - protein, 9 aa, synthetic construct
QQYHSFPFT

SEQ ID NO: 105 - protein, 120 aa, synthetic construct
QLQLQESGPGLVKPSETLSLTCTVSGGSIKSGSHYWGWIRQPPGKGLEWIGNIYYSGSTYYNPSLRSRVTISVDTSKNQFSLKLSSVTAADTAVYYCAREGSYPNWFDPWGQGTLVTVSS

SEQ ID NO: 106 - protein, 107 aa, synthetic construct; identical to SEQ ID NO: 84

SEQ ID NO: 107 - protein, 11 aa, synthetic construct
GSIKSGSHYWG

SEQ ID NO: 108 - protein, 16 aa, synthetic construct
NIYYSGSTYYNPSLKS

SEQ ID NO: 109 - protein, 12 aa, synthetic construct
AREGSYPNWLDP

SEQ ID NO: 110 - protein, 11 aa, synthetic construct
RASQSVSSNLA

SEQ ID NO: 111 - protein, 7 aa, synthetic construct
GASTRAT

SEQ ID NO: 112 - protein, 9 aa, synthetic construct
QQYHSFPFT

SEQ ID NO: 113 - protein, 120 aa, synthetic construct
QLQLQESGPGLVKPSETLSLTCTVSGGSIKSGSHYWGWIRQPPGKGLEWIGNIYYSGSTYYNPSLKSRVTISVDTSKNQFSLKLSSVTAADTAVYYCAREGSYPNWLDPWGQGTLVTVSS

SEQ ID NO: 114 - protein, 107 aa, synthetic construct; identical to SEQ ID NO: 84

SEQ ID NO: 115 - protein, 11 aa, synthetic construct
GSIKSGSYYWG

SEQ ID NO: 116 - protein, 16 aa, synthetic construct
NIYYSGSTYYNPSLKS

SEQ ID NO: 117 - protein, 12 aa, synthetic construct
AREGSYPNQFDP

SEQ ID NO: 118 - protein, 11 aa, synthetic construct
RASQSVSSNLA

SEQ ID NO: 119 - protein, 7 aa, synthetic construct
GASTRAT

SEQ ID NO: 120 - protein, 9 aa, synthetic construct
QQYHSFPFT

SEQ ID NO: 121 - protein, 120 aa, synthetic construct
QLQLQESGPGLVKPSETLSLTCTVSGGSIKSGSYYWGWIRQPPGKGLEWIGNIYYSGSTYYNPSLKSRVTISVDTSKNQFSLKLSSVTAADTAVYYCAREGSYPNQFDPWGQGILVTVSS

SEQ ID NO: 122 - protein, 107 aa, synthetic construct; identical to SEQ ID NO: 84

SEQ ID NO: 123 - protein, 11 aa, synthetic construct
GSIKSGSHYWG

SEQ ID NO: 124 - protein, 16 aa, synthetic construct
NIYYSGSTYYNPSLKS

SEQ ID NO: 125 - protein, 12 aa, synthetic construct
AREGSYPNWFDP

SEQ ID NO: 126 - protein, 11 aa, synthetic construct
RASQSVSTNLA

SEQ ID NO: 127 - protein, 7 aa, synthetic construct
DASARVT

SEQ ID NO: 128 - protein, 9 aa, synthetic construct
QQYHSFPFT

SEQ ID NO: 129 - protein, 120 aa, synthetic construct
QLQLQESGPGLVKPSETLSLTCTVSGGSIKSGSHYWGWIRQPPGKGLEWIGNIYYSGSTYYNPSLKSRVTMSVDTSKNQFSLKLSSVTAADTAVYYCAREGSYPNWFDPWGQGTLVTVSS

SEQ ID NO: 130 - protein, 107 aa, synthetic construct
EIVMTQSPATLSVSPGERATLSCRASQSVSTNLAWYQQKPGQAPRLLIYDASARVTGIPARFSGSGSGTEFTLTISSLQSEDFAVYYCQQYHSFPFTFGGGTKVEIK

SEQ ID NO: 131 - protein, 11 aa, synthetic construct
GSISSSSYYWG

SEQ ID NO: 132 - protein, 16 aa, synthetic construct
NIYYSGSTYYNPSLKS

SEQ ID NO: 133 - protein, 12 aa, synthetic construct
AREGSYTTVLNV

SEQ ID NO: 134 - protein, 12 aa, synthetic construct
RASQSVSSSYLA

SEQ ID NO: 135 - protein, 7 aa, synthetic construct
GASSRAT

SEQ ID NO: 136 - protein, 9 aa, synthetic construct
QQAASYPLT

SEQ ID NO: 137 - protein, 120 aa, synthetic construct
QLQLQESGPGLVKPSETLSLTCTVSGGSISSSSYYWGWIRQPPGKGLEWIGNIYYSGSTYYNPSLKSRVTISVDTSKNQFSLKLSSVTAADTAVYYCAREGSYTTVLNVWGQGTMVTVSS

SEQ ID NO: 138 - protein, 108 aa, synthetic construct
EIVLTQSPGTLSLSPGERATLSCRASQSVSSSYLAWYQQKPGQAPRLLIYGASSRATGIPDRFSGSGSGTDFTLTISRLEPEDFAVYYCQQAASYPLTFGGGTKVEIK

SEQ ID NO: 139 - protein, 11 aa, synthetic construct
GSIGRGSYYWG

SEQ ID NO: 140 - protein, 16 aa, synthetic construct
NIYYSGSTYYNPSLKS

SEQ ID NO: 141 - protein, 12 aa, synthetic construct
AREGSYTTVLNV

SEQ ID NO: 142 - protein, 12 aa, synthetic construct
RASQSVASSHLA

SEQ ID NO: 143 - protein, 7 aa, synthetic construct
DAVSRAT

SEQ ID NO: 144 - protein, 9 aa, synthetic construct
QQAASYPLT

SEQ ID NO: 145 - protein, 120 aa, synthetic construct
QLQLQESGPGLVKPSETLSLTCTVSGGSIGRGSYYWGWIRQPPGKGLEWIGNIYYSGSTYYNPSLKSRVTISVDTSKNQFSLKLSSVTAADTAVYYCAREGSYTTVLNVWGQGTMVTVSS

SEQ ID NO: 146 - protein, 108 aa, synthetic construct
EIVLTQSPGTLSLSPGERATLSCRASQSVASSHLAWYQQKPGQAPRLLIYDAVSRATGIPDRFSGSGSGTDFTLTISRLEPEDFAVYYCQQAASYPLTFGGGTKVEIK

SEQ ID NO: 147 - protein, 11 aa, synthetic construct
GSISSGGYYWS

SEQ ID NO: 148 - protein, 16 aa, synthetic construct
NIYYSGSTYYNPSLKS

SEQ ID NO: 149 - protein, 13 aa, synthetic construct
ARESSTISADFDL

SEQ ID NO: 150 - protein, 11 aa, synthetic construct
RASQGISRWLA

SEQ ID NO: 151 - protein, 7 aa, synthetic construct
AASSLQS

SEQ ID NO: 152 - protein, 9 aa, synthetic construct
QQAHTFPYT

SEQ ID NO: 153 - protein, 121 aa, synthetic construct
QVQLQESGPGLVKPSQTLSLTCTVSGGSISSGGYYWSWIRQHPGKGLEWIGNIYYSGSTYYNPSLKSRVTISVDTSKNQFSLKLSSVTAADTAVYYCARESSTISADFDLWGRGTLVTVSS

SEQ ID NO: 154 - protein, 107 aa, synthetic construct
DIQMTQSPSSVSASVGDRVTITCRASQGISRWLAWYQQKPGKAPKLLIYAASSLQSGVPSRFSGSGSGTDFTLTISSLQPEDFATYYCQQAHTFPYTFGGGTKVEIK

SEQ ID NO: 155 - protein, 11 aa, synthetic construct
GSISHGGYYWS

SEQ ID NO: 156 - protein, 16 aa, synthetic construct
NIYYSGSTYYNPSLKS

SEQ ID NO: 157 - protein, 13 aa, synthetic construct
ARESSTISADFDL

SEQ ID NO: 158 - protein, 11 aa, synthetic construct
RASQGISRWLA

SEQ ID NO: 159 - protein, 7 aa, synthetic construct
AASSLQS

SEQ ID NO: 160 - protein, 9 aa, synthetic construct
QQAHTFPYT

SEQ ID NO: 161 - protein, 121 aa, synthetic construct
QLQLQESGPGLVKPSETLSLTCTASGGSISHGGYYWSWIRQHPGKGLEWIGNIYYSGSTYYNPSLKSRVTMSVDTSKNQFSLKLSSVTAADTAVYYCARESSTISADFDLWGRGTLVTVSS

SEQ ID NO: 162 - protein, 107 aa, synthetic construct; identical to SEQ ID NO: 154

SEQ ID NO: 163 - protein, 11 aa, synthetic construct
GSISSGGYYWS

SEQ ID NO: 164 - protein, 16 aa, synthetic construct
NIYYSGSTYYNPSLKS

SEQ ID NO: 165 - protein, 13 aa, synthetic construct
ARGLSTIDEAFDP

SEQ ID NO: 166 - protein, 11 aa, synthetic construct
RASQSISSWLA

SEQ ID NO: 167 - protein, 7 aa, synthetic construct
KASSLES

SEQ ID NO: 168 - protein, 9 aa, synthetic construct
QQDNSYPYT

SEQ ID NO: 169 - protein, 121 aa, synthetic construct
QVQLQESGPGLVKPSQTLSLTCTVSGGSISSGGYYWSWIRQHPGKGLEWIGNIYYSGSTYYNPSLKSRVTISVDTSKNQFSLKLSSVTAADTAVYYCARGLSTIDEAFDPWGQGTLVTVSS

SEQ ID NO: 170 - protein, 107 aa, synthetic construct
DIQMTQSPSTLSASVGDRVTITCRASQSISSWLAWYQQKPGKAPKLLIYKASSLESGVPSRFSGSGSGTEFTLTISSLQPDDFATYYCQQDNSYPYTFGGGTKVEIK

SEQ ID NO: 171 - protein, 11 aa, synthetic construct
GSISDGSYYWS

SEQ ID NO: 172 - protein, 16 aa, synthetic construct
NIYYSGSTYYNPSLRS

SEQ ID NO: 173 - protein, 13 aa, synthetic construct
ARGLSTIDEAFDP

SEQ ID NO: 174 - protein, 11 aa, synthetic construct
RASQSISSWLA

SEQ ID NO: 175 - protein, 7 aa, synthetic construct
KASSLES

SEQ ID NO: 176 - protein, 9 aa, synthetic construct
QQDNSYPYT

SEQ ID NO: 177 - protein, 121 aa, synthetic construct
QLQLQESGPGLVKPSETLSLTCTVSGGSISDGSYYWSWIRQHPGKGLEWIGNIYYSGSTYYNPSLRSRVTMSVDTSKNQFSLKLSSVTAADTAVYYCARGLSTIDEAFDPWGQGTLVTVSS

SEQ ID NO: 178 - protein, 107 aa, synthetic construct; identical to SEQ ID NO: 170

SEQ ID NO: 179 - protein, 11 aa, synthetic construct
GSISDGSYYWS

SEQ ID NO: 180 - protein, 16 aa, synthetic construct
NIYYSGSTYYNPSLRS

SEQ ID NO: 181 - protein, 13 aa, synthetic construct
ARGLSTIDEAFDP

SEQ ID NO: 182 - protein, 11 aa, synthetic construct
RASKSISSWLA

SEQ ID NO: 183 - protein, 7 aa, synthetic construct
EASSLHS

SEQ ID NO: 184 - protein, 9 aa, synthetic construct
QQDNSYPYT

SEQ ID NO: 185 - protein, 121 aa, synthetic construct
QVQLQESGPGLVKPSQTLSLTCTVSGGSISDGSYYWSWIRQHPGKGLEWIGNIYYSGSTYYNPSLRSRVTMSVDTSKNQFSLKLSSVTAADTAVYYCARGLSTIDEAFDPWGQGTLVTVSS

SEQ ID NO: 186 - protein, 107 aa, synthetic construct
DIQMTQSPSTLSASVGDRVTITCRASKSISSWLAWYQQKPGKAPKLLIYEASSLHSGVPSRFSGSGSGTEFTLTISSLQPDDFATYYCQQDNSYPYTFGGGTKVEIK

SEQ ID NO: 187 - protein, 9 aa, synthetic construct
GSISSYYWS

SEQ ID NO: 188 - protein, 16 aa, synthetic construct
YIYSSGSTNYNPSLKS

SEQ ID NO: 189 - protein, 15 aa, synthetic construct
ARGSGQYAAPDYGMD

SEQ ID NO: 190 - protein, 11 aa, synthetic construct
RASQSISSWLA

SEQ ID NO: 191 - protein, 7 aa, synthetic construct
KASSLES

SEQ ID NO: 192 - protein, 9 aa, synthetic construct
QQDNSFPFT

SEQ ID NO: 193 - protein, 122 aa, synthetic construct
QVQLQESGPGLVKPSETLSLTCTVSGGSISSYYWSWIRQPPGKGLEWIGYIYSSGSTNYNPSLKSRVTISVDTSKNQFSLKLSSVTAADTAVYYCARGSGQYAAPDYGMDVWGQGTTVTVSS

SEQ ID NO: 194 - protein, 107 aa, synthetic construct
DIQMTQSPSTLSASVGDRVTITCRASQSISSWLAWYQQKPGKAPKLLIYKASSLESGVPSRFSGSGSGTEFTLTISSLQPDDFATYYCQQDNSFPFTFGGGTKVEIK

SEQ ID NO: 195 - protein, 9 aa, synthetic construct
GSIISYYWG

SEQ ID NO: 196 - protein, 16 aa, synthetic construct
YIYSSGSTSYNPSLKS

SEQ ID NO: 197 - protein, 16 aa, synthetic construct
ARGSGLYAAPDYGLDV

SEQ ID NO: 198 - protein, 11 aa, synthetic construct
RASQSISSWLA

SEQ ID NO: 199 - protein, 7 aa, synthetic construct
KASSLES

SEQ ID NO: 200 - protein, 9 aa, synthetic construct
QQDNSFPFT

SEQ ID NO: 201 - protein, 122 aa, synthetic construct
QVQLQESGPGLVKPSETLSLTCTVSGGSIISYYWGWIRQPPGKGLEWIGYIYSSGSTSYNPSLKSRVTISVDTSKNQFSLKLSSVTAADTAVYYCARGSGLYAAPDYGLDVWGQGTTVTVSS

SEQ ID NO: 202 - protein, 107 aa, synthetic construct; identical to SEQ ID NO: 194

SEQ ID NO: 203 - protein, 9 aa, synthetic construct
FTFSSYAMS

SEQ ID NO: 204 - protein, 17 aa, synthetic construct
TISGSGGSTYYADSVKG

SEQ ID NO: 205 - protein, 13 aa, synthetic construct
ARGAGHYDLVGRY

SEQ ID NO: 206 - protein, 11 aa, synthetic construct
RASQSISSYLN

SEQ ID NO: 207 - protein, 7 aa, synthetic construct
AASSLQS

SEQ ID NO: 208 - protein, 9 aa, synthetic construct
QQLYSLPPT

SEQ ID NO: 209 - protein, 120 aa, synthetic construct
EVQLLESGGGLVQPGGSLRLSCAASGFTFSSYAMSWVRQAPGKGLEWVSTISGSGGSTYYADSVKGRFTISRDNSKNTLYLQMNSLRAEDTAVYYCARGAGHYDLVGRYWGQGTLVTVSS

SEQ ID NO: 210 - protein, 107 aa, synthetic construct
DIQMTQSPSSLSASVGDRVTITCRASQSISSYLNWYQQKPGKAPKLLIYAASSLQSGVPSRFSGSGSGTDFTLTISSLQPEDFATYYCQQLYSLPPTFGGGTKVEIK

SEQ ID NO: 211 - protein, 9 aa, synthetic construct
FTFSSYAMS

SEQ ID NO: 212 - protein, 17 aa, synthetic construct
AISGSGGSTYYADSVKG

SEQ ID NO: 213 - protein, 10 aa, synthetic construct
ARVGFRALNY

SEQ ID NO: 214 - protein, 11 aa, synthetic construct
RASQDISSWLA

SEQ ID NO: 215 - protein, 7 aa, synthetic construct
AASSLQS

SEQ ID NO: 216 - protein, 10 aa, synthetic construct
QQATSYPPWT

SEQ ID NO: 217 - protein, 117 aa, synthetic construct
EVQLLESGGGLVQPGGSLRLSCAASGFTFSSYAMSWVRQAPGKGLEWVSAISGSGGSTYYADSVKGRFTISRDNSKNTLYLQMNSLRAEDTAVYYCARVGFRALNYWGQGTTVTVSS

SEQ ID NO: 218 - protein, 108 aa, synthetic construct
DIQLTQSPSSVSASVGDRVTITCRASQDISSWLAWYQQKPGKAPKLLIYAASSLQSGVPSRFSGSGSGTDFTLTISSLQPEDFATYYCQQATSYPPWTFGGGTKVEIK

SEQ ID NO: 219 - protein, 9 aa, synthetic construct
GTFSSYAIS

SEQ ID NO: 220 - protein, 17 aa, synthetic construct
GIIPIFGTASYAQKFQG

SEQ ID NO: 221 - protein, 13 aa, synthetic construct
ARQQYDGRRYFGL

SEQ ID NO: 222 - protein, 11 aa, synthetic construct
RASQSVSSNLA

SEQ ID NO: 223 - protein, 7 aa, synthetic construct
SASTRAT

SEQ ID NO: 224 - protein, 9 aa, synthetic construct
QQVNVWPPT

SEQ ID NO: 225 - protein, 120 aa, synthetic construct
QVQLVQSGAEVKKPGSSVKVSCKASGGTFSSYAISWVRQAPGQGLEWMGGIIPIFGTASYAQKFQGRVTITADESTSTAYMELSSLRSEDTAVYYCARQQYDGRRYFGLWGRGTLVTVSS

SEQ ID NO: 226 - protein, 107 aa, synthetic construct
EIVMTQSPATLSVSPGERATLSCRASQSVSSNLAWYQQKPGQAPRLLIYSASTRATGIPARFSGSGSGTEFTLTISSLQSEDFAVYYCQQVNVWPPTFGGGTKVEIK

SEQ ID NO: 227 - protein, 9 aa, synthetic construct
GTFSSYAIS

SEQ ID NO: 228 - protein, 17 aa, synthetic construct
GIIPIFGTANYAQKFQG

SEQ ID NO: 229 - protein, 9 aa, synthetic construct
ARGGPWFDP

SEQ ID NO: 230 - protein, 11 aa, synthetic construct
RASQSISSWLA

SEQ ID NO: 231 - protein, 7 aa, synthetic construct
KASSLES

SEQ ID NO: 232 - protein, 10 aa, synthetic construct
QQYNSYPPFT

SEQ ID NO: 233 - protein, 116 aa, synthetic construct
QVQLVQSGAEVKKPGSSVKVSCKASGGTFSSYAISWVRQAPGQGLEWMGGIIPIFGTANYAQKFQGRVTITADESTSTAYMELSSLRSEDTAVYYCARGGPWFDPWGQGTLVTVSS

SEQ ID NO: 234 - protein, 108 aa, synthetic construct
DIQMTQSPSTLSASVGDRVTITCRASQSISSWLAWYQQKPGKAPKLLIYKASSLESGVPSRFSGSGSGTEFTLTISSLQPDDFATYYCQQYNSYPPFTFGGGTKVEIK

SEQ ID NO: 235 - protein, 9 aa, synthetic construct
FTFSSYAMS

SEQ ID NO: 236 - protein, 17 aa, synthetic construct
AISGSGGSTSYADSVKG

SEQ ID NO: 237 - protein, 13 aa, synthetic construct
AKPSLATMLAFDI

SEQ ID NO: 238 - protein, 11 aa, synthetic construct
RASQSISSWLA

SEQ ID NO: 239 - protein, 7 aa, synthetic construct
DASSLES

SEQ ID NO: 240 - protein, 9 aa, synthetic construct
QQSKSYPRT

SEQ ID NO: 241 - protein, 120 aa, synthetic construct
EVQLLESGGGLVQPGGSLRLSCAASGFTFSSYAMSWVRQAPGKGLEWVSAISGSGGSTSYADSVKGRFTISRDNSKNTLYLQMNSLRAEDTAVYYCAKPSLATMLAFDIWGQGTMVTVSS

SEQ ID NO: 242 - protein, 107 aa, synthetic construct
DIQMTQSPSTLSASVGDRVTITCRASQSISSWLAWYQQKPGKAPKLLIYDASSLESGVPSRFSGSGSGTEFTLTISSLQPDDFATYYCQQSKSYPRTFGGGTKVEIK

SEQ ID NO: 243 - protein, 11 aa, synthetic construct
GSISSSVYYWS

SEQ ID NO: 244 - protein, 16 aa, synthetic construct
SILVSGSTYYNPSLKS

SEQ ID NO: 245 - protein, 9 aa, synthetic construct
ARAVSFLDV

SEQ ID NO: 246 - protein, 11 aa, synthetic construct
RASQSISSYLN

SEQ ID NO: 247 - protein, 7 aa, synthetic construct
GASSLQS

SEQ ID NO: 248 - protein, 9 aa, synthetic construct
QQSYDPPWT

SEQ ID NO: 249 - protein, 117 aa, synthetic construct
QLQLQESGPGLVKPSETLSLTCTVSGGSISSSVYYWSWIRQPPGKGLEWIGSILVSGSTYYNPSLKSRVTISVDTSKNQFSLKLSSVTAADTAVYYCARAVSFLDVWGQGTMVIVSS

SEQ ID NO: 250 - protein, 107 aa, synthetic construct
DIQMTQSPSSLSASVGDRVTITCRASQSISSYLNWYQQKPGKAPKLLIYGASSLQSGVPSRFSGSGSGTDFTLTISSLQPEDFATYYCQQSYDPPWTFGGGTKVEIK

SEQ ID NO: 251 - protein, 450 aa, synthetic construct
QLQLQESGPGLVKPSETLSLTCTVSGGSISSSSYYWGWIRQPPGKGLEWIGNIYYSGSTYYNPSLKSRVTISVDTSKNQFSLKLSSVTAADTAVYYCAREGSYPNWFDPWGQGTLVTVSSASTKGPSVFPLAPSSKSTSGGTAALGCLVKDYFPEPVTVSWNSGALTSGVHTFPAVLQSSGLYSLSSVVTVPSSSLGTQTYICNVNHKPSNTKVDKKVEPKSCDKTHTCPPCPAPELLGGPSVFLFPPKPKDTLMISRTPEVTCVVVDVSHEDPEVKFNWYVDGVEVHNAKTKPREEQYNSTYRVVSVLTVLHQDWLNGKEYKCKVSNKALPAPIEKTISKAKGQPREPQVYTLPPSRDELTKNQVSLTCLVKGFYPSDIAVEWESNGQPENNYKTTPPVLDSDGSFFLYSKLTVDKSRWQQGNVFSCSVMHEALHNHYTQKSLSLSPGK

SEQ ID NO: 252 - protein, 214 aa, synthetic construct; identical to SEQ ID NO: 87

SEQ ID NO: 253 - protein, 450 aa, synthetic construct
QLQLQESGPGLVKPSETLSLTCTVSGGSIKSGSHYWGWIRQPPGKGLEWIGNIYYSGSTYYNPSLRSRVTISVDTSKNQFSLKLSSVTAADTAVYYCAREGSYPNWFDPWGQGTLVTVSSASTKGPSVFPLAPSSKSTSGGTAALGCLVKDYFPEPVTVSWNSGALTSGVHTFPAVLQSSGLYSLSSVVTVPSSSLGTQTYICNVNHKPSNTKVDKKVEPKSCDKTHTCPPCPAPELLGGPSVFLFPPKPKDTLMISRTPEVTCVVVDVSHEDPEVKFNWYVDGVEVHNAKTKPREEQYNSTYRVVSVLTVLHQDWLNGKEYKCKVSNKALPAPIEKTISKAKGQPREPQVYTLPPSRDELTKNQVSLTCLVKGFYPSDIAVEWESNGQPENNYKTTPPVLDSDGSFFLYSKLTVDKSRWQQGNVFSCSVMHEALHNHYTQKSLSLSPGK

SEQ ID NO: 254 - protein, 214 aa, synthetic construct; identical to SEQ ID NO: 87

SEQ ID NO: 255 - protein, 450 aa, synthetic construct
QLQLQESGPGLVKPSETLSLTCTVSGGSIKSGSHYWGWIRQPPGKGLEWIGNIYYSGSTYYNPSLKSRVTISVDTSKNQFSLKLSSVTAADTAVYYCAREGSYPNWLDPWGQGTLVTVSSASTKGPSVFPLAPSSKSTSGGTAALGCLVKDYFPEPVTVSWNSGALTSGVHTFPAVLQSSGLYSLSSVVTVPSSSLGTQTYICNVNHKPSNTKVDKKVEPKSCDKTHTCPPCPAPELLGGPSVFLFPPKPKDTLMISRTPEVTCVVVDVSHEDPEVKFNWYVDGVEVHNAKTKPREEQYNSTYRVVSVLTVLHQDWLNGKEYKCKVSNKALPAPIEKTISKAKGQPREPQVYTLPPSRDELTKNQVSLTCLVKGFYPSDIAVEWESNGQPENNYKTTPPVLDSDGSFFLYSKLTVDKSRWQQGNVFSCSVMHEALHNHYTQKSLSLSPGK

SEQ ID NO: 256 - protein, 214 aa, synthetic construct; identical to SEQ ID NO: 87

SEQ ID NO: 257 - protein, 450 aa, synthetic construct
QLQLQESGPGLVKPSETLSLTCTVSGGSIKSGSYYWGWIRQPPGKGLEWIGNIYYSGSTYYNPSLKSRVTISVDTSKNQFSLKLSSVTAADTAVYYCAREGSYPNQFDPWGQGILVTVSSASTKGPSVFPLAPSSKSTSGGTAALGCLVKDYFPEPVTVSWNSGALTSGVHTFPAVLQSSGLYSLSSVVTVPSSSLGTQTYICNVNHKPSNTKVDKKVEPKSCDKTHTCPPCPAPELLGGPSVFLFPPKPKDTLMISRTPEVTCVVVDVSHEDPEVKFNWYVDGVEVHNAKTKPREEQYNSTYRVVSVLTVLHQDWLNGKEYKCKVSNKALPAPIEKTISKAKGQPREPQVYTLPPSRDELTKNQVSLTCLVKGFYPSDIAVEWESNGQPENNYKTTPPVLDSDGSFFLYSKLTVDKSRWQQGNVFSCSVMHEALHNHYTQKSLSLSPGK

SEQ ID NO: 258 - protein, 214 aa, synthetic construct; identical to SEQ ID NO: 87

SEQ ID NO: 259 - protein, 450 aa, synthetic construct
QLQLQESGPGLVKPSETLSLTCTVSGGSIKSGSHYWGWIRQPPGKGLEWIGNIYYSGSTYYNPSLKSRVTMSVDTSKNQFSLKLSSVTAADTAVYYCAREGSYPNWFDPWGQGTLVTVSSASTKGPSVFPLAPSSKSTSGGTAALGCLVKDYFPEPVTVSWNSGALTSGVHTFPAVLQSSGLYSLSSVVTVPSSSLGTQTYICNVNHKPSNTKVDKKVEPKSCDKTHTCPPCPAPELLGGPSVFLFPPKPKDTLMISRTPEVTCVVVDVSHEDPEVKFNWYVDGVEVHNAKTKPREEQYNSTYRVVSVLTVLHQDWLNGKEYKCKVSNKALPAPIEKTISKAKGQPREPQVYTLPPSRDELTKNQVSLTCLVKGFYPSDIAVEWESNGQPENNYKTTPPVLDSDGSFFLYSKLTVDKSRWQQGNVFSCSVMHEALHNHYTQKSLSLSPGK

SEQ ID NO: 260 - protein, 214 aa, synthetic construct
EIVMTQSPATLSVSPGERATLSCRASQSVSTNLAWYQQKPGQAPRLLIYDASARVTGIPARFSGSGSGTEFTLTISSLQSEDFAVYYCQQYHSFPFTFGGGTKVEIKRTVAAPSVFIFPPSDEQLKSGTASVVCLLNNFYPREAKVQWKVDNALQSGNSQESVTEQDSKDSTYSLSSTLTLSKADYEKHKVYACEVTHQGLSSPVTKSFNRGEC

SEQ ID NO: 261 - protein, 450 aa, synthetic construct
QLQLQESGPGLVKPSETLSLTCTVSGGSISSSSYYWGWIRQPPGKGLEWIGNIYYSGSTYYNPSLKSRVTISVDTSKNQFSLKLSSVTAADTAVYYCAREGSYTTVLNVWGQGTMVTVSSASTKGPSVFPLAPSSKSTSGGTAALGCLVKDYFPEPVTVSWNSGALTSGVHTFPAVLQSSGLYSLSSVVTVPSSSLGTQTYICNVNHKPSNTKVDKKVEPKSCDKTHTCPPCPAPELLGGPSVFLFPPKPKDTLMISRTPEVTCVVVDVSHEDPEVKFNWYVDGVEVHNAKTKPREEQYNSTYRVVSVLTVLHQDWLNGKEYKCKVSNKALPAPIEKTISKAKGQPREPQVYTLPPSRDELTKNQVSLTCLVKGFYPSDIAVEWESNGQPENNYKTTPPVLDSDGSFFLYSKLTVDKSRWQQGNVFSCSVMHEALHNHYTQKSLSLSPGK

SEQ ID NO: 262 - protein, 215 aa, synthetic construct
EIVLTQSPGTLSLSPGERATLSCRASQSVSSSYLAWYQQKPGQAPRLLIYGASSRATGIPDRFSGSGSGTDFTLTISRLEPEDFAVYYCQQAASYPLTFGGGTKVEIKRTVAAPSVFIFPPSDEQLKSGTASVVCLLNNFYPREAKVQWKVDNALQSGNSQESVTEQDSKDSTYSLSSTLTLSKADYEKHKVYACEVTHQGLSSPVTKSFNRGEC

SEQ ID NO: 263 - protein, 450 aa, synthetic construct
QLQLQESGPGLVKPSETLSLTCTVSGGSIGRGSYYWGWIRQPPGKGLEWIGNIYYSGSTYYNPSLKSRVTISVDTSKNQFSLKLSSVTAADTAVYYCAREGSYTTVLNVWGQGTMVTVSSASTKGPSVFPLAPSSKSTSGGTAALGCLVKDYFPEPVTVSWNSGALTSGVHTFPAVLQSSGLYSLSSVVTVPSSSLGTQTYICNVNHKPSNTKVDKKVEPKSCDKTHTCPPCPAPELLGGPSVFLFPPKPKDTLMISRTPEVTCVVVDVSHEDPEVKFNWYVDGVEVHNAKTKPREEQYNSTYRVVSVLTVLHQDWLNGKEYKCKVSNKALPAPIEKTISKAKGQPREPQVYTLPPSRDELTKNQVSLTCLVKGFYPSDIAVEWESNGQPENNYKTTPPVLDSDGSFFLYSKLTVDKSRWQQGNVFSCSVMHEALHNHYTQKSLSLSPGK

SEQ ID NO: 264 - protein, 215 aa, synthetic construct
EIVLTQSPGTLSLSPGERATLSCRASQSVASSHLAWYQQKPGQAPRLLIYDAVSRATGIPDRFSGSGSGTDFTLTISRLEPEDFAVYYCQQAASYPLTFGGGTKVEIKRTVAAPSVFIFPPSDEQLKSGTASVVCLLNNFYPREAKVQWKVDNALQSGNSQESVTEQDSKDSTYSLSSTLTLSKADYEKHKVYACEVTHQGLSSPVTKSFNRGEC

SEQ ID NO: 265 - protein, 451 aa, synthetic construct
QVQLQESGPGLVKPSQTLSLTCTVSGGSISSGGYYWSWIRQHPGKGLEWIGNIYYSGSTYYNPSLKSRVTISVDTSKNQFSLKLSSVTAADTAVYYCARESSTISADFDLWGRGTLVTVSSASTKGPSVFPLAPSSKSTSGGTAALGCLVKDYFPEPVTVSWNSGALTSGVHTFPAVLQSSGLYSLSSVVTVPSSSLGTQTYICNVNHKPSNTKVDKKVEPKSCDKTHTCPPCPAPELLGGPSVFLFPPKPKDTLMISRTPEVTCVVVDVSHEDPEVKFNWYVDGVEVHNAKTKPREEQYNSTYRVVSVLTVLHQDWLNGKEYKCKVSNKALPAPIEKTISKAKGQPREPQVYTLPPSRDELTKNQVSLTCLVKGFYPSDIAVEWESNGQPENNYKTTPPVLDSDGSFFLYSKLTVDKSRWQQGNVFSCSVMHEALHNHYTQKSLSLSPGK

SEQ ID NO: 266 - protein, 214 aa, synthetic construct
DIQMTQSPSSVSASVGDRVTITCRASQGISRWLAWYQQKPGKAPKLLIYAASSLQSGVPSRFSGSGSGTDFTLTISSLQPEDFATYYCQQAHTFPYTFGGGTKVEIKRTVAAPSVFIFPPSDEQLKSGTASVVCLLNNFYPREAKVQWKVDNALQSGNSQESVTEQDSKDSTYSLSSTLTLSKADYEKHKVYACEVTHQGLSSPVTKSFNRGEC

SEQ ID NO: 267 - protein, 451 aa, synthetic construct
QLQLQESGPGLVKPSETLSLTCTASGGSISHGGYYWSWIRQHPGKGLEWIGNIYYSGSTYYNPSLKSRVTMSVDTSKNQFSLKLSSVTAADTAVYYCARESSTISADFDLWGRGTLVTVSSASTKGPSVFPLAPSSKSTSGGTAALGCLVKDYFPEPVTVSWNSGALTSGVHTFPAVLQSSGLYSLSSVVTVPSSSLGTQTYICNVNHKPSNTKVDKKVEPKSCDKTHTCPPCPAPELLGGPSVFLFPPKPKDTLMISRTPEVTCVVVDVSHEDPEVKFNWYVDGVEVHNAKTKPREEQYNSTYRVVSVLTVLHQDWLNGKEYKCKVSNKALPAPIEKTISKAKGQPREPQVYTLPPSRDELTKNQVSLTCLVKGFYPSDIAVEWESNGQPENNYKTTPPVLDSDGSFFLYSKLTVDKSRWQQGNVFSCSVMHEALHNHYTQKSLSLSPGK

SEQ ID NO: 268 - protein, 214 aa, synthetic construct; identical to SEQ ID NO: 266

SEQ ID NO: 269 - protein, 451 aa, synthetic construct
QVQLQESGPGLVKPSQTLSLTCTVSGGSISSGGYYWSWIRQHPGKGLEWIGNIYYSGSTYYNPSLKSRVTISVDTSKNQFSLKLSSVTAADTAVYYCARGLSTIDEAFDPWGQGTLVTVSSASTKGPSVFPLAPSSKSTSGGTAALGCLVKDYFPEPVTVSWNSGALTSGVHTFPAVLQSSGLYSLSSVVTVPSSSLGTQTYICNVNHKPSNTKVDKKVEPKSCDKTHTCPPCPAPELLGGPSVFLFPPKPKDTLMISRTPEVTCVVVDVSHEDPEVKFNWYVDGVEVHNAKTKPREEQYNSTYRVVSVLTVLHQDWLNGKEYKCKVSNKALPAPIEKTISKAKGQPREPQVYTLPPSRDELTKNQVSLTCLVKGFYPSDIAVEWESNGQPENNYKTTPPVLDSDGSFFLYSKLTVDKSRWQQGNVFSCSVMHEALHNHYTQKSLSLSPGK

SEQ ID NO: 270 - protein, 214 aa, synthetic construct
DIQMTQSPSTLSASVGDRVTITCRASQSISSWLAWYQQKPGKAPKLLIYKASSLESGVPSRFSGSGSGTEFTLTISSLQPDDFATYYCQQDNSYPYTFGGGTKVEIKRTVAAPSVFIFPPSDEQLKSGTASVVCLLNNFYPREAKVQWKVDNALQSGNSQESVTEQDSKDSTYSLSSTLTLSKADYEKHKVYACEVTHQGLSSPVTKSFNRGEC

SEQ ID NO: 271 - protein, 451 aa, synthetic construct
QLQLQESGPGLVKPSETLSLTCTVSGGSISDGSYYWSWIRQHPGKGLEWIGNIYYSGSTYYNPSLRSRVTMSVDTSKNQFSLKLSSVTAADTAVYYCARGLSTIDEAFDPWGQGTLVTVSSASTKGPSVFPLAPSSKSTSGGTAALGCLVKDYFPEPVTVSWNSGALTSGVHTFPAVLQSSGLYSLSSVVTVPSSSLGTQTYICNVNHKPSNTKVDKKVEPKSCDKTHTCPPCPAPELLGGPSVFLFPPKPKDTLMISRTPEVTCVVVDVSHEDPEVKFNWYVDGVEVHNAKTKPREEQYNSTYRVVSVLTVLHQDWLNGKEYKCKVSNKALPAPIEKTISKAKGQPREPQVYTLPPSRDELTKNQVSLTCLVKGFYPSDIAVEWESNGQPENNYKTTPPVLDSDGSFFLYSKLTVDKSRWQQGNVFSCSVMHEALHNHYTQKSLSLSPGK

SEQ ID NO: 272 - protein, 214 aa, synthetic construct; identical to SEQ ID NO: 270

SEQ ID NO: 273 - protein, 451 aa, synthetic construct
QVQLQESGPGLVKPSQTLSLTCTVSGGSISDGSYYWSWIRQHPGKGLEWIGNIYYSGSTYYNPSLRSRVTMSVDTSKNQFSLKLSSVTAADTAVYYCARGLSTIDEAFDPWGQGTLVTVSSASTKGPSVFPLAPSSKSTSGGTAALGCLVKDYFPEPVTVSWNSGALTSGVHTFPAVLQSSGLYSLSSVVTVPSSSLGTQTYICNVNHKPSNTKVDKKVEPKSCDKTHTCPPCPAPELLGGPSVFLFPPKPKDTLMISRTPEVTCVVVDVSHEDPEVKFNWYVDGVEVHNAKTKPREEQYNSTYRVVSVLTVLHQDWLNGKEYKCKVSNKALPAPIEKTISKAKGQPREPQVYTLPPSRDELTKNQVSLTCLVKGFYPSDIAVEWESNGQPENNYKTTPPVLDSDGSFFLYSKLTVDKSRWQQGNVFSCSVMHEALHNHYTQKSLSLSPGK

SEQ ID NO: 274 - protein, 214 aa, synthetic construct
DIQMTQSPSTLSASVGDRVTITCRASKSISSWLAWYQQKPGKAPKLLIYEASSLHSGVPSRFSGSGSGTEFTLTISSLQPDDFATYYCQQDNSYPYTFGGGTKVEIKRTVAAPSVFIFPPSDEQLKSGTASVVCLLNNFYPREAKVQWKVDNALQSGNSQESVTEQDSKDSTYSLSSTLTLSKADYEKHKVYACEVTHQGLSSPVTKSFNRGEC

SEQ ID NO: 275 - protein, 452 aa, synthetic construct
QVQLQESGPGLVKPSETLSLTCTVSGGSISSYYWSWIRQPPGKGLEWIGYIYSSGSTNYNPSLKSRVTISVDTSKNQFSLKLSSVTAADTAVYYCARGSGQYAAPDYGMDVWGQGTTVTVSSASTKGPSVFPLAPSSKSTSGGTAALGCLVKDYFPEPVTVSWNSGALTSGVHTFPAVLQSSGLYSLSSVVTVPSSSLGTQTYICNVNHKPSNTKVDKKVEPKSCDKTHTCPPCPAPELLGGPSVFLFPPKPKDTLMISRTPEVTCVVVDVSHEDPEVKFNWYVDGVEVHNAKTKPREEQYNSTYRVVSVLTVLHQDWLNGKEYKCKVSNKALPAPIEKTISKAKGQPREPQVYTLPPSRDELTKNQVSLTCLVKGFYPSDIAVEWESNGQPENNYKTTPPVLDSDGSFFLYSKLTVDKSRWQQGNVFSCSVMHEALHNHYTQKSLSLSPGK

SEQ ID NO: 276 - protein, 214 aa, synthetic construct
DIQMTQSPSTLSASVGDRVTITCRASQSISSWLAWYQQKPGKAPKLLIYKASSLESGVPSRFSGSGSGTEFTLTISSLQPDDFATYYCQQDNSFPFTFGGGTKVEIKRTVAAPSVFIFPPSDEQLKSGTASVVCLLNNFYPREAKVQWKVDNALQSGNSQESVTEQDSKDSTYSLSSTLTLSKADYEKHKVYACEVTHQGLSSPVTKSFNRGEC

SEQ ID NO: 277 - protein, 452 aa, synthetic construct
QVQLQESGPGLVKPSETLSLTCTVSGGSIISYYWGWIRQPPGKGLEWIGYIYSSGSTSYNPSLKSRVTISVDTSKNQFSLKLSSVTAADTAVYYCARGSGLYAAPDYGLDVWGQGTTVTVSSASTKGPSVFPLAPSSKSTSGGTAALGCLVKDYFPEPVTVSWNSGALTSGVHTFPAVLQSSGLYSLSSVVTVPSSSLGTQTYICNVNHKPSNTKVDKKVEPKSCDKTHTCPPCPAPELLGGPSVFLFPPKPKDTLMISRTPEVTCVVVDVSHEDPEVKFNWYVDGVEVHNAKTKPREEQYNSTYRVVSVLTVLHQDWLNGKEYKCKVSNKALPAPIEKTISKAKGQPREPQVYTLPPSRDELTKNQVSLTCLVKGFYPSDIAVEWESNGQPENNYKTTPPVLDSDGSFFLYSKLTVDKSRWQQGNVFSCSVMHEALHNHYTQKSLSLSPGK

SEQ ID NO: 278 - protein, 214 aa, synthetic construct; identical to SEQ ID NO: 276

SEQ ID NO: 279 - protein, 450 aa, synthetic construct
EVQLLESGGGLVQPGGSLRLSCAASGFTFSSYAMSWVRQAPGKGLEWVSTISGSGGSTYYADSVKGRFTISRDNSKNTLYLQMNSLRAEDTAVYYCARGAGHYDLVGRYWGQGTLVTVSSASTKGPSVFPLAPSSKSTSGGTAALGCLVKDYFPEPVTVSWNSGALTSGVHTFPAVLQSSGLYSLSSVVTVPSSSLGTQTYICNVNHKPSNTKVDKKVEPKSCDKTHTCPPCPAPELLGGPSVFLFPPKPKDTLMISRTPEVTCVVVDVSHEDPEVKFNWYVDGVEVHNAKTKPREEQYNSTYRVVSVLTVLHQDWLNGKEYKCKVSNKALPAPIEKTISKAKGQPREPQVYTLPPSRDELTKNQVSLTCLVKGFYPSDIAVEWESNGQPENNYKTTPPVLDSDGSFFLYSKLTVDKSRWQQGNVFSCSVMHEALHNHYTQKSLSLSPGK

SEQ ID NO: 280 - protein, 214 aa, synthetic construct
DIQMTQSPSSLSASVGDRVTITCRASQSISSYLNWYQQKPGKAPKLLIYAASSLQSGVPSRFSGSGSGTDFTLTISSLQPEDFATYYCQQLYSLPPTFGGGTKVEIKRTVAAPSVFIFPPSDEQLKSGTASVVCLLNNFYPREAKVQWKVDNALQSGNSQESVTEQDSKDSTYSLSSTLTLSKADYEKHKVYACEVTHQGLSSPVTKSFNRGEC

SEQ ID NO: 281 - protein, 447 aa, synthetic construct
EVQLLESGGGLVQPGGSLRLSCAASGFTFSSYAMSWVRQAPGKGLEWVSAISGSGGSTYYADSVKGRFTISRDNSKNTLYLQMNSLRAEDTAVYYCARVGFRALNYWGQGTTVTVSSASTKGPSVFPLAPSSKSTSGGTAALGCLVKDYFPEPVTVSWNSGALTSGVHTFPAVLQSSGLYSLSSVVTVPSSSLGTQTYICNVNHKPSNTKVDKKVEPKSCDKTHTCPPCPAPELLGGPSVFLFPPKPKDTLMISRTPEVTCVVVDVSHEDPEVKFNWYVDGVEVHNAKTKPREEQYNSTYRVVSVLTVLHQDWLNGKEYKCKVSNKALPAPIEKTISKAKGQPREPQVYTLPPSRDELTKNQVSLTCLVKGFYPSDIAVEWESNGQPENNYKTTPPVLDSDGSFFLYSKLTVDKSRWQQGNVFSCSVMHEALHNHYTQKSLSLSPGK

SEQ ID NO: 282 - protein, 215 aa, synthetic construct
DIQLTQSPSSVSASVGDRVTITCRASQDISSWLAWYQQKPGKAPKLLIYAASSLQSGVPSRFSGSGSGTDFTLTISSLQPEDFATYYCQQATSYPPWTFGGGTKVEIKRTVAAPSVFIFPPSDEQLKSGTASVVCLLNNFYPREAKVQWKVDNALQSGNSQESVTEQDSKDSTYSLSSTLTLSKADYEKHKVYACEVTHQGLSSPVTKSFNRGEC

SEQ ID NO: 283 - protein, 450 aa, synthetic construct
QVQLVQSGAEVKKPGSSVKVSCKASGGTFSSYAISWVRQAPGQGLEWMGGIIPIFGTASYAQKFQGRVTITADESTSTAYMELSSLRSEDTAVYYCARQQYDGRRYFGLWGRGTLVTVSSASTKGPSVFPLAPSSKSTSGGTAALGCLVKDYFPEPVTVSWNSGALTSGVHTFPAVLQSSGLYSLSSVVTVPSSSLGTQTYICNVNHKPSNTKVDKKVEPKSCDKTHTCPPCPAPELLGGPSVFLFPPKPKDTLMISRTPEVTCVVVDVSHEDPEVKFNWYVDGVEVHNAKTKPREEQYNSTYRVVSVLTVLHQDWLNGKEYKCKVSNKALPAPIEKTISKAKGQPREPQVYTLPPSRDELTKNQVSLTCLVKGFYPSDIAVEWESNGQPENNYKTTPPVLDSDGSFFLYSKLTVDKSRWQQGNVFSCSVMHEALHNHYTQKSLSLSPGK

SEQ ID NO: 284 - protein, 214 aa, synthetic construct
EIVMTQSPATLSVSPGERATLSCRASQSVSSNLAWYQQKPGQAPRLLIYSASTRATGIPARFSGSGSGTEFTLTISSLQSEDFAVYYCQQVNVWPPTFGGGTKVEIKRTVAAPSVFIFPPSDEQLKSGTASVVCLLNNFYPREAKVQWKVDNALQSGNSQESVTEQDSKDSTYSLSSTLTLSKADYEKHKVYACEVTHQGLSSPVTKSFNRGEC

SEQ ID NO: 285 - protein, 446 aa, synthetic construct
QVQLVQSGAEVKKPGSSVKVSCKASGGTFSSYAISWVRQAPGQGLEWMGGIIPIFGTANYAQKFQGRVTITADESTSTAYMELSSLRSEDTAVYYCARGGPWFDPWGQGTLVTVSSASTKGPSVFPLAPSSKSTSGGTAALGCLVKDYFPEPVTVSWNSGALTSGVHTFPAVLQSSGLYSLSSVVTVPSSSLGTQTYICNVNHKPSNTKVDKKVEPKSCDKTHTCPPCPAPELLGGPSVFLFPPKPKDTLMISRTPEVTCVVVDVSHEDPEVKFNWYVDGVEVHNAKTKPREEQYNSTYRVVSVLTVLHQDWLNGKEYKCKVSNKALPAPIEKTISKAKGQPREPQVYTLPPSRDELTKNQVSLTCLVKGFYPSDIAVEWESNGQPENNYKTTPPVLDSDGSFFLYSKLTVDKSRWQQGNVFSCSVMHEALHNHYTQKSLSLSPGK

SEQ ID NO: 286 - protein, 215 aa, synthetic construct
DIQMTQSPSTLSASVGDRVTITCRASQSISSWLAWYQQKPGKAPKLLIYKASSLESGVPSRFSGSGSGTEFTLTISSLQPDDFATYYCQQYNSYPPFTFGGGTKVEIKRTVAAPSVFIFPPSDEQLKSGTASVVCLLNNFYPREAKVQWKVDNALQSGNSQESVTEQDSKDSTYSLSSTLTLSKADYEKHKVYACEVTHQGLSSPVTKSFNRGEC

SEQ ID NO: 287 - protein, 450 aa, synthetic construct
EVQLLESGGGLVQPGGSLRLSCAASGFTFSSYAMSWVRQAPGKGLEWVSAISGSGGSTSYADSVKGRFTISRDNSKNTLYLQMNSLRAEDTAVYYCAKPSLATMLAFDIWGQGTMVTVSSASTKGPSVFPLAPSSKSTSGGTAALGCLVKDYFPEPVTVSWNSGALTSGVHTFPAVLQSSGLYSLSSVVTVPSSSLGTQTYICNVNHKPSNTKVDKKVEPKSCDKTHTCPPCPAPELLGGPSVFLFPPKPKDTLMISRTPEVTCVVVDVSHEDPEVKFNWYVDGVEVHNAKTKPREEQYNSTYRVVSVLTVLHQDWLNGKEYKCKVSNKALPAPIEKTISKAKGQPREPQVYTLPPSRDELTKNQVSLTCLVKGFYPSDIAVEWESNGQPENNYKTTPPVLDSDGSFFLYSKLTVDKSRWQQGNVFSCSVMHEALHNHYTQKSLSLSPGK

SEQ ID NO: 288 - protein, 214 aa, synthetic construct
DIQMTQSPSTLSASVGDRVTITCRASQSISSWLAWYQQKPGKAPKLLIYDASSLESGVPSRFSGSGSGTEFTLTISSLQPDDFATYYCQQSKSYPRTFGGGTKVEIKRTVAAPSVFIFPPSDEQLKSGTASVVCLLNNFYPREAKVQWKVDNALQSGNSQESVTEQDSKDSTYSLSSTLTLSKADYEKHKVYACEVTHQGLSSPVTKSFNRGEC

SEQ ID NO: 289 - protein, 447 aa, synthetic construct
QLQLQESGPGLVKPSETLSLTCTVSGGSISSSVYYWSWIRQPPGKGLEWIGSILVSGSTYYNPSLKSRVTISVDTSKNQFSLKLSSVTAADTAVYYCARAVSFLDVWGQGTMVIVSSASTKGPSVFPLAPSSKSTSGGTAALGCLVKDYFPEPVTVSWNSGALTSGVHTFPAVLQSSGLYSLSSVVTVPSSSLGTQTYICNVNHKPSNTKVDKKVEPKSCDKTHTCPPCPAPELLGGPSVFLFPPKPKDTLMISRTPEVTCVVVDVSHEDPEVKFNWYVDGVEVHNAKTKPREEQYNSTYRVVSVLTVLHQDWLNGKEYKCKVSNKALPAPIEKTISKAKGQPREPQVYTLPPSRDELTKNQVSLTCLVKGFYPSDIAVEWESNGQPENNYKTTPPVLDSDGSFFLYSKLTVDKSRWQQGNVFSCSVMHEALHNHYTQKSLSLSPGK

SEQ ID NO: 290 - protein, 214 aa, synthetic construct
DIQMTQSPSSLSASVGDRVTITCRASQSISSYLNWYQQKPGKAPKLLIYGASSLQSGVPSRFSGSGSGTDFTLTISSLQPEDFATYYCQQSYDPPWTFGGGTKVEIKRTVAAPSVFIFPPSDEQLKSGTASVVCLLNNFYPREAKVQWKVDNALQSGNSQESVTEQDSKDSTYSLSSTLTLSKADYEKHKVYACEVTHQGLSSPVTKSFNRGEC

SEQ ID NO: 291 - protein, 5 aa, synthetic construct
NYGMN

SEQ ID NO: 292 - protein, 17 aa, synthetic construct
WINTYTGEPTYADAFKG

SEQ ID NO: 293 - protein, 9 aa, synthetic construct
DYGDYGMDY

SEQ ID NO: 294 - protein, 15 aa, synthetic construct
RASKSVSTSGYSFMH

SEQ ID NO: 295 - protein, 7 aa, synthetic construct
LASNLES

SEQ ID NO: 296 - protein, 9 aa, synthetic construct
QHSREVPWT

SEQ ID NO: 297 - protein, 118 aa, synthetic construct
QVQLVQSGAEVKKPGASVKVSCKASGYTFTNYGMNWVRQAPGQGLKWMGWINTYTGEPTYADAFKGRVTMTRDTSISTAYMELSRLRSDDTAVYYCARDYGDYGMDYWGQGTTVTVSS

SEQ ID NO: 298 - protein, 111 aa, synthetic construct
DIVMTQSPDSLAVSLGERATINCRASKSVSTSGYSFMHWYQQKPGQPPKLLIYLASNLESGVPDRFSGSGSGTDFTLTISSLQAEDVAVYYCQHSREVPWTFGQGTKVEIK

SEQ ID NO: 299 - protein, 448 aa, synthetic construct
QVQLVQSGAEVKKPGASVKVSCKASGYTFTNYGMNWVRQAPGQGLKWMGWINTYTGEPTYADAFKGRVTMTRDTSISTAYMELSRLRSDDTAVYYCARDYGDYGMDYWGQGTTVTVSSASTKGPSVFPLAPSSKSTSGGTAALGCLVKDYFPEPVTVSWNSGALTSGVHTFPAVLQSSGLYSLSSVVTVPSSSLGTQTYICNVNHKPSNTKVDKKVEPKSCDKTHTCPPCPAPELLGGPSVFLFPPKPKDTLMISRTPEVTCVVVDVSHEDPEVKFNWYVDGVEVHNAKTKPREEQYNSTYRVVSVLTVLHQDWLNGKEYKCKVSNKALPAPIEKTISKAKGQPREPQVYTLPPSRDELTKNQVSLTCLVKGFYPSDIAVEWESNGQPENNYKTTPPVLDSDGSFFLYSKLTVDKSRWQQGNVFSCSVMHEALHNHYTQKSLSLSPGK

SEQ ID NO: 300 - protein, 218 aa, synthetic construct
DIVMTQSPDSLAVSLGERATINCRASKSVSTSGYSFMHWYQQKPGQPPKLLIYLASNLESGVPDRFSGSGSGTDFTLTISSLQAEDVAVYYCQHSREVPWTFGQGTKVEIKRTVAAPSVFIFPPSDEQLKSGTASVVCLLNNFYPREAKVQWKVDNALQSGNSQESVTEQDSKDSTYSLSSTLTLSKADYEKHKVYACEVTHQGLSSPVTKSFNRGEC

SEQ ID NO: 301 - protein, 5 aa, synthetic construct
NYGMN

SEQ ID NO: 302 - protein, 17 aa, synthetic construct
WINTYTGEPTYTDDFKG

SEQ ID NO: 303 - protein, 12 aa, synthetic construct
GGFGSSYWYFDV

SEQ ID NO: 304 - protein, 11 aa, synthetic construct
KASQDVSIAVA

SEQ ID NO: 305 - protein, 7 aa, synthetic construct
SASYRYT

SEQ ID NO: 306 - protein, 9 aa, synthetic construct
QQHYITPLT

SEQ ID NO: 307 - protein, 121 aa, synthetic construct
QVQLQQSGSELKKPGASVKVSCKASGYTFTNYGMNWVKQAPGQGLKWMGWINTYTGEPTYTDDFKGRFAFSLDTSVSTAYLQISSLKADDTAVYFCARGGFGSSYWYFDVWGQGSLVTVSS

SEQ ID NO: 308 - protein, 107 aa, synthetic construct
DIQLTQSPSSLSASVGDRVSITCKASQDVSIAVAWYQQKPGKAPKLLIYSASYRYTGVPDRFSGSGSGTDFTLTISSLQPEDFAVYYCQQHYITPLTFGAGTKVEIK

SEQ ID NO: 309 - protein, 5 aa, synthetic construct
TAGMQ

SEQ ID NO: 310 - protein, 17 aa, synthetic construct
WINTHSGVPKYAEDFKG

SEQ ID NO: 311 - protein, 12 aa, synthetic construct
SGFGSSYWYFDV

SEQ ID NO: 312 - protein, 11 aa, synthetic construct
KASQDVSTAVA

SEQ ID NO: 313 - protein, 7 aa, synthetic construct
SASYRYT

SEQ ID NO: 314 - protein, 9 aa, synthetic construct
QQHYITPLT

SEQ ID NO: 315 - protein, 121 aa, synthetic construct
QVQLVQSGAEVKKPGASVKVSCKASGYTFTTAGMQWVRQAPGQGLEWMGWINTHSGVPKYAEDFKGRVTISADTSTSTAYLQLSSLKSEDTAVYYCARSGFGSSYWYFDVWGQGTLVTVSS

SEQ ID NO: 316 - protein, 107 aa, synthetic construct
DIQMTQSPSSLSASVGDRVTITCKASQDVSTAVAWYQQKPGKAPKLLIYSASYRYTGVPSRFSGSGSGTDFTLTISSLQPEDFAVYYCQQHYITPLTFGQGTKLEIK

SEQ ID NO: 317 - protein, 5 aa, synthetic construct
SQNIY

SEQ ID NO: 318 - protein, 17 aa, synthetic construct
YIEPYNVVPMYNPKFKG

SEQ ID NO: 319 - protein, 8 aa, synthetic construct
SGSSNFDY

SEQ ID NO: 320 - protein, 12 aa, synthetic construct
SASSSISSHYLH

SEQ ID NO: 321 - protein, 7 aa, synthetic construct
RTSNLAS

SEQ ID NO: 322 - protein, 9 aa, synthetic construct
QQGSSLPLT

SEQ ID NO: 323 - protein, 117 aa, synthetic construct
EIQLVQSGAEVKKPGASVKVSCKASGYAFTSQNIYWVRQAPGQGLEWIGYIEPYNVVPMYNPKFKGRATLTVDKSTSTAYLELSSLRSEDTAVYYCARSGSSNFDYWGQGTLVTVSS

SEQ ID NO: 324 - protein, 108 aa, synthetic construct
DIQLTQSPSSLSASVGDRVTITCSASSSISSHYLHWYQQKPGKSPKLLIYRTSNLASGVPSRFSGSGSGTDYTLTISSLQPEDFATYYCQQGSSLPLTFGQGTKVEIK

SEQ ID NO: 325 - protein, 5 aa, synthetic construct
NYAMH

SEQ ID NO: 326 - protein, 17 aa, synthetic construct
LIWYDGSNKFYGDSVKG

SEQ ID NO: 327 - protein, 6 aa, synthetic construct
EGSGHY

SEQ ID NO: 328 - protein, 11 aa, synthetic construct
RASQGISSALA

SEQ ID NO: 329 - protein, 7 aa, synthetic construct
DASSLES

SEQ ID NO: 330 - protein, 9 aa, synthetic construct
QQFNSYPIT

SEQ ID NO: 331 - protein, 115 aa, synthetic construct
QVQLVESGGGVVQPGRSLRLSCAASGFTFSNYAMHWVRQAPGEGLEWVALIWYDGSNKFYGDSVKGRFTISRDNSKNTLYLQMNSLSAEDTAVYYCAREGSGHYWGQGTLVTVSS

SEQ ID NO: 332 - protein, 107 aa, synthetic construct
AIQLTQSPSSLSASVGDRVTITCRASQGISSALAWYQQKPGKVPKSLIYDASSLESGVPSRFSGSGSGTDFTLTISSLQPEDFATYYCQQFNSYPITFGQGTRLEIK

SEQ ID NO: 333 - protein, 5 aa, synthetic construct
NYAMS

SEQ ID NO: 334 - protein, 17 aa, synthetic construct
YISPGGDYIYYADSVKG

SEQ ID NO: 335 - protein, 12 aa, synthetic construct
DRRHYGSYAMDY

SEQ ID NO: 336 - protein, 16 aa, synthetic construct
RSSKSLLHSNLNTYLY

SEQ ID NO: 337 - protein, 7 aa, synthetic construct
RMSNLAS

SEQ ID NO: 338 - protein, 9 aa, synthetic construct
MQHLEYPFT

SEQ ID NO: 339 - protein, 121 aa, synthetic construct
QVQLVESGGGLVKPGGSLRLSCAASGFTFSNYAMSWIRQAPGKGLEWVSYISPGGDYIYYADSVKGRFTISRDNAKNSLYLQMNSLRAEDTAVYYCTTDRRHYGSYAMDYWGQGTLVTVSS

SEQ ID NO: 340 - protein, 112 aa, synthetic construct
DIVMTQSPLSLPVTPGEPASISCRSSKSLLHSNLNTYLYWFLQKPGQSPQILIYRMSNLASGVPDRFSGSGSGTAFTLKISRVEAEDVGVYYCMQHLEYPFTFGPGTKLEIK

SEQ ID NO: 341 - protein, 5 aa, synthetic construct
TYAFH

SEQ ID NO: 342 - protein, 17 aa, synthetic construct
GIVPIFGTLKYAQKFQD

SEQ ID NO: 343 - protein, 11 aa, synthetic construct
AIQLEGRPFDH

SEQ ID NO: 344 - protein, 11 aa, synthetic construct
RASQGITSYLA

SEQ ID NO: 345 - protein, 7 aa, synthetic construct
AASALQS

SEQ ID NO: 346 - protein, 10 aa, synthetic construct
QQVNRGAAIT

SEQ ID NO: 347 - protein, 120 aa, synthetic construct
QVQLVQSGAEVKKPGSSVRVSCRASGGSSTTYAFHWVRQAPGQGLEWMGGIVPIFGTLKYAQKFQDRVTLTADKSTGTAYMELNSLRLDDTAVYYCARAIQLEGRPFDHWGQGTQVTVSA

SEQ ID NO: 348 - protein, 108 aa, synthetic construct
DIQLTQSPSFLSASVGDRVTITCRASQGITSYLAWYQQKPGKAPKLLIYAASALQSGVPSRFSGRGSGTEFTLTISSLQPEDFATYYCQQVNRGAAITFGHGTRLDIK

SEQ ID NO: 349 - protein, 5 aa, synthetic construct
RYTMH

SEQ ID NO: 350 - protein, 17 aa, synthetic construct
VISFDGSNKYYVDSVKG

SEQ ID NO: 351 - protein, 10 aa, synthetic construct
EARGSYAFDI

SEQ ID NO: 352 - protein, 11 aa, synthetic construct
RASQSVSSYLA

SEQ ID NO: 353 - protein, 7 aa, synthetic construct
DASNRAT

SEQ ID NO: 354 - protein, 10 aa, synthetic construct
QQRSNWPPFT

SEQ ID NO: 355 - protein, 119 aa, synthetic construct
QVQLVESGGGVVQPGRSRRLSCAASGFTFSRYTMHWVRQAPGKGLEWVAVISFDGSNKYYVDSVKGRFTISRDNSENTLYLQVNILRAEDTAVYYCAREARGSYAFDIWGQGTMVTVSS

SEQ ID NO: 356 - protein, 108 aa, synthetic construct
EIVLTQSPATLSLSPGERATLSCRASQSVSSYLAWYQQKPGQAPRLLIYDASNRATGIPARFSGSGSGTDFTLTISSLEPEDFAVYYCQQRSNWPPFTFGPGTKVDIK

SEQ ID NO: 357 - protein, 5 aa, synthetic construct
SFWMH

SEQ ID NO: 358 - protein, 17 aa, synthetic construct
YINPRSGYTEYNEIFRD

SEQ ID NO: 359 - protein, 9 aa, synthetic construct
FLGRGAMDY

SEQ ID NO: 360 - protein, 11 aa, synthetic construct
RASQDISNYLA

SEQ ID NO: 361 - protein, 7 aa, synthetic construct
YTSKIHS

SEQ ID NO: 362 - protein, 9 aa, synthetic construct
QQGNTFPYT

SEQ ID NO: 363 - protein, 118 aa, synthetic construct [sequence omitted]

SEQ ID NO: 364 - protein, 107 aa, synthetic construct [sequence omitted]

SEQ ID NO: 365 - protein, 7 aa, synthetic construct
TSSYYWG

SEQ ID NO: 366 - protein, 16 aa, synthetic construct
TIYYNGSTYYSPSLKS

SEQ ID NO: 367 - protein, 11 aa, synthetic construct
QGYDIKINIDV

SEQ ID NO: 368 - protein, 11 aa, synthetic construct
RASQSVSSYLA

SEQ ID NO: 369 - protein, 7 aa, synthetic construct
VASNRAT

SEQ ID NO: 370 - protein, 9 aa, synthetic construct
QQRSNWPLT

SEQ ID NO: 371 - protein, 121 aa, synthetic construct
QLQLQESGPGLVKPSETLSLTCTVSGGSISTSSYYWGWIRQPPGKGLEWIGTIYYNGSTYYSPSLKSRVSISVDTSKNQFSLKLSSVTAADTSVYYCARQGYDIKINIDVWGQGTTVTVSS

SEQ ID NO: 372 - protein, 107 aa, synthetic construct
EIVLTQSPATLSLSPGERATLSCRASQSVSSYLAWYQQKPGQAPRLLIYVASNRATGIPARFSGSGSGTDFTLTISSLEPEDFAVYYCQQRSNWPLTFGGGTKVEIK

SEQ ID NO: 373 - protein, 5 aa, synthetic construct
SSWMN

SEQ ID NO: 374 - protein, 17 aa, synthetic construct
RIYPGDGNTHYAQKFQG

SEQ ID NO: 375 - protein, 8 aa, synthetic construct
GYLDPMDY

SEQ ID NO: 376 - protein, 11 aa, synthetic construct
QASQGINNYLN

SEQ ID NO: 377 - protein, 7 aa, synthetic construct
YTSGLHA

SEQ ID NO: 378 - protein, 9 aa, synthetic construct
QQYSILPWT

SEQ ID NO: 379 - protein, 117 aa, synthetic construct
QVQLVQSGAEVKKPGSSVKVSCKASGYAFTSSWMNWVRQAPGQGLEWMGRIYPGDGNTHYAQKFQGRVTLTADKSTSTAYMELSSLRSEDTAVYYCGEGYLDPMDYWGQGTLVTVSS

SEQ ID NO: 380 - protein, 107 aa, synthetic construct
DIQMTQSPSSLSASVGDRVTITCQASQGINNYLNWYQQKPGKAPKLLIHYTSGLHAGVPSRFSGSGSGTDYTLTISSLEPEDVATYYCQQYSILPWTFGGGTKVEIK

SEQ ID NO: 381 - protein, 5 aa, synthetic construct
SYGMH

SEQ ID NO: 382 - protein, 17 aa, synthetic construct
VISYDGSNKYYADSVKG

SEQ ID NO: 383 - protein, 18 aa, synthetic construct
DMGWGSGWRPYYYYGMDV

SEQ ID NO: 384 - protein, 11 aa, synthetic construct
RTSQSISSYLN

SEQ ID NO: 385 - protein, 7 aa, synthetic construct
WASTRES

SEQ ID NO: 386 - protein, 9 aa, synthetic construct
QQSYDIPYT

SEQ ID NO: 387 - protein, 127 aa, synthetic construct
EVQLLESGGGVVQPGRSLRLSCAASGFTFSSYGMHWVRQAPGKGLEWVAVISYDGSNKYYADSVKGRFTISRDNSKNTLYLQMNSLRAEDTAVYYCAKDMGWGSGWRPYYYYGMDVWGQGTTVTVSS

SEQ ID NO: 388 - protein, 107 aa, synthetic construct
ELQMTQSPSSLSASVGDRVTITCRTSQSISSYLNWYQQKPGQPPKLLIYWASTRESGVPDRFSGSGSGTDFTLTISSLQPEDSATYYCQQSYDIPYTFGQGTKLEIK

SEQ ID NO: 389 - protein, 5 aa, synthetic construct
NYWMS

SEQ ID NO: 390 - protein, 17 aa, synthetic construct
NIKQDGSEKFYADSVKG

SEQ ID NO: 391 - protein, 9 aa, synthetic construct
VGPSWEQDY

SEQ ID NO: 392 - protein, 14 aa, synthetic construct
TGSSSNIGSYYGVH

SEQ ID NO: 393 - protein, 7 aa, synthetic construct
SDTNRPS

SEQ ID NO: 394 - protein, 11 aa, synthetic construct
QSYDKGFGHRV

SEQ ID NO: 395 - protein, 118 aa, synthetic construct
EVQLVESGGGLVQPGGSLRLSCAASGFTFSNYWMSWVRQAPGKGLEWVANIKQDGSEKFYADSVKGRFTISRDNAKNSLYLQMNSLRAEDTAVYYCARVGPSWEQDYWGQGTLVTVSA

SEQ ID NO: 396 - protein, 111 aa, synthetic construct
QSVLTQPPSVSGAPGQRVTISCTGSSSNIGSYYGVHWYQQLPGTAPKLLIYSDTNRPSGVPDRFSGSKSGTSASLAITGLQAEDEADYYCQSYDKGFGHRVFGGGTKLTVL

SEQ ID NO: 397 - protein, 5 aa, synthetic construct
SYAIS

SEQ ID NO: 398 - protein, 17 aa, synthetic construct
GIIPIFGTANYAQKFQG

SEQ ID NO: 399 - protein, 6 aa, synthetic construct
GLLWNY

SEQ ID NO: 400 - protein, 11 aa, synthetic construct
RASQSVSSNLA

SEQ ID NO: 401 - protein, 7 aa, synthetic construct
GASTTAS

SEQ ID NO: 402 - protein, 11 aa, synthetic construct
QQYNNWPPAYT

SEQ ID NO: 403 - protein, 115 aa, synthetic construct
QVQLVQSGAEVKKPGSSVKVSCKASGGTFSSYAISWVRQAPGQGLEWMGGIIPIFGTANYAQKFQGRVTITADESTSTAYMELSSLRSEDTAVYYCARGLLWNYWGQGTLVTVSS

SEQ ID NO: 404 - protein, 109 aa, synthetic construct
EIVMTQSPATLSVSPGERATLSCRASQSVSSNLAWYQQKPGQAPRLIIYGASTTASGIPARFSASGSGTDFTLTISSLQSEDFAVYYCQQYNNWPPAYTFGQGTKLEIK

SEQ ID NO: 405 - protein, 5 aa, synthetic construct
NYGMN

SEQ ID NO: 406 - protein, 17 aa, synthetic construct
WINTYTGEPTYGEDFKG

SEQ ID NO: 407 - protein, 7 aa, synthetic construct
FGNYVDY

SEQ ID NO: 408 - protein, 16 aa, synthetic construct
RSSKNLLHSNGITYLY

SEQ ID NO: 409 - protein, 7 aa, synthetic construct
QMSNLAS

SEQ ID NO: 410 - protein, 9 aa, synthetic construct
AQNLEIPRT

SEQ ID NO: 411 - protein, 116 aa, synthetic construct
QVQLVQSGPEVKKPGASVKVSCKASGYTFTNYGMNWVRQAPGQGLEWMGWINTYTGEPTYGEDFKGRFAFSLDTSASTAYMELSSLRSEDTAVYFCARFGNYVDYWGQGSLVTVSS

SEQ ID NO: 412 - protein, 112 aa, synthetic construct
DIVMTQSPLSLPVTPGEPASISCRSSKNLLHSNGITYLYWYLQKPGQSPQLLIYQMSNLASGVPDRFSSSGSGTDFTLKISRVEAEDVGVYYCAQNLEIPRTFGQGTKVEIK

SEQ ID NO: 413 - protein, 5 aa, synthetic construct
KYGMN

SEQ ID NO: 414 - protein, 17 aa, synthetic construct
WINTYTEEPTYGDDFKG

SEQ ID NO: 415 - protein, 7 aa, synthetic construct
FGSAVDY

SEQ ID NO: 416 - protein, 16 aa, synthetic construct
RSSKSLLHSNGITYLY

SEQ ID NO: 417 - protein, 7 aa, synthetic construct
QMSNRAS

SEQ ID NO: 418 - protein, 9 aa, synthetic construct
AQNLELPRT

SEQ ID NO: 419 - protein, 116 aa, synthetic construct
QIQLVQSGPEVKKPGESVKISCKASGYTFTKYGMNWVKQAPGQGLKWMGWINTYTEEPTYGDDFKGRFTFTLDTSTSTAYLEISSLRSEDTATYFCARFGSAVDYWGQGTLVTVSS

SEQ ID NO: 420 - protein, 113 aa, synthetic construct
DIVMTQSALSNPVTLGESGSISCRSSKSLLHSNGITYLYWYLQKPGQSPQLLIYQMSNRASGVPDRFSSSGSGTDFTLKISRVEAEDVGVYYCAQNLELPRTFGQGTKLEMKR

SEQ ID NO: 421 - protein, 5 aa, synthetic construct
DYSMH

SEQ ID NO: 422 - protein, 17 aa, synthetic construct
WINTETGEPTYADDFKG

SEQ ID NO: 423 - protein, 4 aa, synthetic construct
TAVY

SEQ ID NO: 424 - protein, 11 aa, synthetic construct
RASQEISVSLS

SEQ ID NO: 425 - protein, 7 aa, synthetic construct
ATSTLDS

SEQ ID NO: 426 - protein, 9 aa, synthetic construct
LQYASYPWT

SEQ ID NO: 427 - protein, 113 aa, synthetic construct
QVKLQESGPELKKPGETVKISCKASGYTFTDYSMHWVKQAPGKGLKWMGWINTETGEPTYADDFKGRFAFSLETSASTAYLQINNLKNEDTATYFCARTAVYWGQGTTVTVSS

SEQ ID NO: 428 - protein, 108 aa, synthetic construct
DIQMTQSPSSLSASLGERVSLTCRASQEISVSLSWLQQEPDGTIKRLIYATSTLDSGVPKRFSGSRSGSDYSLTISSLESEDFVDYYCLQYASYPWTFGGGTKLEIKR

SEQ ID NO: 429 - protein, 5 aa, synthetic construct
NYGMN

SEQ ID NO: 430 - protein, 17 aa, synthetic construct
WINTYSGEPRYADDFKG

SEQ ID NO: 431 - protein, 9 aa, synthetic construct
DYGRWYFDV

SEQ ID NO: 432 - protein, 10 aa, synthetic construct
RASSSVSHMH

SEQ ID NO: 433 - protein, 7 aa, synthetic construct
ATSNLAS

SEQ ID NO: 434 - protein, 9 aa, synthetic construct
QQWSSTPRT

SEQ ID NO: 435 - protein, 118 aa, synthetic construct
QIQLVQSGSELKKPGASVKVSCKASGYTFTNYGMNWVRQAPGQDLKWMGWINTYSGEPRYADDFKGRFVFSLDKSVNTAYLQISSLKAEDTAVYYCARDYGRWYFDVWGQGTTVTVSS

SEQ ID NO: 436 - protein, 107 aa, synthetic construct
QIVLSQSPATLSLSPGERATMSCRASSSVSHMHWYQQKPGQAPRPWIYATSNLASGVPARFSGSGSGTDYTLTISSLEPEDFAVYYCQQWSSTPRTFGGGTKVEIKR

SEQ ID NO: 437 - protein, 5 aa, synthetic construct
RYWMS

SEQ ID NO: 438 - protein, 17 aa, synthetic construct
EINPDSSTINYAPSLKD

SEQ ID NO: 439 - protein, 10 aa, synthetic construct
PDGNYWYFDV

SEQ ID NO: 440 - protein, 11 aa, synthetic construct
KASQDVGIAVA

SEQ ID NO: 441 - protein, 7 aa, synthetic construct
WASTRHT

SEQ ID NO: 442 - protein, 9 aa, synthetic construct
QQYSSYPYT

SEQ ID NO: 443 - protein, 119 aa, synthetic construct
EVQLVESGGGLVQPGGSLRLSCAASGFDFSRYWMSWVRQAPGKGLEWIGEINPDSSTINYAPSLKDKFIISRDNAKNSLYLQMNSLRAEDTAVYYCARPDGNYWYFDVWGQGTLVTVSS

SEQ ID NO: 444 - protein, 108 aa, synthetic construct
DIQMTQSPSSLSASVGDRVTITCKASQDVGIAVAWYQQKPGKVPKLLIYWASTRHTGVPDRFSGSGSGTDFTLTISSLQPEDVATYYCQQYSSYPYTFGQGTKVEIKR

SEQ ID NO: 445 - protein, 5 aa, synthetic construct
SFAMS

SEQ ID NO: 446 - protein, 17 aa, synthetic construct
AISGSGGGTYYADSVKG

SEQ ID NO: 447 - protein, 13 aa, synthetic construct
DKILWFGEPVFDY

SEQ ID NO: 448 - protein, 11 aa, synthetic construct
RASQSVSSYLA

SEQ ID NO: 449 - protein, 7 aa, synthetic construct
DASNRAT

SEQ ID NO: 450 - protein, 9 aa, synthetic construct
QQRSNWPPT

SEQ ID NO: 451 - protein, 122 aa, synthetic construct [sequence omitted]

SEQ ID NO: 452 - protein, 108 aa, synthetic construct
EIVLTQSPATLSLSPGERATLSCRASQSVSSYLAWYQQKPGQAPRLLIYDASNRATGIPARFSGSGSGTDFTLTISSLEPEDFAVYYCQQRSNWPPTFGQGTKVEIKR

SEQ ID NO: 453 - protein, 5 aa, synthetic construct
SYRMH

SEQ ID NO: 454 - protein, 17 aa, synthetic construct
YINPSTGYTEYNQKFKD

SEQ ID NO: 455 - protein, 7 aa, synthetic construct
GGGVFDY

SEQ ID NO: 456 - protein, 10 aa, synthetic construct
SASSSISYMH

SEQ ID NO: 457 - protein, 7 aa, synthetic construct
TTSNLAS

SEQ ID NO: 458 - protein, 9 aa, synthetic construct
HQRSTYPLT

SEQ ID NO: 459 - protein, 116 aa, synthetic construct
QVQLVQSGAEVKKPGSSVKVSCKASGYTFTSYRMHWVRQAPGQGLEWIGYINPSTGYTEYNQKFKDKATITADESTNTAYMELSSLRSEDTAVYYCARGGGVFDYWGQGTLVTVSS

SEQ ID NO: 460 - protein, 106 aa, synthetic construct
DIQMTQSPSTLSASVGDRVTITCSASSSISYMHWYQQKPGKAPKLLIYTTSNLASGVPARFSGSGSGTEFTLTISSLQPDDFATYYCHQRSTYPLTFGQGTKVEVK

SEQ ID NO: 461 - protein, 5 aa, synthetic construct
SYWMH

SEQ ID NO: 462 - protein, 17 aa, synthetic construct
EIIPINGHTNYNEKFKS

SEQ ID NO: 463 - protein, 14 aa, synthetic construct
GGYYYYGSRDYFDY

SEQ ID NO: 464 - protein, 15 aa, synthetic construct
KASQSVDYDGDSYMN

SEQ ID NO: 465 - protein, 7 aa, synthetic construct
AASDLES

SEQ ID NO: 466 - protein, 9 aa, synthetic construct
QQSHEDPFT

SEQ ID NO: 467 - protein, 123 aa, synthetic construct
QVQLQQPGAELVKPGASVKLSCKASGYTFTSYWMHWVKQRPGQGLEWIGEIIPINGHTNYNEKFKSKATLTLDKSSSTAYMQLSSLASEDSAVYYCARGGYYYYGSRDYFDYWGQGTTLTVSS

SEQ ID NO: 468 - protein, 111 aa, synthetic construct
DIVLTQSPASLAVSLGQRATISCKASQSVDYDGDSYMNWYQQIPGQPPKLLIYAASDLESGIPARFSGSGSGTDFTLNIHPVEEEDAATYYCQQSHEDPFTFGGGTKLEIK

SEQ ID NO: 469 - protein, 5 aa, synthetic construct
SYWMH

SEQ ID NO: 470 - protein, 17 aa, synthetic construct
EIIPIFGHTNYNEKFKS

SEQ ID NO: 471 - protein, 14 aa, synthetic construct
GGYYYYPRQGFLDY

SEQ ID NO: 472 - protein, 15 aa, synthetic construct
KASQSVDYSGDSYMN

SEQ ID NO: 473 - protein, 7 aa, synthetic construct
AASDLES

SEQ ID NO: 474 - protein, 9 aa, synthetic construct
QQSHEDPFT

SEQ ID NO: 475 - protein, 123 aa, synthetic construct
EVQLVESGGGLVKPGGSLRLSCAASGFTFSSYWMHWVRQAPGKGLEWVGEIIPIFGHTNYNEKFKSRFTISLDNSKNTLYLQMGSLRAEDTAVYYCARGGYYYYPRQGFLDYWGQGTTVTVSS

SEQ ID NO: 476 - protein, 111 aa, synthetic construct
DIVMTQSPDSLAVSLGERATISCKASQSVDYSGDSYMNWYQQKPGQPPKLLIYAASDLESGIPARFSGSGSGTDFTLTISSLEPEDFATYYCQQSHEDPFTFGQGTKLEIK

SEQ ID NO: 477 - protein, 5 aa, synthetic construct
SYGMN

SEQ ID NO: 478 - protein, 17 aa, synthetic construct
YISSSSSTIYYADSVKG

SEQ ID NO: 479 - protein, 6 aa, synthetic construct
GPGMDV

SEQ ID NO: 480 - protein, 17 aa, synthetic construct
KSSQSVLYSSNNKNYLA

SEQ ID NO: 481 - protein, 7 aa, synthetic construct
WASTRES

SEQ ID NO: 482 - protein, 10 aa, synthetic construct
QQYYSTPQLT

SEQ ID NO: 483 - protein, 114 aa, synthetic construct
QVQLQQSGGGVVQPGRSLGLSCAASGFTFSSYGMNWVRQAPGKGLEWVSYISSSSSTIYYADSVKGRFTISRDNSKNTLYLQMNSLRAEDTAVYYCARGPGMDVWGQGTTVTVS

SEQ ID NO: 484 - protein, 114 aa, synthetic construct
DIVLTQSPDSLAVSLGERATINCKSSQSVLYSSNNKNYLAWYQQKPGQPPKLLIYWASTRESGVPDRFSGSGSGTDFTPAISSLQAEDVAVYYCQQYYSTPQLTFGGGTKVDIK

SEQ ID NO: 485 - protein, 7 aa, synthetic construct
TSGMGVG

SEQ ID NO: 486 - protein, 16 aa, synthetic construct
HIWWDDDKRYNPALKS

SEQ ID NO: 487 - protein, 10 aa, synthetic construct
MELWSYYFDY

SEQ ID NO: 488 - protein, 10 aa, synthetic construct
SASSSVSYMH

SEQ ID NO: 489 - protein, 7 aa, synthetic construct
DTSKLAS

SEQ ID NO: 490 - protein, 9 aa, synthetic construct
FQGSVYPFT

SEQ ID NO: 491 - protein, 120 aa, synthetic construct
QVQLQESGPGLVKPSQTLSLTCTVSGGSISTSGMGVGWIRQHPGKGLEWIGHIWWDDDKRYNPALKSRVTISVDTSKNQFSLKLSSVTAADTAVYYCARMELWSYYFDYWGQGTLVTVSS

SEQ ID NO: 492 - protein, 107 aa, synthetic construct
EIVLTQSPATLSLSPGERATLSCSASSSVSYMHWYQQKPGQAPRLLIYDTSKLASGIPARFSGSGSGTDFTLTISSLEPEDVAVYYCFQGSVYPFTFGQGTKLEIKR

SEQ ID NO: 493 - protein, 450 aa, synthetic construct
QVQLQESGPGLVKPSQTLSLTCTVSGGSISTSGMGVGWIRQHPGKGLEWIGHIWWDDDKRYNPALKSRVTISVDTSKNQFSLKLSSVTAADTAVYYCARMELWSYYFDYWGQGTLVTVSSASTKGPSVFPLAPSSKSTSGGTAALGCLVKDYFPEPVTVSWNSGALTSGVHTFPAVLQSSGLYSLSSVVTVPSSSLGTQTYICNVNHKPSNTKVDKKVEPKSCDKTHTCPPCPAPELLGGPSVFLFPPKPKDTLMISRTPEVTCVVVDVSHEDPEVKFNWYVDGVEVHNAKTKPREEQYNSTYRVVSVLTVLHQDWLNGKEYKCKVSNKALPAPIEKTISKAKGQPREPQVYTLPPSRDELTKNQVSLTCLVKGFYPSDIAVEWESNGQPENNYKTTPPVLDSDGSFFLYSKLTVDKSRWQQGNVFSCSVMHEALHNHYTQKSLSLSPGK

SEQ ID NO: 494 - protein, 213 aa, synthetic construct
EIVLTQSPATLSLSPGERATLSCSASSSVSYMHWYQQKPGQAPRLLIYDTSKLASGIPARFSGSGSGTDFTLTISSLEPEDVAVYYCFQGSVYPFTFGQGTKLEIKRTVAAPSVFIFPPSDEQLKSGTASVVCLLNNFYPREAKVQWKVDNALQSGNSQESVTEQDSKDSTYSLSSTLTLSKADYEKHKVYACEVTHQGLSSPVTKSFNRGEC

SEQ ID NO: 495 - protein, 5 aa, synthetic construct
NYWIE

SEQ ID NO: 496 - protein, 17 aa, synthetic construct
EILPGTGRTIYNEKFKG

SEQ ID NO: 497 - protein, 13 aa, synthetic construct
RDYYGNFYYAMDY

SEQ ID NO: 498 - protein, 11 aa, synthetic construct
SASQGINNYLN

SEQ ID NO: 499 - protein, 7 aa, synthetic construct
YTSTLQS

SEQ ID NO: 500 - protein, 9 aa, synthetic construct
QQYSKLPRT

SEQ ID NO: 501 - protein, 122 aa, synthetic construct
QVQLQQSGSELMMPGASVKISCKATGYTFSNYWIEWVKQRPGHGLEWIGEILPGTGRTIYNEKFKGKATFTADISSNTVQMQLSSLTSEDSAVYYCARRDYYGNFYYAMDYWGQGTSVTVSS

SEQ ID NO: 502 - protein, 107 aa, synthetic construct
DIQMTQSTSSLSASLGDRVTISCSASQGINNYLNWYQQKPDGTVELLIYYTSTLQSGVPSRFSGSGSGTDYSLTISNLEPEDIGTYYCQQYSKLPRTFGGGTKLEIK

SEQ ID NO: 503 - protein, 7 aa, synthetic construct
TYGMGVG

SEQ ID NO: 504 - protein, 16 aa, synthetic construct
NIWWSEDKHYSPSLKS

SEQ ID NO: 505 - protein, 11 aa, synthetic construct
IDYGNDYAFTY

SEQ ID NO: 506 - protein, 16 aa, synthetic construct
RSSKSLLHSNGITYLY

SEQ ID NO: 507 - protein, 7 aa, synthetic construct
QMSNLAS

SEQ ID NO: 508 - protein, 9 aa, synthetic construct
AQNLELPYT

SEQ ID NO: 509 - protein, 121 aa, synthetic construct
QITLKESGPTLVKPTQTLTLTCTFSGFSLSTYGMGVGWIRQPPGKALEWLANIWWSEDKHYSPSLKSRLTITKDTSKNQVVLTITNVDPVDTATYYCVQIDYGNDYAFTYWGQGTLVTVSS

SEQ ID NO: 510 - protein, 112 aa, synthetic construct
DIVMTQSPLSLPVTPGEPASISCRSSKSLLHSNGITYLYWYLQKPGQSPQLLIYQMSNLASGVPDRFSGSGSGTDFTLKISRVEAEDVGVYYCAQNLELPYTFGQGTKLEIK

SEQ ID NO: 511 - protein, 5 aa, synthetic construct
SFGMH

SEQ ID NO: 512 - protein, 17 aa, synthetic construct
YISSGSFTIYYADSVKG

SEQ ID NO: 513 - protein, 9 aa, synthetic construct
MRKGYAMDY

SEQ ID NO: 514 - protein, 16 aa, synthetic construct
RSSQIIIHSDGNTYLE

SEQ ID NO: 515 - protein, 7 aa, synthetic construct
KVSNRFS

SEQ ID NO: 516 - protein, 9 aa, synthetic construct
FQGSHVPHT

SEQ ID NO: 517 - protein, 118 aa, synthetic construct
QVQLVESGGGVVQPGRSLRLSCAASGFTFSSFGMHWVRQAPGKGLEWVAYISSGSFTIYYADSVKGRFTISRDNSKNTLYLQMNSLRAEDTAVYYCARMRKGYAMDYWGQGTLVTVSS

SEQ ID NO: 518 - protein, 112 aa, synthetic construct
DVVMTQSPLSLPVTLGQPASISCRSSQIIIHSDGNTYLEWFQQRPGQSPRRLIYKVSNRFSGVPDRFSGSGSGTDFTLKISRVEAEDVGVYYCFQGSHVPHTFGQGTKVEIK

SEQ ID NO: 519 - protein, 5 aa, synthetic construct
NYGVN

SEQ ID NO: 520 - protein, 17 aa, synthetic construct
WINPNTGEPTFDDDFKG

SEQ ID NO: 521 - protein, 11 aa, synthetic construct
SRGKNEAWFAY

SEQ ID NO: 522 - protein, 16 aa, synthetic construct
RSSQSLVHRNGNTYLH

SEQ ID NO: 523 - protein, 7 aa, synthetic construct
TVSNRFS

SEQ ID NO: 524 - protein, 9 aa, synthetic construct
SQSSHVPPT

SEQ ID NO: 525 - protein, 120 aa, synthetic construct
QVQLQQSGSELKKPGASVKVSCKASGYTFTNYGVNWIKQAPGQGLQWMGWINPNTGEPTFDDDFKGRFAFSLDTSVSTAYLQISSLKADDTAVYFCSRSRGKNEAWFAYWGQGTLVTVSS

SEQ ID NO: 526 - protein, 112 aa, synthetic construct
DIQLTQSPLSLPVTLGQPASISCRSSQSLVHRNGNTYLHWFQQRPGQSPRLLIYTVSNRFSGVPDRFSGSGSGTDFTLKISRVEAEDVGVYFCSQSSHVPPTFGAGTRLEIK

SEQ ID NO: 527 - protein, 5 aa, synthetic construct
TYWMS

SEQ ID NO: 528 - protein, 17 aa, synthetic construct
EIHPDSSTINYAPSLKD

SEQ ID NO: 529 - protein, 10 aa, synthetic construct
LYFGFPWFAY

SEQ ID NO: 530 - protein, 11 aa, synthetic construct
KASQDVGTSVA

SEQ ID NO: 531 - protein, 7 aa, synthetic construct
WTSTRHT

SEQ ID NO: 532 - protein, 8 aa, synthetic construct
QQYSLYRS

SEQ ID NO: 533 - protein, 119 aa, synthetic construct
EVQLVESGGGVVQPGRSLRLSCSASGFDFTTYWMSWVRQAPGKGLEWIGEIHPDSSTINYAPSLKDRFTISRDNAKNTLFLQMDSLRPEDTGVYFCASLYFGFPWFAYWGQGTPVTVSS

SEQ ID NO: 534 - protein, 106 aa, synthetic construct
DIQLTQSPSSLSASVGDRVTITCKASQDVGTSVAWYQQKPGKAPKLLIYWTSTRHTGVPSRFSGSGSGTDFTFTISSLQPEDIATYYCQQYSLYRSFGQGTKVEIK

SEQ ID NO: 535 - protein, 5 aa, synthetic construct
YYGMN

SEQ ID NO: 536 - protein, 17 aa, synthetic construct
WIDTTTGEPTYAQKFQG

SEQ ID NO: 537 - protein, 10 aa, synthetic construct
RGPYNWYFDV

SEQ ID NO: 538 - protein, 16 aa, synthetic construct
RSSKSLLHSNGNTYLY

SEQ ID NO: 539 - protein, 7 aa, synthetic construct
RMSNLVS

SEQ ID NO: 540 - protein, 9 aa, synthetic construct
LQHLEYPFT

SEQ ID NO: 541 - protein, 119 aa, synthetic construct
QVQLVQSGAEVKKPGETVKISCKASDYTFTYYGMNWVKQAPGQGLKWMGWIDTTTGEPTYAQKFQGRIAFSLETSASTAYLQIKSLKSEDTATYFCARRGPYNWYFDVWGQGTTVTVSS

SEQ ID NO: 542 - protein, 112 aa, synthetic construct
DIVMTQSPLSVPVTPGEPVSISCRSSKSLLHSNGNTYLYWFLQRPGQSPQLLIYRMSNLVSGVPDRFSGSGSGTAFTLRISRVEAEDVGVYYCLQHLEYPFTFGPGTKLELK

SEQ ID NO: 543 - protein, 5 aa, synthetic construct
NYGMN

SEQ ID NO: 544 - protein, 17 aa, synthetic construct
WINTYTGEPTYADDFKG

SEQ ID NO: 545 - protein, 9 aa, synthetic construct
IGDSSPSDY

SEQ ID NO: 546 - protein, 11 aa, synthetic construct
KASQSVSNDVV

SEQ ID NO: 547 - protein, 7 aa, synthetic construct
YASNRYT

SEQ ID NO: 548 - protein, 9 aa, synthetic construct
QQDYTSPWT

SEQ ID NO: 549 - protein, 118 aa, synthetic construct
QVQLVQSGAEVKKPGASVKVSCKASGYTFTNYGMNWVRQAPGQGLEWMGWINTYTGEPTYADDFKGRVTMTTDTSTSTAYMELRSLRSDDTAVYYCARIGDSSPSDYWGQGTLVTVSS

SEQ ID NO: 550 - protein, 107 aa, synthetic construct
EIVMTQSPATLSVSPGERATLSCKASQSVSNDVVWYQQKPGQAPRLLIYYASNRYTGIPARFSGSGSGTEFTLTISSLQSEDFAVYYCQQDYTSPWTFGQGTKLEIK

SEQ ID NO: 551 - protein, 5 aa, synthetic construct
SYWIE

SEQ ID NO: 552 - protein, 17 aa, synthetic construct
EILPGSGNTYYNERFKD

SEQ ID NO: 553 - protein, 14 aa, synthetic construct
RAAAYYSNPEWFAY

SEQ ID NO: 554 - protein, 12 aa, synthetic construct
TASSSVNSFYLH

SEQ ID NO: 555 - protein, 7 aa, synthetic construct
STSNLAS

SEQ ID NO: 556 - protein, 9 aa, synthetic construct
HQYHRSPYT

SEQ ID NO: 557 - protein, 123 aa, synthetic construct
QVQLVQSGAEVKKPGSSVKVSCKASGGTFSSYWIEWVRQAPGQGLEWMGEILPGSGNTYYNERFKDRVTITADESTSTAYMELSSLRSEDTAVYYCARRAAAYYSNPEWFAYWGQGTLVTVSS

SEQ ID NO: 558 - protein, 108 aa, synthetic construct
EIVLTQSPATLSLSPGERATLSCTASSSVNSFYLHWYQQKPGLAPRLLIYSTSNLASGIPDRFSGSGSGTDFTLTISRLEPEDFAVYYCHQYHRSPYTFGQGTKLEIK

SEQ ID NO: 559 - protein, 5 aa, synthetic construct
SYWMQ

SEQ ID NO: 560 - protein, 17 aa, synthetic construct
TIYPGDGDTTYTQKFQG

SEQ ID NO: 561 - protein, 10 aa, synthetic construct
YDAPGYAMDY

SEQ ID NO: 562 - protein, 11 aa, synthetic construct
RASQDINNYLA

SEQ ID NO: 563 - protein, 7 aa, synthetic construct
YTSTLHP

SEQ ID NO: 564 - protein, 9 aa, synthetic construct
LQYDNLLYT

SEQ ID NO: 565 - protein, 119 aa, synthetic construct
QVQLVQSGAEVAKPGASVKLSCKASGYTFTSYWMQWVKQRPGQGLECIGTIYPGDGDTTYTQKFQGKATLTADKSSSTAYMQLSSLRSEDSAVYYCARYDAPGYAMDYWGQGTLVTVSS

SEQ ID NO: 566 - protein, 107 aa, synthetic construct
DIQMTQSPSSLSASVGDRVTITCRASQDINNYLAWYQHKPGKGPKLLIHYTSTLHPGIPSRFSGSGSGRDYSFSISSLEPEDIATYYCLQYDNLLYTFGQGTKLEIK

SEQ ID NO: 567 - protein, 6 aa, synthetic construct
RDFAWN

SEQ ID NO: 568 - protein, 16 aa, synthetic construct
YISYNGNTRYQPSLKS

SEQ ID NO: 569 - protein, 7 aa, synthetic construct
ASRGFPY

SEQ ID NO: 570 - protein, 11 aa, synthetic construct
HSSQDINSNIG

SEQ ID NO: 571 - protein, 7 aa, synthetic construct
HGTNLDD

SEQ ID NO: 572 - protein, 9 aa, synthetic construct
VQYAQFPWT

SEQ ID NO: 573 - protein, 116 aa, synthetic construct
EVQLQESGPGLVKPSQTLSLTCTVSGYSISRDFAWNWIRQPPGKGLEWMGYISYNGNTRYQPSLKSRITISRDTSKNQFFLKLNSVTAADTATYYCVTASRGFPYWGQGTLVTVSS

SEQ ID NO: 574 - protein, 107 aa, synthetic construct
DIQMTQSPSSMSVSVGDRVTITCHSSQDINSNIGWLQQKPGKSFKGLIYHGTNLDDGVPSRFSGSGSGTDYTLTISSLQPEDFATYYCVQYAQFPWTFGGGTKLEIK

SEQ ID NO: 575 - protein, 5 aa, synthetic construct
NYGVH

SEQ ID NO: 576 - protein, 16 aa, synthetic construct
VIWSGGNTDYNTPFTS

SEQ ID NO: 577 - protein, 11 aa, synthetic construct
ALTYYDYEFAY

SEQ ID NO: 578 - protein, 11 aa, synthetic construct
RASQSIGTNIH

SEQ ID NO: 579 - protein, 7 aa, synthetic construct
YASESIS

SEQ ID NO: 580 - protein, 9 aa, synthetic construct
QQNNNWPTT

SEQ ID NO: 581 - protein, 119 aa, synthetic construct
QVQLKQSGPGLVQPSQSLSITCTVSGFSLTNYGVHWVRQSPGKGLEWLGVIWSGGNTDYNTPFTSRLSINKDNSKSQVFFKMNSLQSNDTAIYYCARALTYYDYEFAYWGQGTLVTVSA

SEQ ID NO: 582 - protein, 107 aa, synthetic construct
DILLTQSPVILSVSPGERVSFSCRASQSIGTNIHWYQQRTNGSPRLLIKYASESISGIPSRFSGSGSGTDFTLSINSVESEDIADYYCQQNNNWPTTFGAGTKLELK

SEQ ID NO: 583 - protein, 5 aa, synthetic construct
GYFMN

SEQ ID NO: 584 - protein, 17 aa, synthetic construct
RIHPYDGDTFYNQKFQG

SEQ ID NO: 585 - protein, 9 aa, synthetic construct
YDGSRAMDY

SEQ ID NO: 586 - protein, 15 aa, synthetic construct
KASQSVSFAGTSLMH

SEQ ID NO: 587 - protein, 7 aa, synthetic construct
RASNLEA

SEQ ID NO: 588 - protein, 9 aa, synthetic construct
QQSREYPYT

SEQ ID NO: 589 - protein, 118 aa, synthetic construct
QVQLVQSGAEVVKPGASVKISCKASGYTFTGYFMNWVKQSPGQSLEWIGRIHPYDGDTFYNQKFQGKATLTVDKSSNTAHMELLSLTSEDFAVYYCTRYDGSRAMDYWGQGTTVTVSS

SEQ ID NO: 590 - protein, 111 aa, synthetic construct
DIVLTQSPLSLAVSLGQPAIISCKASQSVSFAGTSLMHWYHQKPGQQPRLLIYRASNLEAGVPDRFSGSGSKTDFTLTISPVEAEDAATYYCQQSREYPYTFGGGTKLEIK

SEQ ID NO: 591 - protein, 5 aa, synthetic construct
GYGLS

SEQ ID NO: 592 - protein, 17 aa, synthetic construct
MISSGGSYTYYADSVKG

SEQ ID NO: 593 - protein, 10 aa, synthetic construct
HGDDPAWFAY

SEQ ID NO: 594 - protein, 12 aa, synthetic construct
SVSSSISSNNLH

SEQ ID NO: 595 - protein, 7 aa, synthetic construct
GTSNLAS

SEQ ID NO: 596 - protein, 11 aa, synthetic construct
QQWSSYPYMYT

SEQ ID NO: 597 - protein, 119 aa, synthetic construct
EVQLVESGGGVVQPGRSLRLSCSASGFTFSGYGLSWVRQAPGKGLEWVAMISSGGSYTYYADSVKGRFAISRDNAKNTLFLQMDSLRPEDTGVYFCARHGDDPAWFAYWGQGTPVTVSS

SEQ ID NO: 598 - protein, 110 aa, synthetic construct
DIQLTQSPSSLSASVGDRVTITCSVSSSISSNNLHWYQQKPGKAPKPWIYGTSNLASGVPSRFSGSGSGTDYTFTISSLQPEDIATYYCQQWSSYPYMYTFGQGTKVEIK

SEQ ID NO: 599 - protein, 5 aa, synthetic construct
NYWMN

SEQ ID NO: 600 - protein, 19 aa, synthetic construct
EIRLKSNNYTTHYAESVKG

SEQ ID NO: 601 - protein, 6 aa, synthetic construct
HYYFDY

SEQ ID NO: 602 - protein, 16 aa, synthetic construct
RSSKSLLHSNGITYFF

SEQ ID NO: 603 - protein, 7 aa, synthetic construct
QMSNLAS

SEQ ID NO: 604 - protein, 9 aa, synthetic construct
AQNLELPPT

SEQ ID NO: 605 - protein, 117 aa, synthetic construct
EVQLVESGGGLVQPGGSMRLSCVASGFPFSNYWMNWVRQAPGKGLEWVGEIRLKSNNYTTHYAESVKGRFTISRDDSKNSLYLQMNSLKTEDTAVYYCTRHYYFDYWGQGTLVTVSS

SEQ ID NO: 606 - protein, 112 aa, synthetic construct
DIVMTQSPLSNPVTPGEPASISCRSSKSLLHSNGITYFFWYLQKPGQSPQLLIYQMSNLASGVPDRFSGSGSGTDFTLRISRVEAEDVGVYYCAQNLELPPTFGQGTKVEIK

SEQ ID NO: 607 - protein, 5 aa, synthetic construct
SYWIG

SEQ ID NO: 608 - protein, 17 aa, synthetic construct
IIDPGDSRTRYSPSFQG

SEQ ID NO: 609 - protein, 11 aa, synthetic construct
GQLYGGTYMDG

SEQ ID NO: 610 - protein, 14 aa, synthetic construct
TGTSSDIGGYNSVS

SEQ ID NO: 611 - protein, 7 aa, synthetic construct
GVNNRPS

SEQ ID NO: 612 - protein, 11 aa, synthetic construct
SSYDIESATPV

SEQ ID NO: 613 - protein, 120 aa, synthetic construct
QVELVQSGAEVKKPGESLKISCKGSGYSFTSYWIGWVRQAPGKGLEWMGIIDPGDSRTRYSPSFQGQVTISADKSISTAYLQWSSLKASDTAMYYCARGQLYGGTYMDGWGQGTLVTVSS

SEQ ID NO: 614 - protein, 111 aa, synthetic construct
DIALTQPASVSGSPGQSITISCTGTSSDIGGYNSVSWYQQHPGKAPKLMIYGVNNRPSGVSNRFSGSKSGNTASLTISGLQAEDEADYYCSSYDIESATPVFGGGTKLTVL

SEQ ID NO: 615 - protein, 5 aa, synthetic construct
AYNIH

SEQ ID NO: 616 - protein, 17 aa, synthetic construct
SFDPYDGGSSYNQKFKD

SEQ ID NO: 617 - protein, 7 aa, synthetic construct
GWYYFDY

SEQ ID NO: 618 - protein, 11 aa, synthetic construct
RASKSISKYLA

SEQ ID NO: 619 - protein, 7 aa, synthetic construct
SGSTLQS

SEQ ID NO: 620 - protein, 9 aa, synthetic construct
QQHDESPYT

SEQ ID NO: 621 - protein, 116 aa, synthetic construct
QVQLQESGPGLVKPSQTLSLTCTVSGYAFTAYNIHWVRQAPGQGLEWMGSFDPYDGGSSYNQKFKDRLTISKDTSKNQVVLTMTNMDPVDTATYYCARGWYYFDYWGHGTLVTVSS

SEQ ID NO: 622 - protein, 107 aa, synthetic construct
DIVMTQTPLSLPVTPGEPASISCRASKSISKYLAWYQQKPGQAPRLLIYSGSTLQSGIPPRFSGSGYGTDFTLTINNIESEDAAYYFCQQHDESPYTFGEGTKVEIK

SEQ ID NO: 623 - protein, 5 aa, synthetic construct
SFGMH

SEQ ID NO: 624 - protein, 17 aa, synthetic construct
YISSDSSAIYYADTVKG

SEQ ID NO: 625 - protein, 13 aa, synthetic construct
GRENIYYGSRLDY

SEQ ID NO: 626 - protein, 11 aa, synthetic construct
KASQNVDTNVA

SEQ ID NO: 627 - protein, 7 aa, synthetic construct
SASYRYS

SEQ ID NO: 628 - protein, 9 aa, synthetic construct
QQYNNYPFT

SEQ ID NO: 629 - protein, 122 aa, synthetic construct
DVQLVESGGGLVQPGGSRKLSCAASGFTFSSFGMHWVRQAPEKGLEWVAYISSDSSAIYYADTVKGRFTISRDNPKNTLFLQMTSLRSEDTAMYYCGRGRENIYYGSRLDYWGQGTTLTVSS

SEQ ID NO: 630 - protein, 107 aa, synthetic construct
DIAMTQSQKFMSTSVGDRVSVTCKASQNVDTNVAWYQQKPGQSPKALIYSASYRYSGVPDRFTGSGSGTDFTLTINNVQSEDLAEYFCQQYNNYPFTFGSGTKLEIK

SEQ ID NO: 631 - protein, 5 aa, synthetic construct
SYGMS

SEQ ID NO: 632 - protein, 17 aa, synthetic construct
TINSGGSNTYYPDSLKG

SEQ ID NO: 633 - protein, 8 aa, synthetic construct
HDGGAMDY

SEQ ID NO: 634 - protein, 11 aa, synthetic construct
RASESIYSYLA

SEQ ID NO: 635 - protein, 7 aa, synthetic construct
NTKTLPE

SEQ ID NO: 636 - protein, 10 aa, synthetic construct
QHHYGTPPWT

SEQ ID NO: 637 - protein, 117 aa, synthetic construct
EVQLVESGGGLVKPGGSLRLSCAASGFTFSSYGMSWVRQAPGKGLEWVATINSGGSNTYYPDSLKGRFTISRDNAKNSLYLQMNSLRAEDTAVYYCARHDGGAMDYWGQGTTVTVSS

SEQ ID NO: 638 - protein, 108 aa, synthetic construct
DIQMTQSPSSLSASVGDRVTITCRASESIYSYLAWYQQKPGKAPKLLVYNTKTLPEGVPSRFSGSGSGTDFTLTISSLQPEDFATYYCQHHYGTPPWTFGQGTRLEIK

SEQ ID NO: 639 - protein, 5 aa, synthetic construct
SFGMH

SEQ ID NO: 640 - protein, 17 aa, synthetic construct
YISSGSGTIYYADTVKG

SEQ ID NO: 641 - protein, 10 aa, synthetic construct
HGYRYEGFDY

SEQ ID NO: 642 - protein, 11 aa, synthetic construct
KASQNVDTNVA

SEQ ID NO: 643 - protein, 7 aa, synthetic construct
SASYRYS

SEQ ID NO: 644 - protein, 9 aa, synthetic construct
QQYNNYPFT

SEQ ID NO: 645 - protein, 119 aa, synthetic construct
EVQLVESGGGLVQPGGSLRLSCAASGFTFSSFGMHWVRQAPGKGLEWVAYISSGSGTIYYADTVKGRFTISRDNAKNSLYLQMNSLRAEDTAVYYCARHGYRYEGFDYWGQGTTVTVSS

SEQ ID NO: 646 - protein, 107 aa, synthetic construct
DIQMTQSPSFLSASVGDRVTITCKASQNVDTNVAWYQQKPGKAPKALIYSASYRYSGVPSRFSGSGSGTDFTLTISSLQPEDFAEYFCQQYNNYPFTFGQGTKLEIK

SEQ ID NO: 647 - protein, 5 aa, synthetic construct
NYVMH

SEQ ID NO: 648 - protein, 17 aa, synthetic construct
YINPYNDDVKYNEKFKG

SEQ ID NO: 649 - protein, 13 aa, synthetic construct
WGYYGSPLYYFDY

SEQ ID NO: 650 - protein, 10 aa, synthetic construct
RASSRLIYMH

SEQ ID NO: 651 - protein, 7 aa, synthetic construct
ATSNLAS

SEQ ID NO: 652 - protein, 9 aa, synthetic construct
QQWNSNPPT

SEQ ID NO: 653 - protein, 122 aa, synthetic construct
EVQLQQSGPELVKPGASVKMSCKASGYTFTNYVMHWVKQKPGQGLEWIGYINPYNDDVKYNEKFKGKATQTSDKSSSTAYMELSSLTSEDSAVYYCARWGYYGSPLYYFDYWGQGTTLTVSS

SEQ ID NO: 654 - protein, 106 aa, synthetic construct
QIVLSQSPTILSASPGEKVTMTCRASSRLIYMHWYQQKPGSSPKPWIYATSNLASGVPARFSGSGSGTSYSLTISRVEAEDAATYYCQQWNSNPPTFGTGTKLELK

SEQ ID NO: 655 - protein, 5 aa, synthetic construct
NYVMH

SEQ ID NO: 656 - protein, 17 aa, synthetic construct
YINPYNDDVKYNEKFKG

SEQ ID NO: 657 - protein, 13 aa, synthetic construct
WGYYGSPLYYFDY

SEQ ID NO: 658 - protein, 10 aa, synthetic construct
RASSRLIYMH

SEQ ID NO: 659 - protein, 7 aa, synthetic construct
ATSNLAS

SEQ ID NO: 660 - protein, 9 aa, synthetic construct
QQWNSNPPT

SEQ ID NO: 661 - protein, 122 aa, synthetic construct
QVQLVQSGAEVKKPGSSVKVSCKASGYTFTNYVMHWVRQAPGQGLEWMGYINPYNDDVKYNEKFKGRVTITADESTSTAYMELSSLRSEDTAVYYCARWGYYGSPLYYFDYWGQGTLVTVSS

SEQ ID NO: 662 - protein, 106 aa, synthetic construct
EIVLTQSPATLSLSPGERATLSCRASSRLIYMHWYQQKPGQAPRPLIYATSNLASGIPARFSGSGSGTDFTLTISSLEPEDFAVYYCQQWNSNPPTFGQGTKVEIK

SEQ ID NO: 663 - protein, 5 aa, synthetic construct
SYTIH

SEQ ID NO: 664 - protein, 17 aa, synthetic construct
YINPNSRNTDYAQKFQG

SEQ ID NO: 665 - protein, 12 aa, synthetic construct
YSGSTPYWYFDV

SEQ ID NO: 666 - protein, 10 aa, synthetic construct
RASSSVSYMN

SEQ ID NO: 667 - protein, 7 aa, synthetic construct
ATSNLAS

SEQ ID NO: 668 - protein, 9 aa, synthetic construct
QQWSSNPLT

SEQ ID NO: 669 - protein, 121 aa, synthetic construct
EVQLVQSGAEVKKPGSSVKVSCKASGYSFTSYTIHWVRQAPGQGLEWMGYINPNSRNTDYAQKFQGRVTLTADKSTSTAYMELSSLRSEDTAVYYCARYSGSTPYWYFDVWGQGTTVTVSS

SEQ ID NO: 670 - protein, 106 aa, synthetic construct
DIQLTQSPSFLSASVGDRVTITCRASSSVSYMNWYQQKPGKSPKPWIYATSNLASGVPSRFSVSVSGTEHTLTISSLQPEDFATYYCQQWSSNPLTFGQGTKLEIK

SEQ ID NO: 671 - protein, 5 aa, synthetic construct
SYWMH

SEQ ID NO: 672 - protein, 17 aa, synthetic construct
LIHPDSGSTNYNEMFKN

SEQ ID NO: 673 - protein, 8 aa, synthetic construct
GGRLYFDY

SEQ ID NO: 674 - protein, 16 aa, synthetic construct
RSSQSLVHSNGDTYLR

SEQ ID NO: 675 - protein, 7 aa, synthetic construct
KVSNRFS

SEQ ID NO: 676 - protein, 9 aa, synthetic construct
SQSTHVPYT

SEQ ID NO: 677 - protein, 117 aa, synthetic construct
EVQLVQSGAEVKKPGSSVKVSCKASGYTFSSYWMHWVRQAPGQGLEWIGLIHPDSGSTNYNEMFKNRATLTVDRSTSTAYVELSSLRSEDTAVYFCAGGGRLYFDYWGQGTTVTVSS

SEQ ID NO: 678 - protein, 112 aa, synthetic construct
DVVMTQSPLSLPVTPGEPASISCRSSQSLVHSNGDTYLRWYLQKPGQSPQLLIYKVSNRFSGVPDRFSGSGSGTDFTLKISRVEAEDVGVYYCSQSTHVPYTFGGGTKVEIK

SEQ ID NO: 679 - protein, 5 aa, synthetic construct
SYWMH

SEQ ID NO: 680 - protein, 17 aa, synthetic construct
LIHPESGSTNYNEMFKN

SEQ ID NO: 681 - protein, 8 aa, synthetic construct
GGRLYFDY

SEQ ID NO: 682 - protein, 16 aa, synthetic construct
RSSQSLVHSNQDTYLR

SEQ ID NO: 683 - protein, 7 aa, synthetic construct
KVSNRFS

SEQ ID NO: 684 - protein, 9 aa, synthetic construct
SQSTHVPYT

SEQ ID NO: 685 - protein, 117 aa, synthetic construct
EVQLVQSGAEVKKPGSSVKVSCKASGYTFSSYWMHWVRQAPGQGLEWIGLIHPESGSTNYNEMFKNRATLTVDRSTSTAYMELSSLRSEDTAVYYCAGGGRLYFDYWGQGTTVTVSS

SEQ ID NO: 686 - protein, 112 aa, synthetic construct
DIVMTQSPLSLPVTPGEPASISCRSSQSLVHSNQDTYLRWYLQKPGQSPQLLIYKVSNRFSGVPDRFSGSGSGTDFTLKISRVEAEDVGVYYCSQSTHVPYTFGGGTKVEIK

SEQ ID NO: 687 - protein, 6 aa, synthetic construct
SGYSWH

SEQ ID NO: 688 - protein, 16 aa, synthetic construct
YIHSSGSTNYNPSLKS

SEQ ID NO: 689 - protein, 7 aa, synthetic construct
YDDYFEY

SEQ ID NO: 690 - protein, 12 aa, synthetic construct
KASQNVGFNVAW

SEQ ID NO: 691 - protein, 7 aa, synthetic construct
SASYRYS

SEQ ID NO: 692 - protein, 9 aa, synthetic construct
QQYNWYPFT

SEQ ID NO: 693 - protein, 116 aa, synthetic construct
EVQLQESGPGLVKPSETLSLTCAVTGYSITSGYSWHWIRQFPGNGLEWMGYIHSSGSTNYNPSLKSRISISRDTSKNQFFLKLSSVTAADTAVYYCAGYDDYFEYWGQGTTVTVSS

SEQ ID NO: 694 - protein, 107 aa, synthetic construct
DIQMTQSPSSLSASVGDRVTITCKASQNVGFNVAWYQQKPGKSPKALIYSASYRYSGVPSRFSGSGSGTDFTLTISSLQPEDFAEYFCQQYNWYPFTFGQGTKLEIK

SEQ ID NO: 695 - protein, 5 aa, synthetic construct
NYDIN

SEQ ID NO: 696 - protein, 17 aa, synthetic construct
WIFPGDDSTQYNEKFKG

SEQ ID NO: 697 - protein, 9 aa, synthetic construct
QTTGTWFAY

SEQ ID NO: 698 - protein, 11 aa, synthetic construct
RASQSISDYLY

SEQ ID NO: 699 - protein, 7 aa, synthetic construct
YASQSIS

SEQ ID NO: 700 - protein, 9 aa, synthetic construct
QNGHSFPLT

SEQ ID NO: 701 - protein, 118 aa, synthetic construct
QVQLVQSGAEVVKPGASVKLSCKTSGYTFTNYDINWVRQRPGQGLEWIGWIFPGDDSTQYNEKFKGKATLTTDTSTSTAYMELSSLRSEDTAVYFCARQTTGTWFAYWGQGTLVTVSS

SEQ ID NO: 702 - protein, 107 aa, synthetic construct
EIVMTQSPATLSVSPGERVTLSCRASQSISDYLYWYQQKSHESPRLLIKYASQSISGIPARFSGSGSGSEFTLTINSVEPEDVGVYYCQNGHSFPLTFGQGTKLELK

SEQ ID NO: 703 - protein, 119 aa, synthetic construct
QVQLQQSGAEVKKPGSSVKVSCKASGGTFSSYAISWVRQAPGQGLEWMGGIIPILGIANYAQKFQGRVTITADESTSTAYMELSSLRSEDTAVYYCARGGSGSYHMDVWGKGTTVTVSS

SEQ ID NO: 704 - protein, 109 aa, synthetic construct
EIVLTQSPATLSLSPGERATLSCRASQSVSSYLAWYQQKPGQAPRLLIYDASNRATGIPARFSGSGSGTDFTLTISSLEPEDFAVYYCQQRSNWPPRITFGQGTRLEIK

SEQ ID NO: 705 - protein, 5 aa, synthetic construct
IYNVH

SEQ ID NO: 706 - protein, 17 aa, synthetic construct
TIFPGNGDTSYNQKFKD

SEQ ID NO: 707 - protein, 10 aa, synthetic construct
WDDGNVGFAH

SEQ ID NO: 708 - protein, 11 aa, synthetic construct
RASENINNYLT

SEQ ID NO: 709 - protein, 7 aa, synthetic construct
HAKTLAE

SEQ ID NO: 710 - protein, 9 aa, synthetic construct
QHHYGTPPT

SEQ ID NO: 711 - protein, 119 aa, synthetic construct
QVQLQQPGAELVKPGASVKMSCKASGYTFTIYNVHWIKQTPGQGLEWMGTIFPGNGDTSYNQKFKDKATLTTDKSSKTAYMQLNSLTSEDSAVYYCARWDDGNVGFAHWGQGTLVTVSA

SEQ ID NO: 712 - protein, 107 aa, synthetic construct
DIQMTQSPASLSASVGETVTITCRASENINNYLTWFQQKQGKSPQLLVYHAKTLAEGVPSRFSGSGSGTQFSLKINSLQPEDFGSYYCQHHYGTPPTFGGGTKLEIK

SEQ ID NO: 713 - protein, 119 aa, synthetic construct
EVQLVQSGAEVKKPGASVKVSCKASGYTFTIYNVHWVRQAPGQGLEWMGTIFPGNGDTSYNQKFKDKVTMTTDTSTSTAYMELSSLRSEDTAVYYCARWDDGNVGFAHWGQGTLVTVSS

SEQ ID NO: 714 - protein, 107 aa, synthetic construct
DIQMTQSPSSLSASVGDRVTITCRASENINNYLTWFQQKQGKSPQLLIYHAKTLAEGVPSRFSGSGSGTDFTLTISSLQPEDFATYYCQHHYGTPPTFGGGTKVEIK

SEQ ID NO: 715 - protein, 119 aa, synthetic construct
EVQLVQSGAEVKKPGASVKVSCKASGYTFTIYNVHWIRQAPGQGLEWMGTIFPGNGDTSYNQKFKDRATLTTDKSTKTAYMELRSLRSDDTAVYYCARWDDGNVGFAHWGQGTLVTVSS

SEQ ID NO: 716 - protein, 107 aa, synthetic construct
DIQMTQSPSSLSASVGDRVTITCRASENINNYLTWFQQKPGKAPKLLVYHAKTLAEGVPSRFSGSGSGTQFTLTISSLQPEDFATYYCQHHYGTPPTFGQGTKLEIK

SEQ ID NO: 717 - protein, 447 aa, synthetic construct
QVQLQQWGAGLLKPSETLSLTCAVYGGSFSGYYWSWIRQPPGKGLEWIGEINHSGSTNYNPSLKSRVTISVETSKNQFSLKLSSVTAADTAVYYCARDKWTWYFDLWGRGTLVTVSSASTKGPSVFPLAPSSKSTSGGTAALGCLVKDYFPEPVTVSWNSGALTSGVHTFPAVLQSSGLYSLSSVVTVPSSSLGTQTYICNVNHKPSNTKVDKRVEPKSCDKTHTCPPCPAPELLGGPSVFLFPPKPKDTLMISRTPEVTCVVVDVSHEDPEVKFNWYVDGVEVHNAKTKPREEQYNSTYRVVSVLTVLHQDWLNGKEYKCKVSNKALPAPIEKTISKAKGQPREPQVYTLPPSREEMTKNQVSLTCLVKGFYPSDIAVEWESNGQPENNYKTTPPVLDSDGSFFLYSKLTVDKSRWQQGNVFSCSVMHEALHNHYTQKSLSLSPGK

SEQ ID NO: 718 - protein, 220 aa, synthetic construct
DIEMTQSPDSLAVSLGERATINCRSSQSVLYSSSNRNYLAWYQQNPGQPPKLLIYWASTRESGVPDRFSGSGSGTDFTLTISSLQAEDVAVYYCQQYYSTPRTFGQGTKVEIKRTVAAPSVFIFPPSDEQLKSGTASVVCLLNNFYPREAKVQWKVDNALQSGNSQESVTEQDSKDSTYSLSSTLTLSKADYEKHKVYACEVTHQGLSSPVTKSFNRGEC

SEQ ID NO: 719 - protein, 445 aa, synthetic construct
EVQLLESGGGLVQPGGSLRLSCAASGFTFSHYVMAWVRQAPGKGLEWVSSISSSGGWTLYADSVKGRFTISRDNSKNTLYLQMNSLRAEDTAVYYCTRGLKMATIFDYWGQGTLVTVSSASTKGPSVFPLAPCSRSTSESTAALGCLVKDYFPEPVTVSWNSGALTSGVHTFPAVLQSSGLYSLSSVVTVPSSNFGTQTYTCNVDHKPSNTKVDKTVERKCCVECPPCPAPPVAGPSVFLFPPKPKDTLMISRTPEVTCVVVDVSHEDPEVQFNWYVDGVEVHNAKTKPREEQFNSTFRVVSVLTVVHQDWLNGKEYKCKVSNKGLPAPIEKTISKTKGQPREPQVYTLPPSREEMTKNQVSLTCLVKGFYPSDIAVEWESNGQPENNYKTTPPMLDSDGSFFLYSKLTVDKSRWQQGNVFSCSVMHEALHNHYTQKSLSLSPGK

SEQ ID NO: 720 - protein, 217 aa, synthetic construct
QSALTQPASVSGSPGQSITISCTGTSSDVGSYNVVSWYQQHPGKAPKLIIYEVSQRPSGVSNRFSGSKSGNTASLTISGLQTEDEADYYCCSYAGSSIFVIFGGGTKVTVLGQPKAAPSVTLFPPSSEELQANKATLVCLVSDFYPGAVTVAWKADGSPVKVGVETTKPSKQSNNKYAASSYLSLTPEQWKSHRSYSCRVTHEGSTVEKTVAPAECS

SEQ ID NO: 721 - protein, 447 aa, synthetic construct
EVQLLESGGGLVQPGGSLRLSCAASGFTFSSYAMSWVRQAPGKGLEWVSAINSQGKSTYYADSVKGRFTISRDNSKNTLYLQMNSLRAEDTAVYYCARWGDEGFDIWGQGTLVTVSSASTKGPSVFPLAPSSKSTSGGTAALGCLVKDYFPEPVTVSWNSGALTSGVHTFPAVLQSSGLYSLSSVVTVPSSSLGTQTYICNVNHKPSNTKVDKRVEPKSCDKTHTCPPCPAPELLGGPSVFLFPPKPKDTLMISRTPEVTCVVVDVSHEDPEVKFNWYVDGVEVHNAKTKPREEQYNSTYRVVSVLTVLHQDWLNGKEYKCKVSNKALPAPIEKTISKAKGQPREPQVYTLPPSREEMTKNQVSLTCLVKGFYPSDIAVEWESNGQPENNYKTTPPVLDSDGSFFLYSKLTVDKSRWQQGNVFSCSVMHEALHNHYTQKSLSLSPGK

SEQ ID NO: 722 - protein, 214 aa, synthetic construct
DIQMTQSPSSLSASVGDRVTITCRASQGISNWLAWYQQKPGKAPKLLIYGASSLQSGVPSRFSGSGSGTDFTLTISSLQPEDFATYYCQQYSSFPTTFGQGTKVEIKRTVAAPSVFIFPPSDEQLKSGTASVVCLLNNFYPREAKVQWKVDNALQSGNSQESVTEQDSKDSTYSLSSTLTLSKADYEKHKVYACEVTHQGLSSPVTKSFNRGEC

SEQ ID NO: 723 - protein, 449 aa, synthetic construct
QVQLVQSGAEVKKPGASVKVSCKASGYTFRSSYISWVRQAPGQGLEWMGWIYAGTGSPSYNQKLQGRVTMTTDTSTSTAYMELRSLRSDDTAVYYCARHRDYYSNSLTYWGQGTLVTVSSASTKGPSVFPLAPSSKSTSGGTAALGCLVKDYFPEPVTVSWNSGALTSGVHTFPAVLQSSGLYSLSSVVTVPSSSLGTQTYICNVNHKPSNTKVDKKVEPKSCDKTHTCPPCPAPELLGGPSVFLFPPKPKDTLMISRTPEVTCVVVDVSHEDPEVKFNWYVDGVEVHNAKTKPREEQYNSTYRVVSVLTVLHQDWLNGKEYKCKVSNKALPAPIEKTISKAKGQPREPQVYTLPPSRDELTKNQVSLTCLVKGFYPSDIAVEWESNGQPENNYKTTPPVLDSDGSFFLYSKLTVDKSRWQQGNVFSCSVMHEALHNHYTQKSLSLSPG

SEQ ID NO: 724 - protein, 220 aa, synthetic construct
DIVMTQSPDSLAVSLGERATINCKSSQSVLNSGNQKNYLTWYQQKPGQPPKLLIYWASTRESGVPDRFSGSGSGTDFTLTISSLQAEDVAVYYCQSDYSYPYTFGQGTKLEIKRTVAAPSVFIFPPSDEQLKSGTASVVCLLNNFYPREAKVQWKVDNALQSGNSQESVTEQDSKDSTYSLSSTLTLSKADYEKHKVYACEVTHQGLSSPVTKSFNRGEC

SEQ ID NO: 725 - protein, 7 aa, synthetic construct
TSNMGVG

SEQ ID NO: 726 - protein, 16 aa, synthetic construct
HIWWDDDKYYSPSLKS

SEQ ID NO: 727 - protein, 10 aa, synthetic construct
SNYGYAWFAY

SEQ ID NO: 728 - protein, 11 aa, synthetic construct
KASQDIYPYLN

SEQ ID NO: 729 - protein, 7 aa, synthetic construct
RTNRLLD

SEQ ID NO: 730 - protein, 9 aa, synthetic construct
LQYDEFPLT

SEQ ID NO: 731 - protein, 120 aa, synthetic construct
QITLKESGPTLVKPTQTLTLTCTFSGFSLSTSNMGVGWIRQPPGKALEWLAHIWWDDDKYYSPSLKSRLTITKDTSKNQVVLTMTNMDPVDTATYYCVRSNYGYAWFAYWGQGTLVTVSS

SEQ ID NO: 732 - protein, 107 aa, synthetic construct
DIQMTQSPSSLSASVGDRVTITCKASQDIYPYLNWFQQKPGKAPKTLIYRTNRLLDGVPSRFSGSGSGTDFTFTISSLQPEDIATYYCLQYDEFPLTFGAGTKLEIK

SEQ ID NO: 733 - protein, 5 aa, synthetic construct
DYAVH

SEQ ID NO: 734 - protein, 17 aa, synthetic construct
VISTYNDYTYNNQDFKG

SEQ ID NO: 735 - protein, 10 aa, synthetic construct
GNSYFYALDY

SEQ ID NO: 736 - protein, 15 aa, synthetic construct
RASESVDSYGKSFMH

SEQ ID NO: 737 - protein, 7 aa, synthetic construct
RASNLES

SEQ ID NO: 738 - protein, 9 aa, synthetic construct
QQSNEDPWT

SEQ ID NO: 739 - protein, 119 aa, synthetic construct
QVQLVQSGPEVKKPGASVKVSCKASGYTFTDYAVHWVRQAPGKRLEWIGVISTYNDYTYNNQDFKGRVTMTRDTSASTAYMELSRLRSEDTAVYYCARGNSYFYALDYWGQGTSVTVSS

SEQ ID NO: 740 - protein, 111 aa, synthetic construct
EIVLTQSPATLSLSPGERATLSCRASESVDSYGKSFMHWYQQKPGQAPRLLIYRASNLESGIPARFSGSGSGTDFTLTISSLEPEDFAVYYCQQSNEDPWTFGGGTKLEIK

SEQ ID NO: 741 - protein, 5 aa, synthetic construct
RYWMS

SEQ ID NO: 742 - protein, 17 aa, synthetic construct
DLNPDSSAINYVDSVKG

SEQ ID NO: 743 - protein, 11 aa, synthetic construct
ITTLVPYTMDF

SEQ ID NO: 744 - protein, 11 aa, synthetic construct
ITNTDIDDDMN

SEQ ID NO: 745 - protein, 7 aa, synthetic construct
EGNGLRP

SEQ ID NO: 746 - protein, 9 aa, synthetic construct
LQSDNLPLT

SEQ ID NO: 747 - protein, 120 aa, synthetic construct
EVQLVESGGGLVQPGGSLRLSCAASGFDFSRYWMSWVRQAPGKGLEWIGDLNPDSSAINYVDSVKGRFTISRDNAKNSLYLQMNSLRAEDTAVYYCTLITTLVPYTMDFWGQGTSVTVSS

SEQ ID NO: 748 - protein, 107 aa, synthetic construct
ETTLTQSPAFMSATPGDKVNISCITNTDIDDDMNWYQQKPGEAAILLISEGNGLRPGIPPRFSGSGYGTDFTLTINNIESEDAAYYFCLQSDNLPLTFGSGTKLEIK

SEQ ID NO: 749 - protein, 5 aa, synthetic construct
DYYMH

SEQ ID NO: 750 - protein, 17 aa, synthetic construct
WIDPENGDTEYGPKFQG

SEQ ID NO: 751 - protein, 11 aa, synthetic construct
HNAHYGTWFAY

SEQ ID NO: 752 - protein, 16 aa, synthetic construct
RSSQSLLHSSGNTYLE

SEQ ID NO: 753 - protein, 7 aa, synthetic construct
KISTRFS

SEQ ID NO: 754 - protein, 9 aa, synthetic construct
FQGSHVPYT

SEQ ID NO: 755 - protein, 120 aa, synthetic construct
QVQLVQSGAEVKKPGASVKVSCKASGLTIEDYYMHWVRQAPGQGLEWMGWIDPENGDTEYGPKFQGRVTMTRDTSINTAYMELSRLRSDDTAVYYCAVHNAHYGTWFAYWGQGTLVTVSS

SEQ ID NO: 756 - protein, 112 aa, synthetic construct
DVVMTQSPLSLPVTLGQPASISCRSSQSLLHSSGNTYLEWYQQRPGQSPRPLIYKISTRFSGVPDRFSGSGSGTDFTLKISRVEAEDVGVYYCFQGSHVPYTFGGGTKVEIK

SEQ ID NO: 757 - protein, 449 aa, synthetic construct
QVQLVQSGAEVKKPGASVKVSCKASGLTIEDYYMHWVRQAPGQGLEWMGWIDPENGDTEYGPKFQGRVTMTRDTSINTAYMELSRLRSDDTAVYYCAVHNAHYGTWFAYWGQGTLVTVSSASTKGPSVFPLAPSSKSTSGGTAALGCLVKDYFPEPVTVSWNSGALTSGVHTFPAVLQSSGLYSLSSVVTVPSSSLGTQTYICNVNHKPSNTKVDKKVEPKSCDKTHTCPPCPAPELLGGPSVFLFPPKPKDTLMISRTPEVTCVVVDVSHEDPEVKFNWYVDGVEVHNAKTKPREEQYNSTYRVVSVLTVLHQDWLNGKEYKCKVSNKALPAPIEKTISKAKGQPREPQVYTLPPSRDELTKNQVSLTCLVKGFYPSDIAVEWESNGQPENNYKTTPPVLDSDGSFFLYSKLTVDKSRWQQGNVFSCSVMHEALHNHYTQKSLSLSPG

SEQ ID NO: 758 - protein, 219 aa, synthetic construct
DVVMTQSPLSLPVTLGQPASISCRSSQSLLHSSGNTYLEWYQQRPGQSPRPLIYKISTRFSGVPDRFSGSGSGTDFTLKISRVEAEDVGVYYCFQGSHVPYTFGGGTKVEIKRTVAAPSVFIFPPSDEQLKSGTASVVCLLNNFYPREAKVQWKVDNALQSGNSQESVTEQDSKDSTYSLSSTLTLSKADYEKHKVYACEVTHQGLSSPVTKSFNRGEC

SEQ ID NO: 759 - protein, 5 aa, synthetic construct
GYFMN

SEQ ID NO: 760 - protein, 17 aa, synthetic construct
LINPYNGDSFYNQKFKG

SEQ ID NO: 761 - protein, 8 aa, synthetic construct
GLRRDFDY

SEQ ID NO: 762 - protein, 16 aa, synthetic construct
KSSQSLLDSDGKTYLN

SEQ ID NO: 763 - protein, 7 aa, synthetic construct
LVSELDS

SEQ ID NO: 764 - protein, 9 aa, synthetic construct
WQGTHFPRT

SEQ ID NO: 765 - protein, 117 aa, synthetic construct
QVQLVQSGAEVKKPGASVKVSCKASGYSFSGYFMNWVRQAPGQGLEWMGLINPYNGDSFYNQKFKGRVTMTRQTSTSTVYMELSSLRSEDTAVYYCVRGLRRDFDYWGQGTLVTVSS

SEQ ID NO: 766 - protein, 112 aa, synthetic construct
DVVMTQSPLSLPVTLGQPASISCKSSQSLLDSDGKTYLNWLFQRPGQSPRRLIYLVSELDSGVPDRFSGSGSGTDFTLKISRVEAEDVGVYYCWQGTHFPRTFGGGTKLEIK

SEQ ID NO: 767 - protein, 5 aa, synthetic construct
DFGMN

SEQ ID NO: 768 - protein, 17 aa, synthetic construct
WINTFTGEPSYGNVFKG

SEQ ID NO: 769 - protein, 10 aa, synthetic construct
RHGNGNVFDS

SEQ ID NO: 770 - protein, 11 aa, synthetic construct
RASQSIGSNIH

SEQ ID NO: 771 - protein, 7 aa, synthetic construct
YTSESIS

SEQ ID NO: 772 - protein, 9 aa, synthetic construct
QQSNSWPLT

SEQ ID NO: 773 - protein, 119 aa, synthetic construct
QVQLVQSGSELKKPGASVKVSCKASGYTFTDFGMNWVRQAPGQGLEWMGWINTFTGEPSYGNVFKGRFVFSLDTSVSTAYLQISSLKAEDTAVYYCARRHGNGNVFDSWGQGTLVTVSS

SEQ ID NO: 774 - protein, 108 aa, synthetic construct
EIVLTQSPDFQSVTPKEKVTITCRASQSIGSNIHWYQQKPDQSPKLLIKYTSESISGVPSRFSGSGSGTDFTLTINSLEAEDAATYYCQQSNSWPLTFGGGTKVEIKR

SEQ ID NO: 775 - protein, 5 aa, synthetic construct
SYAIS

SEQ ID NO: 776 - protein, 17 aa, synthetic construct
GIIPIFGTANYAQKFQG

SEQ ID NO: 777 - protein, 21 aa, synthetic construct
APLRFLEWSTQDHYYYYYMDV

SEQ ID NO: 778 - protein, 11 aa, synthetic construct
QGDSLRSYYAT

SEQ ID NO: 779 - protein, 7 aa, synthetic construct
GENKRPS

SEQ ID NO: 780 - protein, 11 aa, synthetic construct
KSRDGSGQHLV

SEQ ID NO: 781 - protein, 130 aa, synthetic construct
EVQLVQSGAEVKKPGSSVKVSCKASGGTFSSYAISWVRQAPGQGLEWMGGIIPIFGTANYAQKFQGRVTITADKSTSTAYMELSSLRSEDTAVYYCARAPLRFLEWSTQDHYYYYYMDVWGKGTTVTVSS

SEQ ID NO: 782 - protein, 108 aa, synthetic construct
SSELTQDPAVSVALGQTVRITCQGDSLRSYYATWYQQKPGQAPILVIYGENKRPSGIPDRFSGSSSGNTASLTITGAQAEDEADYYCKSRDGSGQHLVFGGGTKLTVL

SEQ ID NO: 783 - protein, 5 aa, synthetic construct
SYWIN

SEQ ID NO: 784 - protein, 17 aa, synthetic construct
NIYPSDSYTNYNQKFKD

SEQ ID NO: 785 - protein, 9 aa, synthetic construct
SWRGNSFDY

SEQ ID NO: 786 - protein, 17 aa, synthetic construct
KSSQSLLNSGNQKNYLT

SEQ ID NO: 787 - protein, 7 aa, synthetic construct
WASTRES

SEQ ID NO: 788 - protein, 9 aa, synthetic construct
QNDYSYPFT

SEQ ID NO: 789 - protein, 118 aa, synthetic construct
QVQLQQPGAELVRPGASVKLSCKASGYTFTSYWINWVKQRPGQGLEWIGNIYPSDSYTNYNQKFKDKATLTVDKSSSTAYMQLSSPTSEDSAVYYCTRSWRGNSFDYWGQGTTLTVSS

SEQ ID NO: 790 - protein, 113 aa, synthetic construct
DIVMTQSPSSLTVTAGEKVTMSCKSSQSLLNSGNQKNYLTWYQQKPGQPPKLLIYWASTRESGVPDRFTGSGSGTDFTLTISSVQAEDLAVYYCQNDYSYPFTFGSGTKLEIK

SEQ ID NO: 791 - protein, 5 aa, synthetic construct
NYGMN

SEQ ID NO: 792 - protein, 17 aa, synthetic construct
WINTNTGEPTYAEEFKG

SEQ ID NO: 793 - protein, 9 aa, synthetic construct
LGFGNAMDY

SEQ ID NO: 794 - protein, 17 aa, synthetic construct
KSSQSLLNSGNQKNYLT

SEQ ID NO: 795 - protein, 7 aa, synthetic construct
WASTRES

SEQ ID NO: 796 - protein, 9 aa, synthetic construct
QNDYSYPLT

SEQ ID NO: 797 - protein, 118 aa, synthetic construct
QIQLVQSGPELKKPGETVKISCKASGYTFTNYGMNWVKQAPGKGLKWMGWINTNTGEPTYAEEFKGRFAFSLETSASTAYLQINNLKNEDTATYFCARLGFGNAMDYWGQGTSVTVSS

SEQ ID NO: 798 - protein, 113 aa, synthetic construct
DIVMTQSPSSLTVTAGEKVTMSCKSSQSLLNSGNQKNYLTWYQQKPGQPPKLLIYWASTRESGVPDRFTGSGSGTDFTLTISSVQAEDLAVYYCQNDYSYPLTFGAGTKLELK

SEQ ID NO: 799 - protein, 5 aa, synthetic construct
SYNMN

SEQ ID NO: 800 - protein, 17 aa, synthetic construct
YISSSSSTIYYADSVKG

SEQ ID NO: 801 - protein, 8 aa, synthetic construct
AYYYGMDV

SEQ ID NO: 802 - protein, 11 aa, synthetic construct
RASQGISGWLA

SEQ ID NO: 803 - protein, 7 aa, synthetic construct
AASTLQS

SEQ ID NO: 804 - protein, 9 aa, synthetic construct
QQANSFPPT

SEQ ID NO: 805 - protein, 117 aa, synthetic construct
EVQLVESGGGLVQPGGSLRLSCAASGFTFSSYNMNWVRQAPGKGLEWVSYISSSSSTIYYADSVKGRFTISRDNAKNSLSLQMNSLRDEDTAVYYCARAYYYGMDVWGQGTTVTVSS

SEQ ID NO: 806 - protein, 107 aa, synthetic construct
DIQMTQSPSSVSASVGDRVTITCRASQGISGWLAWYQQKPGKAPKFLIYAASTLQSGVPSRFSGSGSGTDFTLTISSLQPEDFATYYCQQANSFPPTFGGGTKVEIK

SEQ ID NO: 807 - protein, 5 aa, synthetic construct
SYGMH

SEQ ID NO: 808 - protein, 17 aa, synthetic construct
VIWYDGSNQYYADSVKG

SEQ ID NO: 809 - protein, 11 aa, synthetic construct
GLTSGRYGMDV

SEQ ID NO: 810 - protein, 16 aa, synthetic construct
RSSQSLLLSHGFNYLD

SEQ ID NO: 811 - protein, 7 aa, synthetic construct
LGSSRAS

SEQ ID NO: 812 - protein, 9 aa, synthetic construct
MQPLQIPWT

SEQ ID NO: 813 - protein, 120 aa, synthetic construct
QVQLVESGGGVVQPGRSLRLSCAASGFTFSSYGMHWVRQAPGKGLEWVAVIWYDGSNQYYADSVKGRFTISRDNSKNTLFLQMHSLRAEDTAVYYCARGLTSGRYGMDVWGQGTTVTVSS

SEQ ID NO: 814 - protein, 112 aa, synthetic construct
DIVMTQSPLSLPVTPGEPASISCRSSQSLLLSHGFNYLDWYLQKPGQSPQLLIYLGSSRASGVPDRFSGSGSGTDFTLKISRVEAEDVGLYYCMQPLQIPWTFGQGTKVEIK

SEQ ID NO: 815 - protein, 5 aa, synthetic construct
NYAMS

SEQ ID NO: 816 - protein, 17 aa, synthetic construct
SISGSGDYTYYTDSVKG

SEQ ID NO: 817 - protein, 9 aa, synthetic construct
SPWGYYLDS

SEQ ID NO: 818 - protein, 11 aa, synthetic construct
RASQGISSRLA

SEQ ID NO: 819 - protein, 7 aa, synthetic construct
AASSLQS

SEQ ID NO: 820 - protein, 9 aa, synthetic construct
QQYNSYPYT

SEQ ID NO: 821 - protein, 118 aa, synthetic construct
EVQLLESGGGLVQPGGSLRLSCAASGFTFSNYAMSWVRQAPGKGLEWVSSISGSGDYTYYTDSVKGRFTISRDNSKNTLYLQMNSLRAEDTAVYYCARSPWGYYLDSWGQGTLVTVSS

SEQ ID NO: 822 - protein, 107 aa, synthetic construct
DIQMTQSPPSLSASAGDRVTITCRASQGISSRLAWYQQKPEKAPKSLIYAASSLQSGVPSRFSGSGSGTDFTLTISSLQPEDFATYYCQQYNSYPYTFGQGTKLEIK

SEQ ID NO: 823 - protein, 5 aa, synthetic construct
DHAIH

SEQ ID NO: 824 - protein, 17 aa, synthetic construct
YFSPGNDDIKYNEKFRG

SEQ ID NO: 825 - protein, 6 aa, synthetic construct
SLSTPY

SEQ ID NO: 826 - protein, 17 aa, synthetic construct
KSSQSLLNRGNHKNYLT

SEQ ID NO: 827 - protein, 7 aa, synthetic construct
WASTRES

SEQ ID NO: 828 - protein, 9 aa, synthetic construct
QNDYTYPYT

SEQ ID NO: 829 - protein, 115 aa, synthetic construct
EVQLVQSGAEVKKPGASVKVSCKASGYTFTDHAIHWVRQAPGQGLEWMGYFSPGNDDIKYNEKFRGRVTMTADKSSSTAYMELRSLRSDDTAVYFCKRSLSTPYWGQGTLVTVSS

SEQ ID NO: 830 - protein, 113 aa, synthetic construct
DIVMTQSPDSLAVSLGERATINCKSSQSLLNRGNHKNYLTWYQQKPGQPPKLLIYWASTRESGVPDRFSGSGSGTDFTLTISSLQAEDVAVYYCQNDYTYPYTFGQGTKVEIK

SEQ ID NO: 831 - protein, 5 aa, synthetic construct
SYNMH

SEQ ID NO: 832 - protein, 17 aa, synthetic construct
AIYPGNGDTSYNQKFKG

SEQ ID NO: 833 - protein, 12 aa, synthetic construct
STYYGGDWYFNV

SEQ ID NO: 834 - protein, 10 aa, synthetic construct
RASSSVSYIH

SEQ ID NO: 835 - protein, 7 aa, synthetic construct
ATSNLAS

SEQ ID NO: 836 - protein, 9 aa, synthetic construct
QQWTSNPPT

SEQ ID NO: 837 - protein, 121 aa, synthetic construct [sequence omitted]

SEQ ID NO: 838 - protein, 106 aa, synthetic construct [sequence omitted]

SEQ ID NO: 839 - protein, 5 aa, synthetic construct
DTYIH

SEQ ID NO: 840 - protein, 17 aa, synthetic construct
RIYPTNGYTRYADSVKG

SEQ ID NO: 841 - protein, 11 aa, synthetic construct
WGGDGFYAMDY

SEQ ID NO: 842 - protein, 11 aa, synthetic construct
RASQDVNTAVA

SEQ ID NO: 843 - protein, 7 aa, synthetic construct
SASFLYS

SEQ ID NO: 844 - protein, 9 aa, synthetic construct
QQHYTTPPT

SEQ ID NO: 845 - protein, 120 aa, synthetic construct [sequence omitted]

SEQ ID NO: 846 - protein, 107 aa, synthetic construct [sequence omitted]

SEQ ID NO: 847 - protein, 5 aa, synthetic construct
SYWIE

SEQ ID NO: 848 - protein, 17 aa, synthetic construct
EILPGGGDTNYNEIFKG

SEQ ID NO: 849 - protein, 8 aa, synthetic construct
RVPIRLDY

SEQ ID NO: 850 - protein, 15 aa, synthetic construct
KASQSVDYEGDSFLN

SEQ ID NO: 851 - protein, 7 aa, synthetic construct
AASNLES

SEQ ID NO: 852 - protein, 9 aa, synthetic construct
QQSNEDPLT

SEQ ID NO: 853 - protein, 117 aa, synthetic construct [sequence omitted]

SEQ ID NO: 854 - protein, 111 aa, synthetic construct [sequence omitted]

SEQ ID NO: 855 - protein, 5 aa, synthetic construct
DFAMS

SEQ ID NO: 856 - protein, 17 aa, synthetic construct
TIGRVAFHTYYPDSMKG

SEQ ID NO: 857 - protein, 11 aa, synthetic construct
HRGFDVGHFDF

SEQ ID NO: 858 - protein, 16 aa, synthetic construct
RSSETLVHSSGNTYLE

SEQ ID NO: 859 - protein, 7 aa, synthetic construct
RVSNRFS

SEQ ID NO: 860 - protein, 9 aa, synthetic construct
FQGSFNPLT

SEQ ID NO: 861 - protein, 120 aa, synthetic construct
EVQLVESGGGLVQPGGSLRLSCAASGFSFSDFAMSWVRQAPGKGLEWVATIGRVAFHTYYPDSMKGRFTISRDNSKNTLYLQMNSLRAEDTAVYYCARHRGFDVGHFDFWGQGTLVTVSS

SEQ ID NO: 862 - protein, 112 aa, synthetic construct
DIQMTQSPSSLSASVGDRVTITCRSSETLVHSSGNTYLEWYQQKPGKAPKLLIYRVSNRFSGVPSRFSGSGSGTDFTLTISSLQPEDFATYYCFQGSFNPLTFGQGTKVEIK

SEQ ID NO: 863 - protein, 6 aa, synthetic construct
NDYAWN

SEQ ID NO: 864 - protein, 16 aa, synthetic construct
YISYSGYTTYNPSLKS

SEQ ID NO: 865 - protein, 7 aa, synthetic construct
WTSGLDY

SEQ ID NO: 866 - protein, 11 aa, synthetic construct
KASDLIHNWLA

SEQ ID NO: 867 - protein, 7 aa, synthetic construct
GATSLET

SEQ ID NO: 868 - protein, 9 aa, synthetic construct
QQYWTTPFT

SEQ ID NO: 869 - protein, 116 aa, synthetic construct
EVQLVESGGGLVQPGGSLRLSCAASGYSITNDYAWNWVRQAPGKGLEWVGYISYSGYTTYNPSLKSRFTISRDTSKNTLYLQMNSLRAEDTAVYYCARWTSGLDYWGQGTLVTVSS

SEQ ID NO: 870 - protein, 107 aa, synthetic construct
DIQMTQSPSSLSASVGDRVTITCKASDLIHNWLAWYQQKPGKAPKLLIYGATSLETGVPSRFSGSGSGTDFTLTISSLQPEDFATYYCQQYWTTPFTFGQGTKVEIK

SEQ ID NO: 871 - protein, 6 aa, synthetic construct
SDYAWN

SEQ ID NO: 872 - protein, 16 aa, synthetic construct
YISNSGSTSYNPSLKS

SEQ ID NO: 873 - protein, 15 aa, synthetic construct
ERNYDYDDYYYAMDY

SEQ ID NO: 874 - protein, 17 aa, synthetic construct
KSSQSLLYRSNQKNYLA

SEQ ID NO: 875 - protein, 7 aa, synthetic construct
WASTRES

SEQ ID NO: 876 - protein, 9 aa, synthetic construct
QQYYNYPRT

SEQ ID NO: 877 - protein, 124 aa, synthetic construct
EVQLVESGGGLVQPGGSLRLSCAVSGYSITSDYAWNWVRQAPGKGLEWVGYISNSGSTSYNPSLKSRFTISRDTSKNTLYLQMNSLRAEDTAVYYCARERNYDYDDYYYAMDYWGQGTLVTVSS

SEQ ID NO: 878 - protein, 113 aa, synthetic construct
DIQMTQSPSSLSASVGDRVTITCKSSQSLLYRSNQKNYLAWYQQKPGKAPKLLIYWASTRESGVPSRFSGSGSGTDFTLTISSLQPEDFATYYCQQYYNYPRTFGQGTKVEIK

SEQ ID NO: 879 - protein, 5 aa, synthetic construct
NYWMH

SEQ ID NO: 880 - protein, 17 aa, synthetic construct
ATYRGHSDTYYNQKFKG

SEQ ID NO: 881 - protein, 12 aa, synthetic construct
GAIYDGYDVLDN

SEQ ID NO: 882 - protein, 11 aa, synthetic construct
SASQDISNYLN

SEQ ID NO: 883 - protein, 7 aa, synthetic construct
YTSNLHS

SEQ ID NO: 884 - protein, 9 aa, synthetic construct
QQYRKLPWT

SEQ ID NO: 885 - protein, 121 aa, synthetic construct
QVQLVQSGAEVKKPGSSVKVSCKASGGTFSNYWMHWVRQAPGQGLEWMGATYRGHSDTYYNQKFKGRVTITADKSTSTAYMELSSLRSEDTAVYYCARGAIYDGYDVLDNWGQGTLVTVSS

SEQ ID NO: 886 - protein, 107 aa, synthetic construct
DIQMTQSPSSLSASVGDRVTITCSASQDISNYLNWYQQKPGKAPKLLIYYTSNLHSGVPSRFSGSGSGTDFTLTISSLQPEDFATYYCQQYRKLPWTFGQGTKLEIK

SEQ ID NO: 887 - protein, 5 aa, synthetic construct
AYTMH

SEQ ID NO: 888 - protein, 17 aa, synthetic construct
WIKPNNGLANYAQKFQG

SEQ ID NO: 889 - protein, 9 aa, synthetic construct
SEITTEFDY

SEQ ID NO: 890 - protein, 15 aa, synthetic construct
KSSESVDSYANSFLH

SEQ ID NO: 891 - protein, 7 aa, synthetic construct
RASTRES

SEQ ID NO: 892 - protein, 9 aa, synthetic construct
QQSKEDPLT

SEQ ID NO: 893 - protein, 118 aa, synthetic construct
QVQLVQSGAEVKKPGASVKVSCKASGYIFTAYTMHWVRQAPGQGLEWMGWIKPNNGLANYAQKFQGRVTMTRDTSISTAYMELSRLRSDDTAVYYCARSEITTEFDYWGQGTLVTVSS

SEQ ID NO: 894 - protein, 111 aa, synthetic construct
DIVMTQSPDSLAVSLGERATINCKSSESVDSYANSFLHWYQQKPGQPPKLLIYRASTRESGVPDRFSGSGSGTDFTLTISSLQAEDVAVYYCQQSKEDPLTFGGGTKVEIK

SEQ ID NO: 895 - protein, 6 aa, synthetic construct
SDFAWN

SEQ ID NO: 896 - protein, 16 aa, synthetic construct
YISYSGNTRYQPSLKS

SEQ ID NO: 897 - protein, 7 aa, synthetic construct
AGRGFPY

SEQ ID NO: 898 - protein, 11 aa, synthetic construct
HSSQDINSNIG

SEQ ID NO: 899 - protein, 7 aa, synthetic construct
HGTNLDD

SEQ ID NO: 900 - protein, 9 aa, synthetic construct
VQYAQFPWT

SEQ ID NO: 901 - protein, 116 aa, synthetic construct
QVQLQESGPGLVKPSQTLSLTCTVSGYSISSDFAWNWIRQPPGKGLEWMGYISYSGNTRYQPSLKSRITISRDTSKNQFFLKLNSVTAADTATYYCVTAGRGFPYWGQGTLVTVSS

SEQ ID NO: 902 - protein, 107 aa, synthetic construct; identical to SEQ ID NO: 574

SEQ ID NO: 903 - protein, 5 aa, synthetic construct
DYYMA

SEQ ID NO: 904 - protein, 17 aa, synthetic construct
SINYDGSSTYYVDSVKG

SEQ ID NO: 905 - protein, 8 aa, synthetic construct
DRGYYFDY

SEQ ID NO: 906 - protein, 16 aa, synthetic construct
RSSQSLVHSNGNTYLH

SEQ ID NO: 907 - protein, 7 aa, synthetic construct
KVSNRFS

SEQ ID NO: 908 - protein, 10 aa, synthetic construct
SQSTHVPPFT

SEQ ID NO: 909 - protein, 117 aa, synthetic construct
EVQLVESGGGLVQPGGSLRLSCAASGFTFSDYYMAWVRQAPGKGLEWVASINYDGSSTYYVDSVKGRFTISRDNAKNSLYLQMNSLRAEDTAVYYCARDRGYYFDYWGQGTTVTVSS

SEQ ID NO: 910 - protein, 113 aa, synthetic construct
DVVMTQTPLSLSVTPGQPASISCRSSQSLVHSNGNTYLHWYLQKPGQSPQLLIYKVSNRFSGVPDRFSGSGSGTDFTLKISRVEAEDVGVYFCSQSTHVPPFTFGGGTKVEIK

SEQ ID NO: 911 - protein, 5 aa, synthetic construct
NAWMS

SEQ ID NO: 912 - protein, 17 aa, synthetic construct
YISSSGSTIYYADSVKG

SEQ ID NO: 913 - protein, 8 aa, synthetic construct
EGLWAFDY

SEQ ID NO: 914 - protein, 14 aa, synthetic construct
TGSSSNIGAGYVVH

SEQ ID NO: 915 - protein, 7 aa, synthetic construct
DNNKRPS

SEQ ID NO: 916 - protein, 11 aa, synthetic construct
AAWDDRLNGPV

SEQ ID NO: 917 - protein, 117 aa, synthetic construct
EVQLLESGGGLVQPGGSLRLSCAASGFTFSNAWMSWVRQAPGKGLEWVSYISSSGSTIYYADSVKGRFTISRDNSKNTLYLQMNSLRAEDTAVYYCAREGLWAFDYWGQGTLVTVSS

SEQ ID NO: 918 - protein, 111 aa, synthetic construct
ESVLTQPPSVSGAPGQRVTISCTGSSSNIGAGYVVHWYQQLPGTAPKLLIYDNNKRPSGVPDRFSGSKSGTSASLAISGLRSEDEADYYCAAWDDRLNGPVFGGGTKLTVL

SEQ ID NO: 919 - protein, 5 aa, synthetic construct
GYYWS

SEQ ID NO: 920 - protein, 16 aa, synthetic construct
EINHRGNTNDNPSLKS

SEQ ID NO: 921 - protein, 11 aa, synthetic construct
ERGYTYGNFDH

SEQ ID NO: 922 - protein, 11 aa, synthetic construct
RASQSVSRNLA

SEQ ID NO: 923 - protein, 7 aa, synthetic construct
GASTRAT

SEQ ID NO: 924 - protein, 9 aa, synthetic construct
QQYKTWPRT

SEQ ID NO: 925 - protein, 119 aa, synthetic construct
QVQLQQWGAGLLKPSETLSLTCAVFGGSFSGYYWSWIRQPPGKGLEWIGEINHRGNTNDNPSLKSRVTISVDTSKNQFALKLSSVTAADTAVYYCARERGYTYGNFDHWGQGTLVTVSS

SEQ ID NO: 926 - protein, 107 aa, synthetic construct
EIVMTQSPATLSVSPGERATLSCRASQSVSRNLAWYQQKPGQAPRLLIYGASTRATGIPARFSGSGSGTEFTLTIGSLQSEDFAVYYCQQYKTWPRTFGQGTNVEIK

SEQ ID NO: 927 - protein, 5 aa, synthetic construct
SYAMN

SEQ ID NO: 928 - protein, 17 aa, synthetic construct
TTSGSGASTYYADSVKG

SEQ ID NO: 929 - protein, 7 aa, synthetic construct
IWIAFDI

SEQ ID NO: 930 - protein, 12 aa, synthetic construct
RASQSVSSSYLA

SEQ ID NO: 931 - protein, 7 aa, synthetic construct
GASSRAT

SEQ ID NO: 932 - protein, 9 aa, synthetic construct
QQYGSSPYT

SEQ ID NO: 933 - protein, 116 aa, synthetic construct
EVQLLESGGGLVQPGGSLRLSCAASGFTFSSYAMNWVRQAPGKGLEWVSTTSGSGASTYYADSVKGRFTISRDNSKNTLYLQMNSLRAEDTAVYYCAKIWIAFDIWGQGTMVTVSS

SEQ ID NO: 934 - protein, 108 aa, synthetic construct
EIVLTQSPGTLSLSPGERATLSCRASQSVSSSYLAWYQQKPGQAPRLLIYGASSRATGIPDRFSGSGSGTDFTLTISRLEPEDFAVYYCQQYGSSPYTFGQGTKLEIK

SEQ ID NO: 935 - protein, 7 aa, synthetic construct
SFNYYWS

SEQ ID NO: 936 - protein, 16 aa, synthetic construct
YIYYSGSTYSNPSLKS

SEQ ID NO: 937 - protein, 9 aa, synthetic construct
GYNWNYFDY

SEQ ID NO: 938 - protein, 11 aa, synthetic construct
RASQSVDNNLV

SEQ ID NO: 939 - protein, 7 aa, synthetic construct
GASTRAT

SEQ ID NO: 940 - protein, 10 aa, synthetic construct [sequence omitted]

SEQ ID NO: 941 - protein, 119 aa, synthetic construct [sequence omitted]

SEQ ID NO: 942 - protein, 108 aa, synthetic construct [sequence omitted]

SEQ ID NO: 943 - protein, 449 aa, synthetic construct
QVQLQESGPGLVKPSQTLSLTCTVSGGSISSFNYYWSWIRHHPGKGLEWIGYIYYSGSTYSNPSLKSRVTISVDTSKNQFSLTLSSVTAADTAVYYCARGYNWNYFDYWGQGTLVTVSSASTKGPSVFPLAPSSKSTSGGTAALGCLVKDYFPEPVTVSWNSGALTSGVHTFPAVLQSSGLYSLSSVVTVPSSSLGTQTYICNVNHKPSNTKVDKKVEPKSCDKTHTCPPCPAPELLGGPSVFLFPPKPKDTLMISRTPEVTCVVVDVSHEDPEVKFNWYVDGVEVHNAKTKPREEQYNSTYRVVSVLTVLHQDWLNGKEYKCKVSNKALPAPIEKTISKAKGQPREPQVYTLPPSRDELTKNQVSLTCLVKGFYPSDIAVEWESNGQPENNYKTTPPVLDSDGSFFLYSKLTVDKSRWQQGNVFSCSVMHEALHNHYTQKSLSLSPGK

SEQ ID NO: 944 - protein, 215 aa, synthetic construct
EIVMTQSPATLSVSPGERATLSCRASQSVDNNLVWYQQKPGQAPRLLIYGASTRATGIPARFSGSGSGTEFTLTISSLQSEDFAVYYCQQYNNWPPWTFGQGTKVEIKRTVAAPSVFIFPPSDEQLKSGTASVVCLLNNFYPREAKVQWKVDNALQSGNSQESVTEQDSKDSTYSLSSTLTLSKADYEKHKVYACEVTHQGLSSPVTKSFNRGEC

SEQ ID NO: 945 - protein, 5 aa, synthetic construct
TYWMH

SEQ ID NO: 946 - protein, 17 aa, synthetic construct
EIDPSDSYSNYNQKFKD

SEQ ID NO: 947 - protein, 11 aa, synthetic construct
NGGLGPAWFSY

SEQ ID NO: 948 - protein, 11 aa, synthetic construct
KASQYVGTAVA

SEQ ID NO: 949 - protein, 7 aa, synthetic construct
SASNRYT

SEQ ID NO: 950 - protein, 9 aa, synthetic construct
QQYSSYPWT

SEQ ID NO: 951 - protein, 120 aa, synthetic construct
EVQLVQSGAEVKKPGSSVKVSCKASGYTFTTYWMHWVRQAPGQGLEWIGEIDPSDSYSNYNQKFKDRATLTVDKSTSTAYMELSSLRSEDTAVYYCARNGGLGPAWFSYWGQGTLVTVSS

SEQ ID NO: 952 - protein, 107 aa, synthetic construct
DIQMTQSPSSVSASVGDRVTITCKASQYVGTAVAWYQQKPGKSPKLLIYSASNRYTGVPSRFSDSGSGTDFTLTISSLQPEDFATYFCQQYSSYPWTFGGGTKVEIK

SEQ ID NO: 953 - protein, 5 aa, synthetic construct
SYAMS

SEQ ID NO: 954 - protein, 17 aa, synthetic construct
AISGSGTSTYYADSVKG

SEQ ID NO: 955 - protein, 13 aa, synthetic construct
VRYNWNHGDWFDP

SEQ ID NO: 956 - protein, 13 aa, synthetic construct
SGSSSNIGNNYVS

SEQ ID NO: 957 - protein, 7 aa, synthetic construct
ENYNRPA

SEQ ID NO: 958 - protein, 11 aa, synthetic construct
SSWDDSLNYWV

SEQ ID NO: 959 - protein, 122 aa, synthetic construct
EVQLLESGGGLVQPGGSLRLSCAASGFTFSSYAMSWVRQAPGKGLEWVSAISGSGTSTYYADSVKGRFTISRDNSKNTLYLQMNSLRAEDTAVYYCARVRYNWNHGDWFDPWGQGTLVTVSS

SEQ ID NO: 960 - protein, 110 aa, synthetic construct
QSVLTQPPSASGTPGQRVTISCSGSSSNIGNNYVSWYQQLPGTAPKLLIYENYNRPAGVPDRFSGSKSGTSASLAISGLRSEDEADYYCSSWDDSLNYWVFGGGTKLTVL

SEQ ID NO: 961 - protein, 5 aa, synthetic construct
SYGMS

SEQ ID NO: 962 - protein, 17 aa, synthetic construct
TISSGGSYKYYVDSVKG

SEQ ID NO: 963 - protein, 11 aa, synthetic construct
HPDYDGVWFAY

SEQ ID NO: 964 - protein, 10 aa, synthetic construct
SVSSSVFYVH

SEQ ID NO: 965 - protein, 7 aa, synthetic construct
DTSKLAS

SEQ ID NO: 966 - protein, 9 aa, synthetic construct
QQWNSNPPT

SEQ ID NO: 967 - protein, 120 aa, synthetic construct
EVQLVESGGGLVQPGGSLRLSCAASGFTFNSYGMSWVRQAPGKGLEWVATISSGGSYKYYVDSVKGRFTISRDNAKNSLYLQMNSLRAEDTAVYYCARHPDYDGVWFAYWGQGTLVTVSS

SEQ ID NO: 968 - protein, 106 aa, synthetic construct
DIQMTQSPSSLSASVGDRVTITCSVSSSVFYVHWYQQKPGKAPKLLIYDTSKLASGVPSRFSGSGSGTDFTFTISSLQPEDIATYYCQQWNSNPPTFGGGTKVEIK

SEQ ID NO: 969 - protein, 5 aa, synthetic construct
SYGMS

SEQ ID NO: 970 - protein, 17 aa, synthetic construct
TISSGGSYTYYPDSVKG

SEQ ID NO: 971 - protein, 11 aa, synthetic construct
HPDYDGVWFAY

SEQ ID NO: 972 - protein, 10 aa, synthetic construct
SVSSSVFYVH

SEQ ID NO: 973 - protein, 7 aa, synthetic construct
DTSKLAS

SEQ ID NO: 974 - protein, 9 aa, synthetic construct
QQWNSNPPT

SEQ ID NO: 975 - protein, 120 aa, synthetic construct
EVQLVESGGDLVKPGGSLKLSCAASGFTFNSYGMSWVRQTPDKRLEWVATISSGGSYTYYPDSVKGRFTISRDNAKNTLYLQMSSLKSEDTAMYYCARHPDYDGVWFAYWGQGTLVTVSA

SEQ ID NO: 976 - protein, 106 aa, synthetic construct
QIVLTQSPAIMSASPGEKVTMTCSVSSSVFYVHWYQQKSGTSPKRWIYDTSKLASGVPARFSGSGSGTSYSLTISSMEAEDAATYYCQQWNSNPPTFGGGTKLEIK

SEQ ID NO: 977 - protein, 5 aa, synthetic construct
SYYMH

SEQ ID NO: 978 - protein, 17 aa, synthetic construct
IINPSGGSTSYAQKFQG

SEQ ID NO: 979 - protein, 19 aa, synthetic construct
DGVLRYFDWLLDYYYYMDV

SEQ ID NO: 980 - protein, 11 aa, synthetic construct
RASQSVGSYLA

SEQ ID NO: 981 - protein, 7 aa, synthetic construct
DASNRAT

SEQ ID NO: 982 - protein, 8 aa, synthetic construct
QQRANVFT

SEQ ID NO: 983 - protein, 128 aa, synthetic construct
EVQLVQSGAEVKKPGASVKVSCKASGYTFTSYYMHWVRQAPGQGLEWMGIINPSGGSTSYAQKFQGRVTMTRDTSTSTVYMELSSLRSEDTAVYYCARDGVLRYFDWLLDYYYYMDVWGKGTTVTVSS

SEQ ID NO: 984 - protein, 106 aa, synthetic construct
EIVLTQSPATLSLSPGERATLSCRASQSVGSYLAWYQQRPGQAPRLLIYDASNRATGIPARFSGSGSGTDFTLTISSLEPEDFAVYYCQQRANVFTFGQGTKVEIK

SEQ ID NO: 985 - protein, 5 aa, synthetic construct
SYYMH

SEQ ID NO: 986 - protein, 17 aa, synthetic construct
IINPSGGSTSYAQKFQG

SEQ ID NO: 987 - protein, 19 aa, synthetic construct
DAELRHFDHLLDYHYYMDV

SEQ ID NO: 988 - protein, 11 aa, synthetic construct
RASQSVGSYLA

SEQ ID NO: 989 - protein, 7 aa, synthetic construct
DASNRAT

SEQ ID NO: 990 - protein, 8 aa, synthetic construct
QQRAQEFT

SEQ ID NO: 991 - protein, 128 aa, synthetic construct
EVQLVQSGAEVKKPGASVKVSCKASGYTFTSYYMHWVRQAPGQGLEWMGIINPSGGSTSYAQKFQGRVTMTRDTSTSTVYMELSSLRSEDTAVYYCARDAELRHFDHLLDYHYYMDVWGQGTTVTVSS

SEQ ID NO: 992 - protein, 106 aa, synthetic construct
EIVMTQSPATLSLSPGERATLSCRASQSVGSYLAWYQQKPGQAPRLLIYDASNRATGIPARFSGSGSGTDFTLTISSLQPEDFAVYYCQQRAQEFTFGQGTKVEIK

SEQ ID NO: 993 - protein, 120 aa, synthetic construct
QVQLVQSGSELKKPGAPVKVSCKASGYTFSTFGMSWVRQAPGQGLKWMGWIHTYAGVPIYGDDFKGRFVFSLDTSVSTAYLQISSLKAEDTAVYFCARRSDNYRYFFDYWGQGTTVTVSS

SEQ ID NO: 994 - protein, 107 aa, synthetic construct
DIQMTQSPSSLSASLGDRVTITCRASQDIRNYLNWYQQKPGKAPKLLIYYTSRLHSGVPSRFSGSGSGTDYTLTISSLQPEDFATYFCQQGHTLPPTFGQGTKLEIK

SEQ ID NO: 995 - protein, 120 aa, synthetic construct
QIQLVQSGPELKKPGAPVKISCKASGYTFTTFGMSWVKQAPGQGLKWMGWIHTYAGVPIYGDDFKGRFVFSLDTSVSTAYLQISSVKAEDTATYFCARRSDNYRYFFDYWGQGTTLTVSS

SEQ ID NO: 996 - protein, 107 aa, synthetic construct; identical to SEQ ID NO: 994

SEQ ID NO: 997 - protein, 5 aa, synthetic construct
NYYMA

SEQ ID NO: 998 - protein, 17 aa, synthetic construct
SITKGGGNTYYRDSVKG

SEQ ID NO: 999 - protein, 14 aa, synthetic construct
QVTIAAVSTSYFDS

SEQ ID NO: 1000 - protein, 15 aa, synthetic construct
KTNQKVDYYGNSYVY

SEQ ID NO: 1001 - protein, 7 aa, synthetic construct
LASNLAS

SEQ ID NO: 1002 - protein, 9 aa, synthetic construct
QQSRNLPYT

SEQ ID NO: 1003 - protein, 123 aa, synthetic construct
EVQLVESGGGLVQSGRSIRLSCAASGFSFSNYYMAWVRQAPSKGLEWVASITKGGGNTYYRDSVKGRFTFSRDNAKSTLYLQMDSLRSEDTATYYCARQVTIAAVSTSYFDSWGQGVMVTVSS

SEQ ID NO: 1004 - protein, 110 aa, synthetic construct
DIVLTQSPALAVSLGQRATISCKTNQKVDYYGNSYVYWYQQKPGQQPKLLIYLASNLASGIPARFSGRGSGTDFTLTIDPVEADDTATYYCQQSRNLPYTFGAGTKLELK

SEQ ID NO: 1005 - protein, 5 aa, synthetic construct
DYYMK

SEQ ID NO: 1006 - protein, 17 aa, synthetic construct
DIIPSNGATFYNQKFKG

SEQ ID NO: 1007 - protein, 11 aa, synthetic construct
SHLLRASWFAY

SEQ ID NO: 1008 - protein, 17 aa, synthetic construct
KSSQSLLNSGNQKNYLT

SEQ ID NO: 1009 - protein, 7 aa, synthetic construct
WASTRES

SEQ ID NO: 1010 - protein, 9 aa, synthetic construct
QNDYSYPYT

SEQ ID NO: 1011 - protein, 120 aa, synthetic construct
QVQLVQSGAEVKKPGASVKMSCKASGYTFTDYYMKWVKQAPGQGLEWIGDIIPSNGATFYNQKFKGKATLTVDRSISTAYMHLNRLRSDDTAVYYCTRSHLLRASWFAYWGQGTLVTVSS

SEQ ID NO: 1012 - protein, 113 aa, synthetic construct
DFVMTQSPDSLAVSLGERATINCKSSQSLLNSGNQKNYLTWYLQKPGQPPKLLIYWASTRESGVPDRFSGSGSGTDFTLTISSLQAEDVAVYYCQNDYSYPYTFGQGTKLEIK

SEQ ID NO: 1013 - protein, 5 aa, synthetic construct
DYEMH

SEQ ID NO: 1014 - protein, 17 aa, synthetic construct
GIDPETGGTAYNQKFKG

SEQ ID NO: 1015 - protein, 6 aa, synthetic construct
YYSFAY

SEQ ID NO: 1016 - protein, 16 aa, synthetic construct
RSSQSIVHSNANTYLQ

SEQ ID NO: 1017 - protein, 7 aa, synthetic construct
KVSNRFS

SEQ ID NO: 1018 - protein, 9 aa, synthetic construct
FQVSHVPYT

SEQ ID NO: 1019 - protein, 115 aa, synthetic construct
EVQLVQSGAEVKKPGATVKISCKVSGYTFTDYEMHWVQQAPGKGLEWMGGIDPETGGTAYNQKFKGRVTLTADKSTDTAYMELSSLRSEDTAVYYCGRYYSFAYWGQGTLVTVSS

SEQ ID NO: 1020 - protein, 112 aa, synthetic construct
DVVMTQSPLSLPVTLGQPASISCRSSQSIVHSNANTYLQWFQQRPGQSPRLLIYKVSNRFSGVPDRFSGSGSGTDFTLKISRVEAEDVGVYYCFQVSHVPYTFGQGTKLEIK

SEQ ID NO: 1021 - protein, 5 aa, synthetic construct
SYAIS

SEQ ID NO: 1022 - protein, 17 aa, synthetic construct
SIIPIFGTANYAQKFQG

SEQ ID NO: 1023 - protein, 16 aa, synthetic construct
GPSEVGAILGYVWFDP

SEQ ID NO: 1024 - protein, 16 aa, synthetic construct
RSSQSLLHSNGYNYLD

SEQ ID NO: 1025 - protein, 7 aa, synthetic construct
LGSNRAS

SEQ ID NO: 1026 - protein, 9 aa, synthetic construct
MQARRIPIT

SEQ ID NO: 1027 - protein, 125 aa, synthetic construct
QVQLVQSGAEVKKPGSSVKVSCKASGGTFSSYAISWVRQAPGQGLEWMGSIIPIFGTANYAQKFQGRVTITADESTSTAYMELSSLRSEDTAVYYCARGPSEVGAILGYVWFDPWGQGTLVTVSS

SEQ ID NO: 1028 - protein, 112 aa, synthetic construct
DIVMTQSPLSLPVTPGEPASISCRSSQSLLHSNGYNYLDWYLQKPGQSPQLLIYLGSNRASGVPDRFSGSGSGTDFTLKISRVEAEDVGVYYCMQARRIPITFGGGTKVEIK

SEQ ID NO: 1029 - protein, 5 aa, synthetic construct
NYDIN

SEQ ID NO: 1030 - protein, 17 aa, synthetic construct
WIYPGDGSTKYNEKFKA

SEQ ID NO: 1031 - protein, 8 aa, synthetic construct
GYEDAMDY

SEQ ID NO: 1032 - protein, 11 aa, synthetic construct
KASQDINSYLS

SEQ ID NO: 1033 - protein, 7 aa, synthetic construct
RANRLVD

SEQ ID NO: 1034 - protein, 9 aa, synthetic construct
LQYDEFPLT

SEQ ID NO: 1035 - protein, 117 aa, synthetic construct
QVQLVQSGAEVKKPGASVKVSCKASGYTFTNYDINWVRQAPGQGLEWIGWIYPGDGSTKYNEKFKAKATLTADTSTSTAYMELRSLRSDDTAVYYCASGYEDAMDYWGQGTTVTVSS

SEQ ID NO: 1036 - protein, 106 aa, synthetic construct
DIQMTQSPSSLSASVGDRVTINCKASQDINSYLSWFQQKPGKAPKTLIYRANRVDGVPSRFSGSGSGQDYTLTISSLQPEDFATYYCLQYDEFPLTFGGGTKVEIK

SEQ ID NO: 1037 - protein, 5 aa, synthetic construct
DYYIH

SEQ ID NO: 1038 - protein, 17 aa, synthetic construct
YINPNSGYTNYAQKFQG

SEQ ID NO: 1039 - protein, 12 aa, synthetic construct
YMWERVTGFFDF

SEQ ID NO: 1040 - protein, 11 aa, synthetic construct
LASEDISDDLA

SEQ ID NO: 1041 - protein, 7 aa, synthetic construct
TTSSLQS

SEQ ID NO: 1042 - protein, 9 aa, synthetic construct
QQTYKFPPT

SEQ ID NO: 1043 - protein, 121 aa, synthetic construct
QVQLVQSGAEVKKPGASVKLSCKASGYTFTDYYIHWVRQAPGQGLEWIGYINPNSGYTNYAQKFQGRATMTADKSINTAYVELSRLRSDDTAVYFCTRYMWERVTGFFDFWGQGTMVTVSS

SEQ ID NO: 1044 - protein, 107 aa, synthetic construct
DIQMTQSPSSVSASVGDRVTITCLASEDISDDLAWYQQKPGKAPKVLVYTTSSLQSGVPSRFSGSGSGTDFTLTISSLQPEDFATYFCQQTYKFPPTFGGGTKVEIK